European Patent Specification EP 3 169 786 B1, published October 23, 2024. Title: QTLs ASSOCIATED WITH AND METHODS FOR IDENTIFYING. Applicant: E.I. DuPont DeNemours & Company. The sequence listing filed with the application follows.

SEQUENCE LISTING (830 sequences)

SEQ ID NO: 1 - DNA, 401 bp, Brassica napus
aaggagagactaaggaaggagcatatgcactgacctttgcatccgtccggtgtatatgcgtttcctgtgtgcaaccacaatgtgcataactaatattagaaatggtggttttgtcgcagatgcacttcatttgggatttagtcgaggaagtattacgtcggtactcttttctgttgtcgcagggcaaggaactcaggaatkaatgattctttgtttgtatcacccatcctagagtaagggtagcatatcccttaccaagtaactgtgttggtcttgtcgcattggacaaagtgtagacttcatccgtcatgaaggccactctacaatgttcttctcttgttgttgttgttgttgtcgagtttccaccattgctctctctatcatgatgccaatagtttgtt

SEQ ID NO: 2 - DNA, 151 bp, Brassica napus
  misc_feature (98)..(98): n is a, c, g, or t
  misc_feature (102)..(102): n is a, c, g, or t
  misc_feature (116)..(116): n is a, c, g, or t
gcttgatctcttcaattcggggattagagctttccggtactcatgcggccccaatccagaatcgatctctcactasggactacttcccttggtacagncgtncccaaggtcgccanttcgcttcgaaatcaaacggtactgatgaaagcag

SEQ ID NO: 3 - DNA, 121 bp, Brassica napus
  misc_feature (9)..(9): n is a, c, g, or t
  misc_feature (65)..(65): n is a, c, g, or t
  misc_feature (106)..(106): n is a, c, g, or t
ttttgtccntagctattcataattaatcaaaaaggtggtccaattttacaccttagtgctrtgantatctttcatacatctctagagtggaacatatgatactgcnaattgcagttatatt

SEQ ID NO: 4 - DNA, 401 bp, Brassica napus
ttatgatggtgacaggagttaagtgtgcatgtgaatgtagatgactgaaaaagatagccaactacttataaccaacatacgaccttttggtctttcctcttctctctctcaacttattttgattatacaaaatgttatgtttgcaaactggcatttaactgggccgcttagctctcttcggttatttttttcttgtgataraccacattcagatatatatatgtcatctcgtcatgtgctgttgttgttttctatatcgtttcgattaatcaagaagttgggaacgtcggaactccaaaccaaatgtcctacgattattaattatacatgtatcctgatcatatctatctaacatgaacgaaaatttgaatctactataaaagaaatattagagacaattc

SEQ ID NO: 5 - DNA, 801 bp, Brassica napus
  misc_feature (1)..(90): n is a, c, g, or t
  misc_feature (214)..(214): n is a, c, g, or t
  misc_feature (229)..(229): n is a, c, g, or t
  misc_feature (384)..(384): n is a, c, g, or t
  misc_feature (561)..(561): n is a, c, g, or t
  misc_feature (633)..(732): n is a, c, g, or t
nnnnnnnnnnnnnnnnnnnnnnnnnnnnnnnnnnnnnnnnnnnnnnnnnnnnnnnnnnnnnnnnnnnnnnnnnnnnnnnnnnnnnnnnnnataactcttttattcaagtggagtttcaactttttgtaaacctcagaatgcttcttttgttccttcaaattcaaacaataatgaataatataacatactctttttatacgcgatattacattanattcaaattcgaatnttcttggatcaaatgcttcaggcctcatgtatgtgggccaattttgaatggaatcgttgggttatacttagaagtagattcatcaggtttagttatgtggggctcatgactcgcgtccattgatcaaacaacaagccctctcatgtacaatgtangattatgttttcttcayaatcaactagttagatttgatgcatagcggtggttaacacataaccgatttgtttttcaattagttgtggacaagcaactctaatttctgaatatagattttatttagtcatatgattagcgccaaagattaacacaaaagttattgaccatagtctacngaaatcacaaccaaacacgagatacggcattgtcaaacacaaagtctaaaagagaatataaagtttgagacnnnnnnnnnnnnnnnnnnnnnnnnnnnnnnnnnnnnnnnnnnnnnnnnnnnnnnnnnnnnnnnnnnnnnnnnnnnnnnnnnnnnnnnnnnnnnnnnnnnnaggtcaggagaaggttctacaagaactgggcaaagtccaagaagaaggctttcaccgggtacgccaagc

SEQ ID NO: 6 - DNA, 801 bp, Brassica napus
  misc_feature (14)..(113): n is a, c, g, or t
  misc_feature (336)..(336): n is a, c, g, or t
  misc_feature (339)..(339): n is a, c, g, or t
  misc_feature (614)..(614): n is a, c, g, or t
  misc_feature (705)..(705): n is a, c, g, or t
  misc_feature (780)..(780): n is a, c, g, or t
acaataaaaatatnnnnnnnnnnnnnnnnnnnnnnnnnnnnnnnnnnnnnnnnnnnnnnnnnnnnnnnnnnnnnnnnnnnnnnnnnnnnnnnnnnnnnnnnnnnnnnnnnnnncactttgatatccataaacctaatcttttataaaccccctcttgaggttctatcctctgcgctcggctgtactttaggagaaatctacaccgtttattttccctgagattaaaatttaatcaccctacgctcttattgggccgggccgggccgagtttgtactgagaaattggtttgagtgaactaatcctctgtagaaagctataccgtacacaaaatcagngcnttttcttcaccgtacgatgaatcagacgaaagtaggatttttttttagtgaacagagagatkaattgggccaggcccattagtagcttcgttctataatttattcgtttcttagaacagaagagtttttgattgtgcaaaaatcagaaagagacgatcacgaagatggcgacggagagctcttcagctaagagatggcttcctcttgaagctaacccagaggttatgaatcaggtattcgtctcactttcccttcttcttcttctccgatcatcngcttttttttcgaaattgggaagattgattctaggtcagttcagtgatttttttttgtattggtgtgtattgtgtacagtttctttggggnctgggtcttgcaccagatgcagcggagtgcaatgatgtgtttggattcgacgacgaacttcttgagatggttccnaagcctgttcttgctgttctc

SEQ ID NO: 7 - DNA, 801 bp, Brassica napus
  misc_feature (69)..(69): n is a, c, g, or t
  misc_feature (423)..(423): n is a, c, g, or t
  misc_feature (676)..(676): n is a, c, g, or t
  misc_feature (748)..(801): n is a, c, g, or t
agcaccaccatcgacatgcgaccccttaggtaacaccatatccgaaacattttagtagctgttattttntttctgattaagatttagccttcatattcttcttggatcataactctttatttgctatattcaatgcacagtcatgaattcatattccatccattattttcgttaatcactcgtaaaatgcatattatattgaggaaaaataacaactccacttaattagacttatatgagccgtttcaaatgtttgaaaaatcaacacaactagatatataattttcttactgatattgtggaaattggctggatgttcaaatgaaataattaatccgcatgaattgatgatgcttcccttcaaagaaagacatttctaatatggataccttgtttttgtrcaacttctaatatggataccangcattcaaaaatatgtaaatgtaatataggctttgattggtaacatgtaaatacttttgagttagacatacaactaacaaatgttaccaactttgaatttttgaaattgtctttgagttgtgatggattattgttgagttacaattttgtgttataacctttataaaattgaccactcaaatgttaaatcaagataaaaaaaatctcatgtattaaaatttgaattggaaaaatgggtttcataataattgcncacgtccatattttattttaacaaattaaacaatttacaaaacatgatcatatagtttagtacgtttaggtnnnnnnnnnnnnnnnnnnnnnnnnnnnnnnnnnnnnnnnnnnnnnnnnnnnnnn

SEQ ID NO: 8 - DNA, 598 bp, Brassica napus
  misc_feature (28)..(28): n is a, c, g, or t
  misc_feature (35)..(36): n is a, c, g, or t
  misc_feature (44)..(44): n is a, c, g, or t
  misc_feature (77)..(77): n is a, c, g, or t
  misc_feature (179)..(179): n is a, c, g, or t
aatctccgaacagagagacatccttgtnaaaagtnngagacttngcgaacccatcaaatgaaaaggaggagttctcntgtgtagtagccatggttccrtaactcacgaagcacagagcaaagaaaaaggatagagctttgagcaacatcgccatagctttgaacagggacaagctcttnttcttcttcttcttcttctagatggaatcttttaggaatcgagaaagagttttactttttcaagaagacaagtaaagttgttttctttgtttttgtgtggatttacgtgaagaagaagattaaaatataatctttgcagaaaccagagaccacgattcgctctcattctctttcttgtagtgcttgctgactaaaggttgtgaatgcatttaatgctgtttctgatgttttttaattcaatgttattattacattctcttttgtttagcctttgagattatgaaacctatgcgcattttcttcaaaacgtttataacatacattaaaatggttgaagaggctttgcttcacactttttgttttacttacgatcagatggttacatacatatatgtaaggacagcttgagtgaatagtac

SEQ ID NO: 9 - DNA, 801 bp, Brassica napus
  misc_feature (188)..(188): n is a, c, g, or t
  misc_feature (305)..(305): n is a, c, g, or t
  misc_feature (447)..(447): n is a, c, g, or t
  misc_feature (493)..(493): n is a, c, g, or t
  misc_feature (615)..(714): n is a, c, g, or t
tcgagctcgttgcgcgcatagggaaacacgtgtacagcagaaatggagtactcacggaggtcaaatccttcggcaaggtcgaattgggttacggcattagaaagctcgacggcagacactatcaggtaccaatgagaattgattcaatttttgccttgttgaatcggtgattagtcgagtccgtagantttgttttgattaggttggccttttggtaaaagctttgctttagcatctttctgatcgattcctattgttaaagaaactagcttttgagcctttgagttgaattatcgaagcagcanagttttgaattttgaattagtttattcaaattagtcacaaggattcttgattcacctctttgagctaacactagtcacaaagatatacagaaccamcatgggtttgcttggtagcattttgtcccttggatctttcagtgtntatatataataacatagttatgtgtgggtgaatggcgcagggacanttgatgcagataacaatgatggcaacaccaaacatgaacaaggagcttcactacctcaacaaggaagacaaactcctgcgctggctcctcgttaaacaccgcgacatcaagattggagcttnnnnnnnnnnnnnnnnnnnnnnnnnnnnnnnnnnnnnnnnnnnnnnnnnnnnnnnnnnnnnnnnnnnnnnnnnnnnnnnnnnnnnnnnnnnnnnnnnnnnacaatcaaagctaatcgagaatggttaaccaaatcgaataaagagtagtcgggatcgttacccataacgacggaactgatccctaac

SEQ ID NO: 10 - DNA, 697 bp, Brassica napus
  misc_feature (43)..(43): n is a, c, g, or t
  misc_feature (148)..(148): n is a, c, g, or t
  misc_feature (199)..(199): n is a, c, g, or t
  misc_feature (247)..(247): n is a, c, g, or t
  misc_feature (427)..(427): n is a, c, g, or t
  misc_feature (460)..(460): n is a, c, g, or t
  misc_feature (466)..(466): n is a, c, g, or t
  misc_feature (532)..(532): n is a, c, g, or t
  misc_feature (574)..(574): n is a, c, g, or t
  misc_feature (580)..(580): n is a, c, g, or t
  misc_feature (592)..(592): n is a, c, g, or t
aagagcaagggtactagcattcactgtgtgttgctgcagaacnggtccaaagaccatggtagggcaaatgctgacgagactaatcccggttcgttttgcaaactcgaaagcttcactttctgcttgtgtctttgacgcacaataccanttctcagttcttttgcaaaactccaggtcagaccaacaagactcatctatnactcgatcctttgaccaattagggttcatcataagcgcagctgcagangaaacgtacayaacacgcttaacatttgcttcgacacaagctttaagcacattcaacgtgccatccacagctggtgccatcacttccacctcagggtttgggactgaagatgatggaacagggctagcgacatggaagacgccgatgcaacctgcgatcgcagattgaagagaggcgtantcaagcaaatcagccttgacgagcttgagtttntcaccngctttctccagcttcttcaaatgagaatacttttcgttatcagggtctctgacagtgccatggacnaagtaatccttggagaggaggagatcgacgacccacgaagcnagaaancctccggcaccngtaacgcaaacctttcctttcgccgccaccgacatttttttattttttttatctccgagatgcttcttcaatattcttctaccttgtctgaatgccaggtgtgtc

SEQ ID NO: 11 - DNA, 151 bp, Brassica napus
  misc_feature (101)..(101): n is a, c, g, or t
tcccgtgttaatgattttacacgttattatcacaataaaaccagagcttccaaattcttggttctgtgtaatcatytggaaaagaaaaaagagaaaaaaantgaatatgtaaatgatgtgatttttggttcgttgcggtttgcatgctcta

SEQ ID NO: 12 - DNA, 401 bp, Brassica napus
ccctaaaaacagtcatattaatcgggggcctgaggcgaatacctttttcaatacactgtaggcacgcctctgatgaaaactacagaaaacttttcattttgccgtgttcatatcggcttacatatagagaacaattaacacatcacctgaccgaaagaaacactagttaagaaaatatagtactaaagataaaattactgwtattagcaatttagcatagctaaatgaagaataattcttacagaaagaattgtaaaccttaattttctcaaaaaaaaaagaactaggataataaattatggtttagtatagcttataaggttttaaatataatgtgtatatcatataattctttcagagaaaaatcattttttctacggtaggaatgtagataagaaaaa

SEQ ID NO: 13 - DNA, 151 bp, Brassica napus
  misc_feature (13)..(13): n is a, c, g, or t
  misc_feature (44)..(45): n is a, c, g, or t
atgagcagacccnttttttatcttttgttgaatggggatttttnngacagtggaggagcttctccaacttccaaaktatcaaatttagctgtctttttctattttcttttgacgtatgtaactcttacatgctcaattctaagttggtaac

SEQ ID NO: 14 - DNA, 626 bp, Brassica napus
  misc_feature (182)..(182): n is a, c, g, or t
  misc_feature (191)..(191): n is a, c, g, or t
  misc_feature (371)..(371): n is a, c, g, or t
  misc_feature (423)..(423): n is a, c, g, or t
  misc_feature (446)..(446): n is a, c, g, or t
  misc_feature (606)..(608): n is a, c, g, or t
agaagcttgctaatattccgacgccggaagccaccgtggacgacgtagacttcaaaggtgtgactcgtcaaggagttgattatcacgccaaggtctccgtcaagaatccttaccctcaggccatccctatttgccagatctcttacatcctcaagagtgacacaaggatgatagcgtctggnacaataccngatccgggttcgttgatcgcgaacgggtcgacggttcttgacgtaccggtcaaggtgccttatagcatagcggtgagtttgatgaaggacatgtgtttggactgggacattgactatcaactcgatattggactgaccatcgatattcctattgttggtgacattactattcctgtctcnactcagggtgagatgaagctcccttcccttcgcgacttcttttaatcatctntataagttataatctgatttttnaataagtacgatccgtaaacgacatagacgatcgttggatgtttcagttgtggaytcttgtgtttgttggttatatgtatttgttgctttgaatattttgttggtgagagttaaaaactacaagatgtcatagttcgaatactaacgaagtgatggagannnaaaaaaaaaaaaaaaaaa

SEQ ID NO: 15 - DNA, 301 bp, Brassica napus
agctggattttgtttcttctacaaaaatgttggatttaaagagttttttactgtgcttgataatgggattactgtggcttttttggtagcaggaagcagagagaaagagtgggaaagaaaagagtaagaagaaaggctttgggaagctaargcgtggagagagcagttcatttcttcccatcttcagagagcctagtagtattgaaaagattttggcagaagctgagagagatcataatcttgttttcaggcctcctactcctcctgatcaatcaaatccaccctcagcctctcctccacc

SEQ ID NO: 16 - DNA, 401 bp, Brassica napus
  misc_feature (209)..(209): n is a, c, g, or t
  misc_feature (235)..(235): n is a, c, g, or t
  misc_feature (321)..(321): n is a, c, g, or t
  misc_feature (345)..(345): n is a, c, g, or t
ctacttgtatttcaattcacattcattgttttgctaaaaacagacaaaggcttttgatatacacctacttttcggcaatgaatacagttgcttgtgaccagtcaaagcgatgagtcaaagcaatgaacaatctggccacacagacggggtgaatatctgtttctattcacatatgggaatggaacaagagaagaatcaackagaagtancagagaaagtcatgagtttttcaagnttaaagaagtgaaaaccttggctttatgaataactttaacagcaacttcttcttgacccttcaggctgccttttttacccttggcngagcaagtgtcctcgacccacctngccgtccatctcatactccttgtcttcaggaatagagacctcgttgggagcctaaa

SEQ ID NO: 17 - DNA, 401 bp, Brassica napus
  misc_feature (29)..(29): n is a, c, g, or t
  misc_feature (39)..(39): n is a, c, g, or t
  misc_feature (119)..(119): n is a, c, g, or t
  misc_feature (137)..(137): n is a, c, g, or t
  misc_feature (220)..(220): n is a, c, g, or t
aatagctatactaccagtctctgactacnacaacaaatnacaattttactcaaaaaggaccatttcttcacctattaacaacaaatgactagtagaaaaatggattgataacaaaggcnaatactgaaacaaacaanattcgtttgaaaaaagcaatcgaatttcagatgttgatcaacaactagcaaatcaaaagtgacmaagttttaaacttgtaatnataagttcgtcaaagaacactttattccaccattatcaacaaaaccaaaagacactgcttcaaagttccaaagcatcaaacatctgatcctctcaatcggaagaatctccggcgagcctctccgcctcgagccgctccagggccttctgatgagcccaagtctcgatcgagagatcaggct

SEQ ID NO: 18 - DNA, 401 bp, Brassica napus
  misc_feature (26)..(26): n is a, c, g, or t
  misc_feature (115)..(115): n is a, c, g, or t
  misc_feature (161)..(161): n is a, c, g, or t
  misc_feature (314)..(314): n is a, c, g, or t
acacgagaagcgctcttcaccgaggngatgatgccctttacaggttaatgggctttctcttgttttttgcttaatgggctttctcttgttttttgcttaatgggctttctcttgntaactctttaactaactgtgaacagtgttgtttgttcttgttgtgntagcaagaaacaagaatgtaaaggagaagaagaagagcastcgaggagttactggcgaccaattggttgggacaggctctctgagcttgttcagacagtgaaggttgatggtgagtggtcagtgcagaacgttgatgtagatcatgaggatgntgatacaacggttgctgagctggctgctccttactgggaccgaccactcgcgggtcccacgtggtggtgccacgtggatgctagcca

SEQ ID NO: 19 - DNA, 401 bp, Brassica napus
  misc_feature (28)..(28): n is a, c, g, or t
  misc_feature (213)..(213): n is a, c, g, or t
atcaggagaacaataagaaacttgtttnaaaggcaaaacaaaatgataaaagccgtttttgctaactcttatggtaatgcaattagaacaatgataataaaaaggttccatctaaggcctaacaacatactttgaatatgttcctctagaaatatgataacatgttgtatagaagtaacagatcattctaactcattgccrccaagtttaacncaatgaactaaacactaatatatataaggggcggtgtagattacctctgagctgaggaagttatgaagcacaataattcgaggggaccaactaactacttcaggcttgacctgcactaaaccaaatcaacattaagaacagaccttgaatttacagaatggatatgataagacttacatagccaagcc

SEQ ID NO: 20 - DNA, 401 bp, Brassica napus
  misc_feature (28)..(28): n is a, c, g, or t
  misc_feature (153)..(153): n is a, c, g, or t
taaactgaaacccatattaacgacagangaatatacgtaacatgtggtgtttacttagttttattttatttaacaattcttttgtcttgtagggttctgattgtagtttcgttttgaagcaagcataatattgtattcatatttttgttatanaagtatttcatgtttctgtcgtgaaaaaataattttctatatttccawtttttttggtaatgtgaaatttattgattagtaaaagatagttcattacaataaaatggtactataaatgataaaagaaaatatgataagcgaataaattttgaatatcgaagtcgctataatactttaaaatgaatatagccagtaagtacggaatccttctttgttatatagcgacttgtataatcgttttattcctt

SEQ ID NO: 21 - DNA, 401 bp, Brassica napus
  misc_feature (58)..(58): n is a, c, g, or t
  misc_feature (128)..(128): n is a, c, g, or t
  misc_feature (175)..(175): n is a, c, g, or t
  misc_feature (222)..(222): n is a, c, g, or t
  misc_feature (257)..(257): n is a, c, g, or t
  misc_feature (259)..(259): n is a, c, g, or t
  misc_feature (397)..(397): n is a, c, g, or t
acggattcaccttctccctctctctctgtatattcttcgcatcttctcaagaagctcnagcttgaggagagagagagagagagagctttagattcttgagtgtctgtaaaattagatctcattgaganagagagagtatccaattctacaaggttttgggcttgtgaatgcactngttgagctgatcttacaggtccattraggttagtttgatcgatctgntctctgttttcttcaccggagctgataaaaatgtnanctttacaatgtggccatgcttgattctgctcccaagtttacatttttatcttatgggttttgagatctatcacggctactgagatctgatggctctcgtgacttgtcattttgaatgcttatgttgttttcattgtgnagcg

SEQ ID NO: 22 - DNA, 401 bp, Brassica napus
  misc_feature (26)..(26): n is a, c, g, or t
  misc_feature (55)..(55): n is a, c, g, or t
  misc_feature (104)..(104): n is a, c, g, or t
  misc_feature (108)..(108): n is a, c, g, or t
  misc_feature (112)..(112): n is a, c, g, or t
  misc_feature (149)..(149): n is a, c, g, or t
  misc_feature (151)..(151): n is a, c, g, or t
  misc_feature (160)..(160): n is a, c, g, or t
  misc_feature (246)..(247): n is a, c, g, or t
gacaaaaaagagacccaacaactcangtgtttctttttctgcttcttcggctcancaaatcagcaccacatttcacactagtcttcacgacattcatgttctcnttgntccntcatttccatcactatcatttatccatttaccacaancntactattcntttatcattttaaagtttacttttatacatcacgagattartactaaaattataactatatactagttttttaaagatttttatanntatatatcattttgtttcaacagaaattaaaagaaactagttgaggaaaaaatgaaacaatggctaacataacatcaaaaaacttattaatattttctgtaatcagaaaactttagaccaaacctcaaacttatttatgagaacatatattcac

SEQ ID NO: 23 - DNA, 401 bp, Brassica napus
  misc_feature (2)..(2): n is a, c, g, or t
  misc_feature (36)..(36): n is a, c, g, or t
  misc_feature (135)..(135): n is a, c, g, or t
  misc_feature (138)..(138): n is a, c, g, or t
  misc_feature (148)..(148): n is a, c, g, or t
  misc_feature (166)..(166): n is a, c, g, or t
  misc_feature (219)..(219): n is a, c, g, or t
  misc_feature (358)..(358): n is a, c, g, or t
  misc_feature (360)..(360): n is a, c, g, or t
gngatgtgtttcatcagaatgatttatggtttcttntagaggcatatatttgtgagatgagggatgtggagagttacagggcctcataatttgatggtttattgaagagcatagaaactccatcagaagcattangcnggaggagttngagagacaaacaaattcngctatgagataattcaaggtgattaagtgatattrgataatattagaattagnggtgggccaaaaaacccaaaaacttttggaaatgggctggcttttttatggatccggatggttcaaggtccatcagcttaatatacgctatgacgtggctaaataatagacttagaatatttcaggtgatgtggcatcnanataaaaccagagatttactttcttttatatagttaaatgat

SEQ ID NO: 24 - DNA, 401 bp, Brassica napus
  misc_feature (7)..(7): n is a, c, g, or t
  misc_feature (48)..(48): n is a, c, g, or t
  misc_feature (160)..(161): n is a, c, g, or t
  misc_feature (204)..(204): n is a, c, g, or t
  misc_feature (209)..(209): n is a, c, g, or t
tagtgtngatataaagccctaatttacggcagctaccgaataaatttnctccggccggtggggtgttcgagagcagatcatcagcttctctagtctccggtaagttaattttttttaattcttatatctcgtaggtttttttttttttgtaatttgatcnntttaattagcttcgaatcgatcagaatctaaacggttatkagnaattntgtttaaattgtgcttttaatatttcaaattgattaagtgcaaagtcaattttgatcagatctcactttctggtagaggagaagaagaagaagaagttttttttcagtgcttgaggaggatctgccatatccatcagaggttttcaaacaatggtaaattttgatccttagctatatgaatactctatataa

SEQ ID NO: 25 - DNA, 401 bp, Brassica napus
  misc_feature (80)..(80): n is a, c, g, or t
  misc_feature (207)..(207): n is a, c, g, or t
ttttcgaaaaaaaaaataaaaaaaaaaatggatggcattttcgtaaattatatgaacttgtggggtgaatagggcaaaancaattttcaaaaaaaaaggaggttagttttgtgtttgactttaagttataggtcaattttgcaaaaatcccattttttatacatgccaaaaccaatatagaaaaaaacaaaacactcttcrtatacnagacaagcactataaatacattccataaccgttaaagcttccaacaccaccaccaccaccactacagcactactccactctctctccctctttaattatctctgaacaagtgtaagttagcgacatacaatggcttcacttcttttcctcttcgtcttcttcttctccatctcctcttgctttgctcattccta

SEQ ID NO: 26 - DNA, 201 bp, Brassica napus
  misc_feature (24)..(24): n is a, c, g, or t
  misc_feature (152)..(152): n is a, c, g, or t
atgttcattgtagttaattagtanagaactatcggggcagaaaaaaataagtcaacgcgttgcccgaaaaattgtatacgaatgtacctgatttaaagaargaaaattccataaaaatacttcaactaaatttttcttaagctttttaagantcatttttccgctatccactttagtacttcaactaattattttgcccag

SEQ ID NO: 27 - DNA, 401 bp, Brassica napus
  misc_feature (116)..(116): n is a, c, g, or t
  misc_feature (218)..(218): n is a, c, g, or t
  misc_feature (221)..(221): n is a, c, g, or t
  misc_feature (289)..(289): n is a, c, g, or t
ttgtatgaactggttttaattaagtaatgcaagtagttggttgacaaaaaaaaagtactacaccgtggatcttcaatcgcctgatcagcataattagtatattcaatcatatgcanaattaatctaggaactaattgataaactaattcttttacagtgtagctaaagcttttattttcttctggatacagataagaatamatactatatggggacanatncttttgtcgatttttctattcagctttgcaatgaagtctgagcaaagatatgaccagactgaaaaggnaattaaaggatgataacatggaaaaaattaaaaacaaaattcatgcatctgctagtgaggttatttggattcattgcatgtatgttgatgattcgttttcctttcacctccc

SEQ ID NO: 28 - DNA, 401 bp, Brassica napus
  misc_feature (29)..(29): n is a, c, g, or t
  misc_feature (75)..(75): n is a, c, g, or t
  misc_feature (79)..(79): n is a, c, g, or t
  misc_feature (223)..(223): n is a, c, g, or t
  misc_feature (229)..(229): n is a, c, g, or t
  misc_feature (301)..(301): n is a, c, g, or t
  misc_feature (305)..(305): n is a, c, g, or t
aatttttacactttggccagagatataangaaaggttgtaaactcatagacttaagagattttttggtttagtcngtangtgattttgtagaaataatagcgcatattgataaatatgcaacacttgctttagcctttgtttgtgaattgtggtgacataagtccatccctacaagtcatgtatttgtaacgacttgaaartaaaatattttcggaagacatntcgatntataatctgcatttcagtccggactccgaatatccatatatatgatctaaattgggtttctgaaataaaaanaaancacaacttacgtcaagtcaacggaggttaaatccaccctgtcgctcttgtttgctcctttggcaaaacaaaagtcaactactattttaggtgcttg

SEQ ID NO: 29 - DNA, 401 bp, Brassica napus
  misc_feature (164)..(164): n is a, c, g, or t
  misc_feature (172)..(173): n is a, c, g, or t
  misc_feature (255)..(255): n is a, c, g, or t
  misc_feature (302)..(302): n is a, c, g, or t
  misc_feature (396)..(396): n is a, c, g, or t
ttgaattggtctgaaagtttgttagctgttactttgaatagatgcctcggagaccatcaggaggaagaaggttcataaagcaccaacctttagcattttcaccgtttatgcggtcacttgctttagcttcaaggcgtaaactgcatcgtcatcaacaagaagangactctcnncgttctgaagagctgatgtcttttggtkagtagtagtagtaatcattaaaactgagaagtttctgttcagaaacattgtaanaacgaatcattcttgttttgttagatcaaaagctcccaactttgtcnaaaaaggagcaaaaagaacagctttctgactcctctgatgaagaagactctcaggtaataagattattcagactcctctgttttgatccttgantctct

SEQ ID NO: 30 - DNA, 401 bp, Brassica napus
  misc_feature (21)..(21): n is a, c, g, or t
  misc_feature (38)..(38): n is a, c, g, or t
  misc_feature (66)..(66): n is a, c, g, or t
  misc_feature (89)..(89): n is a, c, g, or t
  misc_feature (331)..(331): n is a, c, g, or t
  misc_feature (337)..(337): n is a, c, g, or t
aagtgtaaaagttataaaacngagacgttgtgtttggncatgtcatgtaattgttgaatgttgtgnatatgacacagacggtgatgaantcaacaaggagacagctggagagagagctgatgctggaagacataatgcatcttgaagacttgccttcctacgccctcctctctcaatagccttttaagagttttctaaccwcaacactcccgcttttaataacacaaaaggttgctcgctgctgcctcttctttgatctttttcttctactgtttgttggttggctatatgaaaaacagctctaaaactgagttgttgttgttatattaanacaagnaagagggagatagagaaggaggttgtgggataaaatctcaatttggttgtgggtttggaaagtg

SEQ ID NO: 31 - DNA, 401 bp, Brassica napus
  misc_feature (5)..(5): n is a, c, g, or t
  misc_feature (47)..(47): n is a, c, g, or t
  misc_feature (87)..(87): n is a, c, g, or t
  misc_feature (109)..(109): n is a, c, g, or t
  misc_feature (214)..(214): n is a, c, g, or t
  misc_feature (237)..(237): n is a, c, g, or t
  misc_feature (289)..(289): n is a, c, g, or t
tattngaaataatattgagggctgtgacgaaggatgcacgagaaatntcaacagcttcttctctatcactgcattcactcacgaagntgattagttcttgcaccttctncatccgtagagcttgggtggcctcgatacgctgtggtgagaacagatgagtaactgatattttcctcaacagcctgaaaaatataacataaytatttttttaatnaaatacacaaatctattggttcngttaaggtaactatatgttatgtatacagcagttatatatccgggacagtcntctagtataatgaggataatattttggtaatgaccgggatagctcagttggtagagcagatgacaaataaaaagactaccaataggaaaaaaaaacttagcaacggttacct

SEQ ID NO: 32 - DNA, 401 bp, Brassica napus
  misc_feature (85)..(85): n is a, c, g, or t
  misc_feature (243)..(243): n is a, c, g, or t
  misc_feature (259)..(259): n is a, c, g, or t
ggcaacatatatcacagtataaggaagtcaatacaaaaacattataacatttccaaatattgaaagatttctttctcataatacnaatgcactgaatcaaaataaaaaatcaataattttccaaaaacaaaatctaataattctaaggatgatattaactagaaaatattaatcctccattgttgcgtatgacaagctcgyacgttttagccaatctctcacgaacgataccggcgcgtttcntacactcgctcttctntcctcctcccttatattacttaccctcgaactacttcgtatcaacctttaacctttagacaaactcactcgtcacacattctactcatccttgaccttgtgttgtgtgttatatatacactactacacacgcttattatata

SEQ ID NO: 33 - DNA, 401 bp, Brassica napus
  misc_feature (31)..(31): n is a, c, g, or t
  misc_feature (100)..(100): n is a, c, g, or t
  misc_feature (211)..(211): n is a, c, g, or t
  misc_feature (256)..(256): n is a, c, g, or t
  misc_feature (367)..(367): n is a, c, g, or t
  misc_feature (370)..(370): n is a, c, g, or t
  misc_feature (391)..(391): n is a, c, g, or t
ctgctgctgttgctgttgcacggatgaagangaagaagtcggagacgcagcggatgatgtggagttggtccgacccgccggacccatgcccggattccgngcggggcctccgccactgcctccagattgcattcaattcttcgatcaatcaaacctaattcaaatgcacaataagacaaaaattcaaaacaagaaaaaatraagctggganttagcaataaacgtttgaaaacggaaatttacaaagccacacacncactcactcactctctgccactttccttcacttgatttgaatcgattttctgagggagggagggagagagaaacgaaagtcgcgggatgcaacggaataaaccagatcctntgngggtggcttctcgagaaacgnaatccacgga

SEQ ID NO: 34 - DNA, 401 bp, Brassica napus
  misc_feature (115)..(115): n is a, c, g, or t
  misc_feature (144)..(144): n is a, c, g, or t
  misc_feature (227)..(227): n is a, c, g, or t
  misc_feature (286)..(286): n is a, c, g, or t
  misc_feature (376)..(376): n is a, c, g, or t
gtatccttccggctatcaattcccacctatgaaccacataccatagattctaaatcgtcaaatactatattttatgtaaatagctttttaaaataatttaacttaaacaatctgntgaataaataactttcaagtaaaatcaanaaatagaagattagcatggccgttgcgcaaggattacacgcacaaattcgagaaatrgtccaattttttttccagtcaaaaangtaaaatcaagaacaaactggatcagcgagatcaggctgaacatagtcattgacagctnggttccaataataagcaataaaatacataaaaacgaccgacttatgagataaatcaaaagccatagtatattcttttaaaaaaatcagantaaactaaagatggaaacagacaaa

SEQ ID NO: 35 - DNA, 401 bp, Brassica napus
  misc_feature (74)..(74): n is a, c, g, or t
  misc_feature (104)..(104): n is a, c, g, or t
  misc_feature (116)..(116): n is a, c, g, or t
  misc_feature (155)..(155): n is a, c, g, or t
  misc_feature (272)..(272): n is a, c, g, or t
  misc_feature (317)..(317): n is a, c, g, or t
tgagtatcatctttgcctttgttgtaccttttctgaggatttagaacgagattggattgaggattagtcctctntatcctaagaaatacatgcaatttagtgtnttccttactaanatctgattttcacaaatggattgctgcttctcatgactnatcttgaatctcaagacttggttcattttatttaatggacctttgmaacgttgttgttttgttaacacagtggttcgtttacaagaacatgatcttcaaaccagacaggtcaagcantctcccctcaattacataatttggtttcgtctagtgttttctttnagaaatatgaaactcatatttttctatcgtaacgtgtttcagggaggtgctgtttcagaaggtcaaggatacatacagagacat

SEQ ID NO: 36 - DNA, 401 bp, Brassica napus
  misc_feature (8)..(8): n is a, c, g, or t
  misc_feature (158)..(158): n is a, c, g, or t
  misc_feature (241)..(241): n is a, c, g, or t
  misc_feature (354)..(354): n is a, c, g, or t
ttattatngtttttatttattttttgccggccaatcatatcaattagaccaagttctaatttgtcacaaagagttgttccgaataaaatatttgtctgaccatgtctgatctagatggaaaaatacaatgcctctagtccttccatatggtttacaangagttagattaaaacttcccattatcattgtgcaatttccgastgaggaaataacaaattgtatctggagaagcaagaaaggnggtacaaaatcttagcttatcaaaatgttcacttgtctttggtctattgggagtgtcactttttgtcttagttgaagcccatagaaaagcccaaattattagtcggtatctgncccattttttaaaatttgtgaaccggtgtctgtcttcttcgcttgct

SEQ ID NO: 37 - DNA, 401 bp, Brassica napus
  misc_feature (336)..(336): n is a, c, g, or t
tccgagtcaactcaatccgactcgagatccaccaccagtgtgccacggactctcatcggagggctgttgcttgtcgagattggacctgaagcatcgagacagggctttggtggtctcgtttaacgaagaagaaggagcgatgaacttgttggaagaataacacagggaaccgcttaaggtttgatcctcagttcgctcgtstcctaagatgatgaggatcggaaggggatgatttaaagagttcgtataattattcatctgatgggagcgttaatatatatagattttgaatttcaaatgaaacaaaaatattaccgttattcactcaagtcggtnaaaaaaaagtaacttgtgcatcaagcaagtaacttttgtgggctggcctctctgtttctgatgtg

SEQ ID NO: 38 - DNA, 151 bp, Brassica napus
  misc_feature (65)..(65): n is a, c, g, or t
cttgttgcgaagcttctcttattggttcttccatcgtctctcctgaatcagagttttgatattcnaagtctcccasctatcaaaacgatcagagaactttctttcgaatagattaaaacgatgatatctaaaatcgaaacactgaattgca

SEQ ID NO: 39 - DNA, 801 bp, Brassica napus
  misc_feature (468)..(468): n is a, c, g, or t
  misc_feature (548)..(548): n is a, c, g, or t
  misc_feature (644)..(743): n is a, c, g, or t
tccttcttctctccttctgatattttggctttttcttagaatcttccttttttattttcaccaaaaaaaagaaaaatcaaaaagtattaatcatttaccggtatcagttacacctacactttgcgccgctgaacaaatcaataaggataataagaagaagctcgtttgcttccattttcagacattctttgcctagagcaaaaaaacaaaacaaaaagattgagacttgatcttagcaaaatgggtaattgtttggattcatcagctaaagtggatagtagcagccgccatgctaactctggttcgtctcctcctctccttgctttctcttcctttacccagtttcgttgcttccttaagacttaaagacctctccttactctccaattccaagccaaagwcttaacctttaagctgtttggatcttcaaagatcaatccttttcaattaccagctgtctgatttcanagattgtagatatctctttggtactcaatgttggatcaagttgatttaagatggttgatatgcttaacgttgagattaantttatgagccaaagctaaaagtcttaacctttttaagcttctgttttgtctgtgatcttcaaagatcaatccttttgaattacccatctctgcagnnnnnnnnnnnnnnnnnnnnnnnnnnnnnnnnnnnnnnnnnnnnnnnnnnnnnnnnnnnnnnnnnnnnnnnnnnnnnnnnnnnnnnnnnnnnnnnnnnnntctataagaacagcgaggagaaattaaacaaaacaacatcacttcatatttacagtgt

SEQ ID NO: 40 - DNA, 151 bp, Brassica napus
  misc_feature (3)..(3): n is a, c, g, or t
  misc_feature (9)..(9): n is a, c, g, or t
  misc_feature (54)..(54): n is a, c, g, or t
acntcgganttgtccttctcctcggatgcaggctcgtctccgttggtggtggtngtggtttcaccgagacaggtckcctccacgtggacggagacttcttcctctgttttgaaagggttgccgcagatcggacactcgaacatgttcagag

SEQ ID NO: 41 - DNA, 401 bp, Brassica napus
  misc_feature (33)..(33): n is a, c, g, or t
  misc_feature (36)..(36): n is a, c, g, or t
  misc_feature (60)..(60): n is a, c, g, or t
  misc_feature (75)..(75): n is a, c, g, or t
  misc_feature (88)..(88): n is a, c, g, or t
  misc_feature (90)..(90): n is a, c, g, or t
  misc_feature (92)..(92): n is a, c, g, or t
  misc_feature (128)..(128): n is a, c, g, or t
  misc_feature (153)..(153): n is a, c, g, or t
  misc_feature (181)..(181): n is a, c, g, or t
  misc_feature (214)..(214): n is a, c, g, or t
  misc_feature (226)..(226): n is a, c, g, or t
  misc_feature (258)..(258): n is a, c, g, or t
  misc_feature (280)..(280): n is a, c, g, or t
  misc_feature (289)..(290): n is a, c, g, or t
  misc_feature (301)..(302): n is a, c, g, or t
  misc_feature (332)..(332): n is a, c, g, or t
  misc_feature (338)..(339): n is a, c, g, or t
  misc_feature (343)..(344): n is a, c, g, or t
gtccggtgtttctcctgtgctaagaaactccantanagaccaaaccgttttatggaccanggtggttgttgaacnaccattgagttcntntntaaccgacgataatctatggttcactttgaaatccncaggaaagttgaatttgattcgccntgtggttgacgcaaaccctttgatcaanaaggtaacttgatcatcacraaactcgactggncatagtgaaacnttttaagttaggggttgttgttgaggaatganttttctttctttctttctcagntaattgtgnngggatgcacgnngttagttccagaaggaatcattgcatgtgntgaaannttgnngaagaacaatcataagttggagacacttcacatcaatggcgtccctggcttcactaa

SEQ ID NO: 42 - DNA, 801 bp, Brassica napus
  misc_feature (1)..(38): n is a, c, g, or t
  misc_feature (152)..(152): n is a, c, g, or t
  misc_feature (747)..(801): n is a, c, g, or t
nnnnnnnnnnnnnnnnnnnnnnnnnnnnnnnnnnnnnntctgtagtagctgctgggtgatggtcctgaaacgttcttggcctgctgtgtcccactgtatacacggtcattgccacgagttatagtagtatacacgcttgccaagttttaaangaatatatgttatcaagaacacttacaatctggagtttgattgtctttccgtcttgttcaactgtgcggattttctgaatcacatctaacattagccaacactaatatttttttgttttccgagtactaacaagtgatgggaagagtaaacttacaaagtcaacaccaatggtactgatgtagctatccaggtaagaatcatcctgtacacacaaattcaagacatcaaactataagcacacaaagagmaacaacgatactatactgtaacctgagaactaaacaagtattaaacttcaaagacccatagatttgttactcgtgttcaatgttaaaacgcaattaccgaagataatacactcatagtaacaatgatagcatagtgtaaactattttggagagacaagtaattgaacttgaaggacgcacagattgttattaaacggcaattaacacatgcaagtaagaaatctaaaacaattattcagctggagaaagagttacttacagcaaaccttagaagcaagcaagattttccaacaccagagtcaccgataagcaaaagcttgaacaggtagtcactgcaaattaaaannnnnnnnnnnnnnnnnnnnnnnnnnnnnnnnnnnnnnnnnnnnnnnnnnnnnnn

SEQ ID NO: 43 - DNA, 801 bp, Brassica napus
  misc_feature (59)..(59): n is a, c, g, or t
  misc_feature (90)..(90): n is a, c, g, or t
  misc_feature (197)..(197): n is a, c, g, or t
  misc_feature (247)..(247): n is a, c, g, or t
  misc_feature (312)..(312): n is a, c, g, or t
  misc_feature (528)..(528): n is a, c, g, or t
  misc_feature (559)..(559): n is a, c, g, or t
  misc_feature (594)..(594): n is a, c, g, or t
  misc_feature (678)..(678): n is a, c, g, or t
tttcccataccgtgtaagaatatggacaatcaaagaacaagtgatctcgagtctcatcnctttctccacacagtccacagctttgtgtgnttccccaagccctatgtctcctgtagcaagcctgttgagcactgctagccacgtaatgaatgaatacctaggaatgctttgcgtgaaccaaaccaccttactccaancaacctttgctttcttgggtctaatctggttccaagtgttagccgttggnaacatatccctgaaaccatcctccttatgcctccaaagtatcagatcagtccccctactagtatntggaagtggctccgcgagaatttgagtgtttaaactctgaaaccttctgctgcgcttgtttctaagactccaaccgtcccctgaaaccrcattgctcactagtgcactcctaggaagacccaaataggtcgtaccgatggctccagtaacatcaatcaatcttccactgcccatccaattatcgaaccaaaaatatgtggtttctccatttcgaanctctactttcatgaactcataagccaaatcncttagctttagtagcttcctccaaatccatgaacntttggaatcatctctcacgtcccaaaaagagctttgtctgagtagatagtgctttattcacttcagttgagaattgtcaactanttgaaagttaaaaatgtgaagccagaaatgatacatgttaacagctgaagaaattaatatataaccaaaaaaaaaattcattctataaggaaacttttaaaaaaattatacataccaaagttc

SEQ ID NO: 44 - DNA, 496 bp, Brassica napus
  misc_feature (204)..(204): n is a, c, g, or t
  misc_feature (328)..(328): n is a, c, g, or t
  misc_feature (330)..(330): n is a, c, g, or t
  misc_feature (387)..(387): n is a, c, g, or t
  misc_feature (403)..(403): n is a, c, g, or t
  misc_feature (447)..(447): n is a, c, g, or t
  misc_feature (480)..(480): n is a, c, g, or t
tgacctctcattactgttacatcccgataaacatagacaccatttttgacttcaccggctccaatcagagtcctcgtaaaatgctcctgcaaaatacacaaagtgtctgtgaatactgtcaagcagccagtttttcgaagcaatttcgctacagacaatagagtacaattcagattaggaacaaatagaacatttgccaacaanaaactcgcagacaatctcaaactgccactcttggtagccatcacgtkactaccgtctgcaaagctcacatgacaggaatgatactacgtacatcaaccagtaatagaacatcccccttcctgtnangtgatatctggtgtctataataacctcaccagtttgtaccgtaccgtttaaccgatnaggagttggagaaggnttttgacgctccagcagtgatgtcaaggacgcccattgctctanagtgaactgtggcatagaattcccttggtttgnagacgaacttccagtc

SEQ ID NO: 45 - DNA, 801 bp, Brassica napus
  misc_feature (34)..(133): n is a, c, g, or t
  misc_feature (297)..(297): n is a, c, g, or t
  misc_feature (324)..(324): n is a, c, g, or t
  misc_feature (459)..(459): n is a, c, g, or t
  misc_feature (477)..(477): n is a, c, g, or t
  misc_feature (492)..(492): n is a, c, g, or t
  misc_feature (569)..(569): n is a, c, g, or t
  misc_feature (572)..(572): n is a, c, g, or t
  misc_feature (589)..(589): n is a, c, g, or t
  misc_feature (634)..(634): n is a, c, g, or t
  misc_feature (735)..(735): n is a, c, g, or t
  misc_feature (778)..(778): n is a, c, g, or t
tgaccgatgtctaaaacggttcgggggtgttacnnnnnnnnnnnnnnnnnnnnnnnnnnnnnnnnnnnnnnnnnnnnnnnnnnnnnnnnnnnnnnnnnnnnnnnnnnnnnnnnnnnnnnnnnnnnnnnnnnnnattttacatagaaaactaaaaacgtcatataatttggaacatacaaatttctctaaaacgacttatataagaaaacggtgggagtatatattttcatatattaattaatacaaattaacaataatggactcttaaacctaaagtaaaagtgtaaaagaaattanggatcttgtgcatttgcactcttggcncatggccagagccgatgctgcttgtaatgcttctggccattcacagttaatacgttttctatgcccgcattcactcsgttcaattcgttggttcaacattgtaagatagttggtgctttaattttcaaaagtttngaatacttttttactaantgacataaaggatanaatacatttggaagagtcaaataattttcttgaagaaaatctcaacatatatcagaaattgagatattgtaacttanttngcctaaaatgcaaaaantgtcgtacaactgatggttataagaaatttaagttttcaagttgntgaattcagtaagcacttctggaatctaaccggtaagattgttgtcagggagagtggtaaagagatttaaaatataaacatcagttaggaattttccactnaacggaaatcaagaattaacgaaaatataaccggtaattgtgnacgtatcatcactgcccatctac

SEQ ID NO: 46 - DNA, 801 bp, Brassica napus
  misc_feature (152)..(152): n is a, c, g, or t
  misc_feature (598)..(598): n is a, c, g, or t
ttggttagatcgtaattttatgtataagaggtccacacagaatagaagagactgtttgagatttttttgtatgcttagaagactaaaagagattaaatcctgatttggcctagattttttttttaactcacaaaaggttcattaactaaacnaacacaaatccattacttcttacacaaaagaacagacccactagtttttagaccatcaaactaatctattaaaattcacaaatcatcaattatcaagttgaacctcccaaaaagcatttccttcttccatctcttctcaaataaatgttttgtatgtataggtaccttccacaaaccaagtttgacacaagccatgcaacatggaagcctatctggaagtttgagcttgctcattgaagttgagctaasaatatagtttttcatttgtttcatagatctatgacggtgacatcttgttgagaacattttgacatttgtcactataactagtgtaagagcaggagtctcatcttttttcttcaaacgatgtacataaattttctttaaaatatatcgaatagaatcagctaaaatagaacaattttcgcacaatcaatatcttttgngtgcatatctgaaggcaactttaggtttatcatataacggataactttcaccacataaatacatgtgattgagaagatacttgggattaacatgtctgagtgcattggtgatgactcttggcaatagatcatattcgttttgtacaagataaacaatgttttgttgtagatcccatttgatgttgatttattagtataaacaa

SEQ ID NO: 47 - DNA, 801 bp, Brassica napus
  misc_feature (27)..(27): n is a, c, g, or t
  misc_feature (41)..(41): n is a, c, g, or t
  misc_feature (420)..(420): n is a, c, g, or t
  misc_feature (638)..(737): n is a, c, g, or t
actgggtaacatcagataaaatttcanttccacttcagttntggttacgttctagttttaggataatttcggataattcacgtgaaaatcagattttttattttttagtttttcaaatcaaatatcaggtaattttgataaatttagatagtccagataaaaaaatatttggataattcaatttttttatagttcatataatattaaatattttggacaaaatattaaaataattcagtttataagaagcattttagactctttggtaattttagaactaaaaattgtttttaattatataaacggaattttagacgaataccgattcagttttttgttcggtttcagtttttcagtttaagaaatatataaaccgcttagatatttgtgcatatcggttyagtttacttttcggttctnggtttatatgctgaggtctaccatgaactatcgaggttcttatcaaatttttgattatcgtcattgccaatatcctctagtcaaaaatcatggatcgtaaatacatgaatgctgattgctagtataagaaagtaaatcattgacttcaatattaacattgactttgaacagtacacaaaatagttacatgactgggatagatatgcactttgcagagnnnnnnnnnnnnnnnnnnnnnnnnnnnnnnnnnnnnnnnnnnnnnnnnnnnnnnnnnnnnnnnnnnnnnnnnnnnnnnnnnnnnnnnnnnnnnnnnnnnngatttaaagttttttttactattgactacccgtgggcttccagttcggtccaatttggttttgg

SEQ ID NO: 48 - DNA, 801 bp, Brassica napus
  misc_feature (27)..(27): n is a, c, g, or t
  misc_feature (309)..(309): n is a, c, g, or t
  misc_feature (327)..(327): n is a, c, g, or t
cgtccagatatccaactactcggcaanctcacctgtaatgggaagaaagaggggtgagtaacatgggagtcactcatcaaggtatgggatgctaaaaacgcaaaccactgaatcagtaaatagaactctcactatgggagtttagctctaacatgaacaaacacgatgtctaaaggatcacacaaaacaaacaatgcgatgataacacatagctattacacacaccctgaattctcctcataaggatataaaatatcaattgcgccggtagtacaaaagtctgtctctgtaccccagcaatgtccgctntgtgtctacatgcaaacncctttgcaccccgcaatctctgctctgtgtcactatgcaaaccactgcaccccgtaatctcttgaacatctgcrtcgctagctcagacgtctctggtccccgcgatctccacatagtacttatatttataactatatatcagttcaatcaacagttgaatcctctagacccctaattctgatttacaatgaatgtacaaactaccaagcaagactcgaacagactcagttcaaacagacagatcatgcttcaaaactaaattaccatagaaagagttctacactagtttgggatttaacggattaacggaatataccctcaccttagccaatagtagaaacggaaatgaatctgacaacaaccaagataacttgattaccaagaaacatagggttcaccttggatcatgcaagcaatgggtttgccaacttcattggagatttaacacgatccaaagcacgattgcataagggc

SEQ ID NO: 49 - DNA, 401 bp, Brassica napus
ttctctgatagtgctgtgtctctcctttgccctccggtgaaagaaaggaattcttaccttcacacatatttcattgattgtcgggcaatcatccgcgtggtggatgattaggttttggtttcttcatcaatgggttttcttggtgcttacggctccaagttgcttttagtttgggtctttcttgtttgggccatttactcygtttgataatttatctttctcaaggcttttttttacgtaagtatagcctttgtttaataaactttcagtgaaaaaaaaattatgatagctcatacaaaattgaaacatggttgccttggcagtattatctatattatcttattgaaagctgggccaactaacgagagagttcgtgaagctctccatgttcaaaaggtatt

SEQ ID NO: 50 - DNA, 401 bp, Brassica napus
gcacccaaatttgataacgatacacaagcagctaatggcttataaacactgctagaggaacttgaaggaaaaaaaatattgatggtgttggatgatgtttggtctggagctgagtcctccttacttgagaatttacccactaacataccgaatctcaagatcttgttgacttctcggtttaactcgcttgatttcggtgamacttttaaattggaacctttgaaaaaggaacatgccaagacccttctcattcaatatgcatcgcgtcctgatcacgcatctgatgccgagtatgaacgtcttttccagaaggtattctctattgagcctttccattggtgatctaacattttgtaaatgttgtgggtataatgtgtgatgtgcctcagtccgaggaactc

SEQ ID NO: 51 - DNA, 496 bp, Brassica napus
  misc_feature (284)..(284): n is a, c, g, or t
ctttgttgccgcgagcgacaggtttattgctatcccatcctcaaaaacctctcctacagctttatcgctatcgattcccaacgttgctatcatgcagaacaaaacaaacgaccacaaaagccatttgggacctccatggaggtaaaactactcggagcggcaaagttgaagctaaaaatgagaaacttaaaaagagttttaaaataaacctttttatatagagtagtcgagatggtttgatttgcttatgytattctctcattaaaattcagatgagtgataangtgtaattaggctttagaatttagatccatctaacttcacagagtcaacgactgcaaaagattgatttgcgagtaagctaaaccctcgtgatatagtcaatcattcaattatactattatcggacgacgggatggtgggtttacgtagaaacgccaaggcaagacgcaaactcacagtttccatgtaattttgcaggaagtcaacggctaca

SEQ ID NO: 52 - DNA, 401 bp, Brassica napus
cgcagatcaagttctagtttcagtctagttgtatacagctttaattcatgtttatagtcctagtttaattgtatctcagttttggtatatgtcgtgagccgctaaacatgtcaagcataacgtacaagattttctctccttaaatctcattccctcttaaaaatgttatattttcgtttaattgtctgctggttttgaccrtcgcaagtcaccctgtgaaaaagcccacgttttttttgttttctttctttcaccttgcgccgtgctggtctcttggccttgtctcctttagcggcatttgtagggttgagtatttcttagcggtggtggttgcgtggtggtccgatggttttggctgaggctatgatctcacgtattggaactgaatggttggatgtggt

SEQ ID NO: 53 - DNA, 801 bp, Brassica napus
  misc_feature (50)..(50): n is a, c, g, or t
  misc_feature (161)..(161): n is a, c, g, or t
  misc_feature (175)..(175): n is a, c, g, or t
  misc_feature (189)..(189): n is a, c, g, or t
  misc_feature (250)..(251): n is a, c, g, or t
  misc_feature (294)..(294): n is a, c, g, or t
  misc_feature (328)..(328): n is a, c, g, or t
  misc_feature (540)..(540): n is a, c, g, or t
  misc_feature (577)..(577): n is a, c, g, or t
ctggtggagtccagggagaagcacaagaggaaatcatgggacaaagtatntgttaataaagagaaaagaggattggggttcaaagatattactgatttcaacacagcgatgattggtaaacagttatggcgtttgatagggaagacgaacactttattttntcgagttttcaaangtcggtattacaanaacgcatcacccttggaactgatttgttcatattctccgtcatatggctggcggagtatcnnatatgctagatctttggtaagcaaaacactaatcaaaaaggtngaatcaggatcatccatatctgtatggaacgatntctggctctcaaccactcgcccgagactagctaataaaaccaacacaactattacccaaacctcaaagtggasactctcattgattctactccatgttctaaaacgcggtcaccgcggccgcaaacgcggcggttaagcgctccacgactcttaagcgtcttgattttgctatactcggctaattatacagaacaattagaaaagttaattnttttgttctttttgagttcaaaatcaattgctatatnatagatctgtgagtttaatgtgtaaacaacaaaaagtaagcacaagatttaaggactatgtattttttaatggcggtcgcagaaggtttacagtaaacgtaaacccttaaaagaggaagacgaagctaaaaattatgattatgcccttcacattaaaaaaagagagcaaaaagcgttgttgctgcgtttcgaacacgagtcccgacagtacttagggaaagccg

SEQ ID NO: 54 - DNA, 801 bp, Brassica napus
  misc_feature (84)..(84): n is a, c, g, or t
  misc_feature (162)..(162): n is a, c, g, or t
  misc_feature (172)..(172): n is a, c, g, or t
  misc_feature (348)..(348): n is a, c, g, or t
  misc_feature (587)..(587): n is a, c, g, or t
  misc_feature (736)..(736): n is a, c, g, or t
tcaattgcttgataaaataattcaaaatacaacagtataaccccgcacgtacgcctccgtagtaccctgtgaacatctttagangcattaactagtactaattactttaaacattatatatacaaaaatacattatcatgaattaatcatatacggccaacncttaacttcnagaaaaaaatagttgtggatatactgccgatgcatgtataggccattagggatccaacacatacatattatgacctttctaaacgttatatatcaaatataagtttgacatcctcacagtttttttttaatttaaccacagtgtctggcgaccgagattaaccgactattctgtgnaatccagaagtacaatgttaaattctggtggccaacaaaaatcgaactgcagrttcaccgtatcagggttattcctcaagtgctactagcctaaggcccgttggttacatcctcacagttaccaacatatttaacatgtttaccaaaaaacacataattataaaaaaaattaaatatcactagatgcatatattcctaaattatgacatctttgcagcaatatattagttttatatttntaatgtttagatgatattctaaatatttttatatcatcaaatattattttaatatgtagtcagtaaagtgacgacaaaaaatgtagtcagtaaagtaaatgatcaaaattaatgaaatagaacgtctccttcgcgttgacgattgcacnagtgaggcttgtgtgttgtgaccaataggcaatagcccatatgaagtggtagattccttggggtg

SEQ ID NO: 55 - DNA, 401 bp, Brassica napus
atcggggagggaaagccagtgggagaagagttcctcagcgataagagggtttgatttaacggacaaaccgggaagctgcaagagctctggatccagtatatgaacttcctctatatccatcttatccctaaactctacctaccgagtcaattttcgaaaactggatgatcgtttaccactgaaaccctaatttaggatatrtcccaccacggaaaattcaaaaggcagctatgaacaatcgaggaggtcaactaagtacgagaggtttgtattatactcgcgagaaaaagagaagaaaaaacgaaacctagattcgaatttctataaacaaagagactatacaacttcttcttcttctacggtacgatatgtgcgatcgaacgaagagagagtcggagaaa

SEQ ID NO: 56 - DNA, 668 bp, Brassica napus
  misc_feature (85)..(85): n is a, c, g, or t
  misc_feature (108)..(108): n is a, c, g, or t
  misc_feature (135)..(135): n is a, c, g, or t
  misc_feature (170)..(170): n is a, c, g, or t
  misc_feature (187)..(187): n is a, c, g, or t
  misc_feature (212)..(213): n is a, c, g, or t
  misc_feature (293)..(293): n is a, c, g, or t
  misc_feature (339)..(339): n is a, c, g, or t
  misc_feature (429)..(429): n is a, c, g, or t
  misc_feature (447)..(447): n is a, c, g, or t
  misc_feature (494)..(494): n is a, c, g, or t
  misc_feature (515)..(515): n is a, c, g, or t
  misc_feature (550)..(550): n is a, c, g, or t
  misc_feature (558)..(558): n is a, c, g, or t
gccaaattaccattcaaactttgacggctatcgctatgcacaagattgggcctaagctagagaaagctcataactaactaatttnccttgccggtgagtatgatgacncctacagagctatcgtctctggcgtcnttaaacgcacgcataagctccttcacagtctgagnccggaacgcgtttcttntctccggacggtttatagtgatctnnataaccaaaaactattcaactgaagaagaaagaaacacacacaccagagagagatcatcgaacactttacattaacaaancttggcaatatcttcaccgacggctttctcatatataatgtcaacnaactctttygtttctccgtcgtcaccgacgagatcagcttttctccaaacgacttggtgagtcggcacttcaccgtgaaccttatggtanttgtcattcatcgacgangcagtagagagttccactgagtgaacgcgagttggaattgtttccanggggatgagatgattggtgangacggagatacggcggctcgcggtgccgagttccntggagtcngccattggagaggaagacgcgagagacagagaaagatgagactgattgatgatgaagatgacaagagattctatcgcatggactttgacaatatttggataaaatatttt

SEQ ID NO: 57 - DNA, 552 bp, Brassica napus
  misc_feature (64)..(64): n is a, c, g, or t
  misc_feature (100)..(100): n is a, c, g, or t
  misc_feature (166)..(166): n is a, c, g, or t
  misc_feature (211)..(212): n is a, c, g, or t
  misc_feature (367)..(367): n is a, c, g, or t
  misc_feature (372)..(372): n is a, c, g, or t
  misc_feature (376)..(376): n is a, c, g, or t
  misc_feature (422)..(423): n is a, c, g, or t
  misc_feature (440)..(440): n is a, c, g, or t
  misc_feature (477)..(477): n is a, c, g, or t
  misc_feature (479)..(479): n is a, c, g, or t
gtatgacagtgatgatgagtttattgctcctcctaggcaaatcaggcagccattcatcaaccgncaacccgcccctgttacgggtgtccctgttgctccnactttggaccaacgcccgagccgcagtgacccttggagtgcacgtatgagggagaagtatggactngacacgtctgagttcacatacaatccctcacagtcacaccggttnncagcaaatgccgacgcaaccaaatgaagaaaaaggacgatgcaccatcatgtgagtccatgtctttaaaaaagttcagtcagttctcstttcctatttttatttctgcttgcgtataacaatcaagagtgtcagtgaaattagaggtgtgtttcngggtngttnttgatgatgattactctagcactggaggtatctcaaatcaacctanncattttgttgaaactcnttttattgtgtctgtgtagtctttttgtaagtacttnancatcatgaatgttcatcttggttatctgattcggtcctatcattcttattatatataaaattcatctgtttta

SEQ ID NO: 58 - DNA, 401 bp, Brassica napus
gagaagaactgtatagaagcttcacttgattccctaaaactgttgttcgaaacaacatagagtagttgaaaatgacgttgaaatacccaaatgaatttggtttgagagcgattagaataaactgtctctggtggtgagatgatctcctttgtggtagagctgaaagatgatgttctcttcattaaagagagaagttatctygtcataccgaaggaccatagtggtaataagcggttggcttctaaaacatagcagtttcgtggagatggagcagagcctaggaccgtgaagtagcttatttggtggtgacggaggatgctggccggaaatatctgctgtgaacctattgaaaacatctagaaaaagggattttgacgctgaagatcagattggatgaacaa

SEQ ID NO: 59 - DNA, 496 bp, Brassica napus
  misc_feature (61)..(61): n is a, c, g, or t
  misc_feature (83)..(83): n is a, c, g, or t
  misc_feature (102)..(102): n is a, c, g, or t
  misc_feature (159)..(159): n is a, c, g, or t
  misc_feature (316)..(316): n is a, c, g, or t
  misc_feature (324)..(324): n is a, c, g, or t
  misc_feature (409)..(409): n is a, c, g, or t
  misc_feature (477)..(477): n is a, c, g, or t
gtaatgaaggcaaaacgaggcgacccttggacgaaccataccactttactccgattctgcntctctctatgcggttgtatctnctcccatgtttggaaagangagaacctgcacttatactcatccgaccctgatttccatagaaccatgtcctcctcnttaccaacaactagtgctttgaaacttctaacactcgtgattatttgctgtagagtttggtctctgcatcttcgaatctgccaaccagaagmatttgcagcatcagcaaccttggtatatcgcccaatatcaagccgttgtggaccactatcccccnctatgtcnataagtcggcccccaggaagccaggggtccgaccaaaatagagttctctgcccatttttaatttgcattctgatgaattgagcanccagcggcctcagcctcaggagcttcctccacacccacgatcccttagctgactccctaatgtcccanaatgaatcattgctccata

SEQ ID NO: 60 - DNA, 801 bp, Brassica napus
  misc_feature (81)..(81): n is a, c, g, or t
  misc_feature (115)..(115): n is a, c, g, or t
  misc_feature (179)..(179): n is a, c, g, or t
  misc_feature (214)..(214): n is a, c, g, or t
  misc_feature (333)..(333): n is a, c, g, or t
  misc_feature (419)..(419): n is a, c, g, or t
  misc_feature (663)..(663): n is a, c, g, or t
agcgttcacccaatgttcaccgtaccactccgttaacgaggagtggttgctatatctcaccggggccgggattgaaccggnaatatactatgccttcaacggatgaactcacaanccgagccaccgtctttacaactcgatcacctagcttctctctcactctacaatacatctgagtnctgatctaacaagatcctaatcagctcagctcatncttatcctagtctaaccgtcacacgtgcgcacacttcacacgtgagatcaactaactcgagagagagagccggttctaattgattacaagcttaaccgactaaaccaactttaatcccnctatacaattagaacctaaaccaatggatagaaacttgactatatccaacaaaagccttagggtgtargttaattatcttgttcancaaaaccttagctttttatttactgctttaatcataatcatctagttttagttcgaaaactacaaatttattgtgtaaatcctaaagtctatgtcgattcgattcttaaatattgcaattgaaacttttaattaaaagaataaaatcactgtttagggcaatttaaatgatatcacacctactctccggtaacaaaaataaatgtaatcataatgttgatggatggcactacaagatctaaaantcaatcaaatagattttaaaacttcctttctatatggtaatcaagcagtagagatttatatgaaaaaatctaaaaggttggttgtcccataacaagaaaagtctacagacttgttaagtcattatacaaactaaaaca

SEQ ID NO: 61 - DNA, 401 bp, Brassica napus
gaggtaaaaaatcagtaactgtcatgttcttcgttagcaacggaagccctaagtatctgacaggtatattaccagaagcaaaagaaaatgattcatgatctcttctttcttttgatctaaaaaaccagccataaacaaggtagacttttccaagctaatcttcagacaagacattctattaaactcctcaaatactttcartatcccttcaactgatcttctagtgccttcaataaacaccattaagtcatctgcaaagcataggtgagtgatacctatgtttttgcattttgggtggaatccaattagatttcttgaggctgcttcatccagcatctttgatagcacattcatgcagataacaaagaagtagggagataaagagaatccttgacgcagac

SEQ ID NO: 62 - DNA, 801 bp, Brassica napus
  misc_feature (68)..(68): n is a, c, g, or t
  misc_feature (132)..(132): n is a, c, g, or t
  misc_feature (184)..(184): n is a, c, g, or t
  misc_feature (218)..(218): n is a, c, g, or t
  misc_feature (248)..(248): n is a, c, g, or t
  misc_feature (258)..(258): n is a, c, g, or t
  misc_feature (322)..(322): n is a, c, g, or t
  misc_feature (637)..(637): n is a, c, g, or t
  misc_feature (660)..(660): n is a, c, g, or t
aaattgatctgatacagttctcaactggcatgcctatgggtaccctgcctgtctgttatcttggtgtnccattgtgtactaaaaagctcacgctcttaaactgtgaaggtttacttcagcagattatcctcntggagtgccaaatcactctctttcgctggcaggctgctgcttatcaaaacantcatcacaggcataaccactttctggtgtacaangttcatccttccgcaagcatgtgtaaaacncataaattcnctatgtggtgtcttcctctggaaaggtgatattgaggagcactacgcagcacgagcctcttggnaggttgtcacaaagccgaagcaagaaggaggccttgggattaagaatctttcgatatggaacaaagcatgctgccttargttgatctggctacttttctttcaggcaggctcggtttgggttgcttggttcaaggaggaagttctggatggatatgtctcaacaatctctggactatggttccacatagacgctactcttggcaggttaataagcttcttaaactgagctcctctatcttcaattgagttaagcttcgtgtccaaaatagtctctcttgtcggttctggagtgacaactggtccccttacggctntatgaggtcttatcttagcatcngctccaactcaactatggggatcgcagcacaagcaactttagcatcccttcatcataacaacaactggtggattcctcctgcaagatcagaagctcttgtcaatgtccatgccctattgaccaccattgaactaaacaata

SEQ ID NO: 63 - DNA, 801 bp, Brassica napus
  misc_feature (255)..(255): n is a, c, g, or t
  misc_feature (412)..(412): n is a, c, g, or t
  misc_feature (460)..(460): n is a, c, g, or t
cttcttagactaaaaatagtaattaaaaattctaagatgtttgctaagagttttcattgataatgttgctcttaggatgatgcacaaaactgtgactgtggcatataatatatcaaagttatctgcagcttcaccacacaacaaaaaatacctataatttctccattcttctacaaggtagcagactagcaatcaataataatacactactaaatctctcttcaagaataatcacgtgcacgaacgattgttctntatcgatatctgcttaacattacatgctctccctgaagttaatagatcttgacatatctgcagggtttgtttgaaggtttagatacgtcttagggacaaatctattgttgcagctctttgtttcaaacccattagaggaaaaactsaattgatgtgncttctcgcgtttcatcggtaccggatacaacacacgattattcgtagntacgtcaatacttcgagattgtgagtccaatcttgctcttacaaaagtgtctttgttttctctaacactttcatgtgttttagcacaaaaaacacttatcatgtaaagcttcgtctcttgtccttttccctagacacgtggaagtctctagagtataccaaaatggtaccatgcagccccagtagacaaggatgtggtagaatgtagggtaaagaggacactggtgagggccgtgaggccatggaggcgaaaaaggggatgttacttgcgaaggaagaaatccttgggagttgttgaaatctttgaaaacagagtcagaagttatcttcactttgcttgat

SEQ ID NO: 64 - DNA, 401 bp, Brassica napus
tgtacactttcccttgcttggccatccatgagttgaagatcagcatggcctcagcgtcgaaaacgctgtcgctgtggctgggaccagtggccacacggtggccagaactgccaacaacatggtggttatagtcgtatgaaacgacggacatgtccatggccgtggcacaagatgcgatgagcattgctagtaagaagatcmgcatggctgatttagcactacccatcaaaactaatgaaactttaatttatgtttgtttcaacaagtttaaaaaagctcatagaaaaagagaacaagattttgtgctgattaattttgcctactatatgagagtatttatagtattcagagctcagataggtaacacttgtgttaagaatctcacatcagaagaggtgata

SEQ ID NO: 65 - DNA, 401 bp, Brassica napus
gcctctgttattccctccggctctctggttggtgttattcctgctactgttcagagctccgcctctgttattccctccggttctccggttggtagtctttcctccggtcctccgattggtattcttcctgctgcaattcagagctctgcctctgtctctccatctggatcaccggttggtgctctcccctctggctctctrgcgggcgttgttcctcctgagacagtgacggtgataagtcctcgctctgctcatgctcctctagcttccatagctccatcacaaaactatgcttctctgttgaagaaatcttctcagttgaaagagctgggaacgccggtggaacacgtctctggtgtaccgtttgtcatgatccctgataaaaacattgagtcagcaaa

SEQ ID NO: 66 - DNA, 151 bp, Brassica napus
  misc_feature (2)..(2): n is a, c, g, or t
  misc_feature (105)..(105): n is a, c, g, or t
  misc_feature (144)..(144): n is a, c, g, or t
cnaacgactcccaaacgatcacactttgttttcaattattcatcgataactatattcatcgactcccaaacaacawaagttaccaccagttcacaacaaaagtanaacataaagatctaccacgcagatggtccaaatagcatncggacaa

SEQ ID NO: 67 - DNA, 801 bp, Brassica napus
  misc_feature (15)..(114): n is a, c, g, or t
  misc_feature (206)..(206): n is a, c, g, or t
  misc_feature (300)..(300): n is a, c, g, or t
  misc_feature (308)..(308): n is a, c, g, or t
  misc_feature (538)..(538): n is a, c, g, or t
  misc_feature (575)..(575): n is a, c, g, or t
  misc_feature (695)..(695): n is a, c, g, or t
gtttgcgaattatannnnnnnnnnnnnnnnnnnnnnnnnnnnnnnnnnnnnnnnnnnnnnnnnnnnnnnnnnnnnnnnnnnnnnnnnnnnnnnnnnnnnnnnnnnnnnnnnnnntgtaaaagaagcttatgtacccgtattttgtggaagcacgcaagggcgaatccaaagattattttcagtgggtgcacaaattaaagtgtatncttacgtatgatcgtaggtgtatacatcaaatttgttaagaaatatactaaaaaatttaaaattattatgggggcaagtgcatccataatcctntacctagnttcgtcagaacatcgtagtctattgattaaggttcaaaagcttatacacttaagtctttgaatttcaaactatgcattttttttgccgattargatgcgaagctcatcagaagttttagagtattgtaagtagagctgtttgttgtggtgatggaaagagtttgtctatcgcggatgtcgtacatgctggaccgtctgtcgatccaaatgtttcggaaagaactttatcngaaaattcttatccatcatcaatattgcatatattgnaggtagttgagcagcacatttaaaaagttaagtagaattttgatcgctgttttacctacagaagctggcgagacactagtgtaagagagattgtattgagtgaacatttgatattgatantggattttccaaaactaaccacctcgtgagtatatgctgcaatcattttgattagacactgaaacaagtaatcttgtatgtcttttcgatttcaacttatgcttat

SEQ ID NO: 68 - DNA, 801 bp, Brassica napus
  misc_feature (1)..(48): n is a, c, g, or t
  misc_feature (106)..(106): n is a, c, g, or t
  misc_feature (693)..(792): n is a, c, g, or t
nnnnnnnnnnnnnnnnnnnnnnnnnnnnnnnnnnnnnnnnnnnnnnnncaatattttaaatttttttagaggaagacacctagtataatttttaattaactaaaanggggattacataattggatcctacgttaccgaagccggactccttccgcctctgtcgatctgcagtcttgccgctcctccaaaacaccgccacgtaaagccattccggtgagagacaaccaggttcaaagtaagatgcatatcgaacagaaaaatcaacgatggagagataggcaaaaagaaaaaagagtaacctccggcaccgcttattgctggaccggaaaaaagatcttttgcgcttgagagcttttaaagagagatagttctgttagagagagggtccactgcatgcaatkatatattctttctcatcagactttgattggtatggtgcttaaatgggctgaaagccttatatagtatttatcgttcatgataatcaattatataagtttcttaacaaataaattaaaataaagattttttgaatgattgaatctgaaaaatatatcgcaaaagcggcagcctagggttagatcaacttctccatggacacgtacactagccagattaggtcctcaaggggccgataaggttcgaaagtgaggctgctcgggaagccttcctcgagaggaacttaaggccccnnnnnnnnnnnnnnnnnnnnnnnnnnnnnnnnnnnnnnnnnnnnnnnnnnnnnnnnnnnnnnnnnnnnnnnnnnnnnnnnnnnnnnnnnnnnnnnnnnnntttggtttg

SEQ ID NO: 69 - DNA, 401 bp, Brassica napus
atcacagagctgcatataacagatacagaaatactagatattggttcatgggtcaaggaactctctcatctaggccgacttgtactctacggatgcaagaacctggtatctctcccacagcttccaggttccctactagaccttgatgcatcaaactgtgagtccctggagagactagatagctcccttcacaacctgaamtctactactttcagattcattaactgcttcaaacttaatcaagaagccatacatctcatcagccagactccatgtcgcctagttgcagttttacccggtggagaagtgcctgcctgctttacttaccgagcttttgggaatttcgtaacagtagagttggatgggaggtctcttcctagatcgaaaaaatttagggcttg

SEQ ID NO: 70 - DNA, 668 bp, Brassica napus
  misc_feature (6)..(6): n is a, c, g, or t
  misc_feature (72)..(72): n is a, c, g, or t
  misc_feature (210)..(210): n is a, c, g, or t
  misc_feature (213)..(213): n is a, c, g, or t
  misc_feature (266)..(267): n is a, c, g, or t
  misc_feature (287)..(288): n is a, c, g, or t
  misc_feature (481)..(481): n is a, c, g, or t
  misc_feature (506)..(506): n is a, c, g, or t
  misc_feature (542)..(542): n is a, c, g, or t
  misc_feature (545)..(545): n is a, c, g, or t
  misc_feature (566)..(566): n is a, c, g, or t
  misc_feature (580)..(580): n is a, c, g, or t
  misc_feature (584)..(584): n is a, c, g, or t
  misc_feature (620)..(620): n is a, c, g, or t
  misc_feature (631)..(631): n is a, c, g, or t
cttganccgccaatagatgagtctcctgaaccgtttccttcatatttccacaggccagtatcttgggatgcnaacttcttgactgcagaaacataatctggcttgaagaaaaacatattatcctttccagcagattggtaatggttccctgtttgttgcatatcatcsccaccaaactgtgcagggcttagggcaggaaaatccatgggngtnagattaggagccggagcaggagcaggaatcttaggcctcatgttctgattcannccattatccacttgtagctnnagtacaaacataaccaaatcactcgaatgaacaaaacattcataaagtagcaaaacaacatgattggagcaaaaaaaaaggacatcaacacattcaataacttaaaaattacaattagcatcaacattgaaccatatgttcacaaggaataatgagtttcataggaagagaagcagaaagctagggagaatanctcaagctgagtaagcatctcaacngtcaactgcaaatcacacccattagcaaaataaacntcngcaagactctcagcagcaaanccagggaactgagnagcnagaaactccacagggttcacctccatttcccctatncttggattctnggaaaccatgaatcgaccaaaagggtttcttctctcc

SEQ ID NO: 71 - DNA, 801 bp, Brassica napus
  misc_feature (207)..(207): n is a, c, g, or t
  misc_feature (267)..(267): n is a, c, g, or t
  misc_feature (317)..(317): n is a, c, g, or t
  misc_feature (351)..(351): n is a, c, g, or t
  misc_feature (543)..(543): n is a, c, g, or t
  misc_feature (670)..(769): n is a, c, g, or t
cttcataaataattgacacaatatatttgaatatatgatatatttaataaaaacctcaatacataaaaataattaatagtattaattttaatatatatatttatattcactctattcattactattaaaatttggatattatataaattaaaaactatgattatatttttattgatatatgatattgtatttttttttaaagaaggnaagcgtgattccaaaacagaatcataagcttccaacatgtttttaaagagaatattttgnaagcgttttggaatcgagattccgtaagcttccacaaggttccgattccngttccaaagcgggaagcagatgtccggatgaagnttccatgcaacgtaggaaacaagtatcaaaaggataagagaaaggaaaakatagagaagttcacacataccaaaacaattcgacctcgaggtttagacctaatcttcggccaggttccttctatcatcctttgttactttccgttagattgtaacccatattctctgtaacctttcagttactaatatatanacatttcttttcgtcaatcttgatatgtatcttgcctagccaacaactggatcgtgagtgttaaacgtcttccgatcatatttattcaatttcgcatcacaattcgctaggcccaatccaaacgacnnnnnnnnnnnnnnnnnnnnnnnnnnnnnnnnnnnnnnnnnnnnnnnnnnnnnnnnnnnnnnnnnnnnnnnnnnnnnnnnnnnnnnnnnnnnnnnnnnnntacgtagccgcttccgtttccatgtaaagtag

SEQ ID NO: 72 - DNA, 151 bp, Brassica napus
  misc_feature (144)..(144): n is a, c, g, or t
  misc_feature (149)..(149): n is a, c, g, or t
gccgccgagcgaagttcccttgccggcgttcttcgcgaagagaagcgtctcctcgttcgaaccagccgacgcaacsaccgatctgatcagaatcttggggatagacgtcgatcgatctcagatctccgattaataagaaaaagntatcnct

SEQ ID NO: 73 - DNA, 401 bp, Brassica napus
ataaaagtttggatacttatataataaagtaattatatacgaataaaagtgaaatatgataaaaatcatgatgaatagttggaaacaaacatgaccttgtctcttttttcctgaacaacacatgaccttgtcctaagaaatgaaaagataattaaataaaacgaaccaacaaacaacataaaaaactaagaaatagccacraatgaaaatatagagggaggaaaatcctagtaataaatgtttggatacttaaataaagtgaaatgtgatatattcatgatgaatggttggaaacaaacatgacattgtcctaagaaaccaaaagataattaactaaaatgaaattaaaaaaactaagaaaaagaccacaaatggaaaaatatagggagagaaactctagt

SEQ ID NO: 74 - DNA, 301 bp, Brassica napus
  misc_feature (42)..(42): n is a, c, g, or t
gggtgacccgggttcgatccccggcaacggcgaatctttttnttacattttaagaaattgaaatgttttcatgaaaatgaacaaaagattataatggcttcgcccgggttcgaaccggagaccttcagtgtgttagactgacgtgataacmaactacaccacggaacctttgtgcttacattgggaacaaagagctttgataattttgatgtctaagaaatctttagatgtttggtccgtagagtcatgtaagctgctctgtctattaagccatctcgactgctctgatcttctgtaaaaa

SEQ ID NO: 75 - DNA, 151 bp, Brassica napus
  misc_feature (11)..(11): n is a, c, g, or t
  misc_feature (19)..(19): n is a, c, g, or t
cctcatgcatngttcaagnggaagatcagagacttcaacaactggttcatctggaatagcatctaccacagacttrtctgtttctttgcatccatcttcactggcgtttacaccaccattctcattattctgagtggtctgagttgagtcc

SEQ ID NO: 76 - DNA, 801 bp, Brassica napus
  misc_feature (41)..(41): n is a, c, g, or t
  misc_feature (68)..(68): n is a, c, g, or t
  misc_feature (336)..(336): n is a, c, g, or t
  misc_feature (421)..(421): n is a, c, g, or t
  misc_feature (745)..(801): n is a, c, g, or t
gctcaaattgctacaacgattgaatagaatttcccgtacanaacactgtagttggccagatacgttgnaggtttaagaagtgtaatgtatcttgtattccttatttatttttccttttttttgctaaaaatatgctttattttttacaattaatttctcttattttttacaattaatttctcttatttccttttacaattaatttctcttatttcccgtacataattatttgttttattttaaatttattatgtttgtattaatttatttcagtagtcagattgaaataacagttaaaatgaataaatttcattacttccgatcatgtattgttangtttagaactacaagcttactgatcatgttagttggcagttttttgtatcttttgagtatgcagrtatgtcaatattttcaaatnatatatttttctaaatatcatattcaatttctcttacaaacaatggctctcattaatctacattaatttattctaaaataataataaccctttgtaaatatcaatcctaacatttagggaggtgtattcaattgggagtttgaagtgatttttattaaaatgataaatctactgttcttaaaacatgattttttattaaaaaaactactttgaaatctagtagtattgaacttgttatttcataaaacactcttaaatgcactattattgaataaatttaagttagaaattttagagtgatttatttctatagtgtttgaggannnnnnnnnnnnnnnnnnnnnnnnnnnnnnnnnnnnnnnnnnnnnnnnnnnnnnnnn

SEQ ID NO: 77 - DNA, 1001 bp, Brassica napus
  misc_feature (28)..(28): n is a, c, g, or t
  misc_feature (41)..(41): n is a, c, g, or t
  misc_feature (55)..(55): n is a, c, g, or t
  misc_feature (64)..(64): n is a, c, g, or t
  misc_feature (81)..(81): n is a, c, g, or t
  misc_feature (160)..(160): n is a, c, g, or t
  misc_feature (189)..(189): n is a, c, g, or t
  misc_feature (204)..(204): n is a, c, g, or t
  misc_feature (252)..(252): n is a, c, g, or t
  misc_feature (306)..(306): n is a, c, g, or t
  misc_feature (324)..(324): n is a, c, g, or t
  misc_feature (405)..(406): n is a, c, g, or t
  misc_feature (450)..(450): n is a, c, g, or t
  misc_feature (475)..(475): n is a, c, g, or t
  misc_feature (559)..(559): n is a, c, g, or t
  misc_feature (582)..(582): n is a, c, g, or t
  misc_feature (604)..(604): n is a, c, g, or t
  misc_feature (617)..(618): n is a, c, g, or t
  misc_feature (701)..(702): n is a, c, g, or t
  misc_feature (753)..(753): n is a, c, g, or t
  misc_feature (924)..(924): n is a, c, g, or t
  misc_feature (931)..(931): n is a, c, g, or t
  misc_feature (966)..(966): n is a, c, g, or t
  misc_feature (970)..(970): n is a, c, g, or t
tctttgactcctgtttgacatctcctangtgcattttgtantgaaagagctggtnagaaagtcnatttcagaaacagaggngagaagacgccttctgttgtgacaattcctctttaactctttacgttctgtttcaaccctaaaatgccatttttttatnaggagctgaagcgattcccaactctagcnagcgatatagcagcngctgcaaatgaagctcttgaaagattcagagacgaaagcaggaaaacngttctgcgtctggtggacatggaatccagctacctcactgttgagttcttcagnaaacttcacatggaaccngagaaagagaaaccaaacccgaggaatgccccacagccaaacgcagacatatactccgacagtcacttcagaaagatcggnncgtctctgcttacctcactatgaatgaatgagacatatcaaatntgtgttgacttttgaatataactcnggatccaacgtgagtgcatacataawcatggtctgcgacacattgagaatctctcttccaaaagctgttgtctactgccaagtnagagaagctaagagatcgctccntaacttcttctacgctcaagtnggcaggaaagagnnaagtaattttctaaactagagaatatctgaatcattttaaagagtgaagaacactttctaatgatcattaaaaaaaatgggtnnagaaggagaagctgggggcgatgttggacgaagacccacagctgatggaangaagaggaacattagccaaacggctcgagctttacaaacaagctagagacgacatcgatgctgtggcttggaagtaaggtgtgatcaaaaagggtttcctaagaaaatattctttatatcttttaattgctttgctcgtgtgggcacttatgttggaagttctaacctccnatccatngctgcacacacatacagacgataactcgtattttntttngccgctaatatttgtttcccacttttttggt

SEQ ID NO: 78 - DNA, 121 bp, Brassica napus
  misc_feature (40)..(40): n is a, c, g, or t
tgatttgcctagaccaatttttagaacactggtaataagngacactgtttgtctttggttrtagttgatacttcagcttaacggttcatgttttaaccatttcctaactattattgattct

SEQ ID NO: 79 - DNA, 151 bp, Brassica napus
  misc_feature (31)..(31): n is a, c, g, or t
  misc_feature (47)..(47): n is a, c, g, or t
  misc_feature (50)..(50): n is a, c, g, or t
  misc_feature (55)..(55): n is a, c, g, or t
agtttccttctcctccgagaaagttagctcntttctcttgttctctntcnaaaanatctctcctttcaacgttaartcgtttagttgtttgagtgatgtctacggatacggaggcgaatttacttgcgttagcggctgtgttccgcaggag

SEQ ID NO: 80 - DNA, 801 bp, Brassica napus
  misc_feature (56)..(155): n is a, c, g, or t
taattaacgtgatatattatttccataattatgcacaaattatttgttaacataannnnnnnnnnnnnnnnnnnnnnnnnnnnnnnnnnnnnnnnnnnnnnnnnnnnnnnnnnnnnnnnnnnnnnnnnnnnnnnnnnnnnnnnnnnnnnnnnnnngaaaaaaggtgtattgcacaattatgttaacaaataatttgtgcataattatggaaatattacatcacgttaagccttttagtcttatgtttagatcaatgttataaaaattggtagacggtggttaagcgtcttgtaaaagattattgtttagttggatatctaggcgccgcttaaacagatttttataacactaatttatatagaaaatatgtaaaactttttccatcatccatttctaacatmgtggaaataaataaacaacttagacaatataaaattacaaatagattattagtttttacaaaaaaagtataaatagattattatggcacccatcatatattgcataggctatattcttctcgccttaagcgtaaaaaagagacaaaatattctttagtgaagatgggaacagagacgtcgacgatgacggcgaagttagcattcttcccaccaaatccgccgacgtacacggtggtgacggatgaatcgacggggaagatcgatgaggatatcggcggacatgattcgtcgtcatagacgaggaaattgaagtggtgaagataatgactagaagagggaatgagatcgtggggttgtatgtaaagaatccaacggctaaactcaccggtgtgtattctca

SEQ ID NO: 81 - DNA, 801 bp, Brassica napus
  misc_feature (1)..(14): n is a, c, g, or t
  misc_feature (280)..(280): n is a, c, g, or t
  misc_feature (353)..(353): n is a, c, g, or t
  misc_feature (359)..(359): n is a, c, g, or t
  misc_feature (364)..(364): n is a, c, g, or t
  misc_feature (624)..(624): n is a, c, g, or t
  misc_feature (641)..(641): n is a, c, g, or t
nnnnnnnnnnnnnnacaacaagctatcgtttttatataataagtctttgcatattcattttaaattctgaaccgtttgtgtttgatctaggttgatacttggtactgcccgagtgatatggacactccacactgaaagaattgtgaaaaaaaattagataataaattatagtttttttttgtaacttagtaaattataatgtttagaagctaaaaacataacacggagttatggacagtcgatactgactgaatcacacttcagacatatccaaatatantttgacttgcattcctatttttaaaaaattaacgttttgatgtgaaaatataagtttcacatcgagatcgaanattcanttganacatgaataatatataaaagatttggatcaatccacrtattaccaatttattttaatttgaaaactcatgataaatccaaacttaacatgatattatagttcgaacacatgctagctgcccaaccgaccgaaattgattaggctcatcgaaagaggttcaattgatcctaaacctcatggcctgaatggtctggcgaactgaccgaaccaaatcctaaattgagatattgtcgaggttaatggttataagaatcactatnttgaagaggcgtgtganaatataaactcacatattggaagtttaagtgggacatgaataatatataaatagttaaagctaatccacttatcatcaattggttttaagttaaaagcctatgataaatccaaatttaacatatttgcttattaatcagtgttttagataaaagtggata

SEQ ID NO: 82 - DNA, 401 bp, Brassica napus
ctagcttcctcaccatgaaatcaatacggtccaatctcgaaaggatgggttcttccactatagccataatgttgataacacaccgttgttctgttgcacacttcacagctttggttgttgccgtggagtagttaaagccttaaagacaagacactatatgaaacgccaaaactggtcatcttggagattgaagacatgaaytacgacacgtttaatattacagagagagctggttacggtcttacgcgtgtcgttgatcacacgtactgggtttagtttgtggacacctcttctgtctcacacgtccaacattattccatccttccttatcttaatcgctgacgcctctccgagattatatcagacgcaagataaaatttctagtgtttattgcaagtgtt

SEQ ID NO: 83 - DNA, 801 bp, Brassica napus
  misc_feature (431)..(431): n is a, c, g, or t
  misc_feature (483)..(483): n is a, c, g, or t
  misc_feature (572)..(572): n is a, c, g, or t
  misc_feature (598)..(598): n is a, c, g, or t
  misc_feature (626)..(626): n is a, c, g, or t
gttaaaactcgtgagtggtaatcttgtaaattgatgaagacttgggttctaagttggctgaaaccaaatggggtttctgcgcgcttcgccgtcgaccgatgacacaggatgtgcatcgatcgattattatctctgaatgtcgaccgatggtcttgctcgatggtcagctcggatgctttctccaaatatttccaaaatgctccaaaatcatcactttctttcaaatcactcatgatcgtataaatatactaaatagattttataatataataattagttattaaaacatctataaaccgtgggtaaaagtgggtaaaatccatggcattccaataccttccgccaagttttaaacaaaatcaataaatcatattttctataatagaagactcgaatggtgsttgaaacttcaaactaaaccacaaagcttnacgtttttatatcgaaattcaaagatacactatacaactattaactgcacanctaatctctaagttactataaatccagcaaaacgaagttgttgacatgttcgcgtcagagtgtgagaggtacaatttttaagaatgatncgaaactaagaagatatgagtaacgnaaggtattaaaaacatatatgaggttgnagtgaagattcagttttggtgaataaaatgactgatcagaatattttgaacatgtacatatataagtgtgtatcagattcagattgtagattatagatttctttaattgtgtgaggatatttatgaagatcgcattactctggttcgtatgtcaaaaacatagttggtagcttca

SEQ ID NO: 84 - DNA, 401 bp, Brassica napus
taagaaaagaaactgagattaatcgcggtctaagtgctagtttgaggtgacttttatgaaagtataccattacagtaaaactgactcttagtcatagcctcataggtttatcattcaacccataaactagaataatattactcagccaattttaagtaaatcattgaatattgttagtgtgagattacccctctctgagtwaattgattctataaacataaatacccatatccccatgcaatgatacaacacatactatttcgaaatccctccgtgattgaaaatatgcattgttcacgcctcttctctattttatctctaattgtaaccatcgccggagctttcgccgccgctctagagtgttcatgtaatgatctggtctgtttatttaatataaatca

SEQ ID NO: 85 - DNA, 801 bp, Brassica napus
  misc_feature (51)..(51): n is a, c, g, or t
  misc_feature (296)..(296): n is a, c, g, or t
  misc_feature (329)..(329): n is a, c, g, or t
  misc_feature (622)..(622): n is a, c, g, or t
agtataaggaagatgtttgaaaacatggaaactcacatattatttagaagnctgccttaccattgccaattgttagccacaacaaaaaataccaatctaacaaggtactttcatgactcgatctcaacttagcaacctaaccattttcagcccacagctcataggagttatccaaattcactatcactgacctcatttaagactaaaagtgcagtctcatcgagggagtatcgatcataagacacatggactcttacctattcaagtatctgatcacacatataattttactctgntttctttcctctctctttctcatttcctcattngatttctctatactctgtagggtatcattttatttttctatcgactgagtttattagacaagattccatgasacacaagcactgatggtggtaaccactaagcacgcgatgcacttcttgttgatttttatcttttttctttcattttttttgaagagaagagagagtaaaaccatattcacacagactagtctttttagacgtgagcaagaagtccaacccaatgtataccaagatttaagacaagagaatcaaatagattaggtgagaggtcagctttggatccttcgaangcccaacaaacatggatggcagatcaatccactttggcaacaatgtcttttgttcagtattgctacttggaaagcaaaacacaaaagcagcttatttgttttattttcttctcatacttgtgtggttcaactggaagtagctcagtttggaagggttccatcatagtgttctctgtagg

SEQ ID NO: 86 - DNA, 801 bp, Brassica napus
  misc_feature (1)..(85): n is a, c, g, or t
  misc_feature (369)..(369): n is a, c, g, or t
  misc_feature (612)..(612): n is a, c, g, or t
  misc_feature (681)..(681): n is a, c, g, or t
  misc_feature (704)..(704): n is a, c, g, or t
nnnnnnnnnnnnnnnnnnnnnnnnnnnnnnnnnnnnnnnnnnnnnnnnnnnnnnnnnnnnnnnnnnnnnnnnnnnnnnnnnnnnncctttattacatgccagttcatcgtcattcgtcactgtattgacacgtgtcgtaagaccattatatactttctgtaatcccatgaaacagtagttaattacacttttaacttctgcacgtaagactaaagatgaagggaagatgaatgacatcttatgcatgtgcactgcacgcggccggcgactcccgccggtttcgggtttaagtgggtctctcttctgcatgaatagtagtagctttctttttttaaatgtgtatatagtagctatatagtttatttatgnttcctagtaatatataatgtgttttattttcsagacttctcaattactcaattctttataataattaggtaacactgttgttaattttttattttctttcttaaaatggttttagcaaaattaaataagctagatagatatagctaatatacatctttcattttaagtgtttgtgtgtatttttgtaaatttgaagttcaaaaacgagtatttaaatgattggatccgcttgcaagtggtatngacaattagcacaaaattccactctaactctcagtatcgtttacaaagaaaagcgtatggaaataaatnaacctttacgtattagattttangaacgaaaactcaaatcctaatatgataattgtctttaattataaaaagttataaataattacatattactagcaacctccagtgactcttaattag

SEQ ID NO: 87 - DNA, 401 bp, Brassica napus
accagaactagatattgatccttatccctgaataatctggtatattcggaaggctcgaaatgaaaaaactctttaagggatagacatggatcctttggagctagttcgctatgcagagagtgagtgtcaagtctgattcaatgcaaacaagatggtaacgccaactacacaagagcataattttgaagaccctcaagtctkaaacttgggtaatatttgcattgtaacttccacagcttcgttcagcgggtgtggttgggtttggaaggatatatagctcggggaaggttcaacttatggggacacgaaattatagacggtgagagattgctttgctttcagaagtggaggtcttacaatgggcgatggagagcatgctgcagaattcgacatgccagagt

SEQ ID NO: 88 - DNA, 401 bp, Brassica napus
aatatatctttttttgaaaaatcgtgtatctttaaaacagaagcgcacgtaatccacttttctctcagtttcgagtctctcttttcctcggagcttgtcaccaagagagagagagagacatggaaagacttctgcaaccaccgtcttcttccacaatctctccttccaaattcacctcgaggaatccccctctccttcctygtctccggttcgtctcaacgtacagacccgagtcacgccgagtgagctccatttcctgcagcaatctccagagcccatttgtgggatctaatcagaccaacatttccttgaatggatctccttcctcatctcctgtagcaggagaatcgaaccctaatcatgggtttttccaacggatcgtcaccacggctgatgagcag

SEQ ID NO: 89 - DNA, 401 bp, Brassica napus
tcacaagggctttaaagtaaactcccatcagacccatgaccatatctactaacttcaaatcagaccctgaagtggtgtgcactgtttggtcaactgtcttcatgaatcatgatggcctctcccctggtgattcgttcttggtatttcacctctcatgttgctataaggttatctatcttcagtcagatctcatggcaatgygagaagttgttaagtttcctttagttcaatttgtgattgcttcagaatattgactctttggctatgactttaatgtgtgattgattctgcggatttgaagggccagtcctattactggaactatcagaagcttcatcagttacttcagtttctgcttgtattctctgtgtgttagtggttttgtctagctccttgctaat

SEQ ID NO: 90 - DNA, 801 bp, Brassica napus
  misc_feature (583)..(583): n is a, c, g, or t
  misc_feature (636)..(636): n is a, c, g, or t
  misc_feature (693)..(693): n is a, c, g, or t
  misc_feature (714)..(714): n is a, c, g, or t
atttattgaattcttaacaagcgtgaacattttagaaaatttaacttttgagaatagagggagtagtactgatatttttaaccagtatctactatctacattggttttagtaatgtgttattcatggccgtggttaagttaatctggttaattaaaaataagaaacaaattaccgtggtgtctgatagacacgggcttgagcgaatgagtaaaataagaaagcgtggggagtggaaactcgagcctcacagaatcaatcacctagactaaatattctttgaacaatgacagtcacatcctcttattatagtgtatttataatttactagattaatttatagttctttttctcacaaagatcatgtactcattacttcttttccatgatatggacaatcttrtgttgcggttggccatctcttttggcttgcaagctttttgactgaaaaagttagatcctctttctaggtggtgacttttgttgcaagtgatctggattatgggttttcatcctgtatctgtagtttataaatatatctgtgaggaaaaaagaagaagatcatgtactcgtaattcagtattnttctgcagcacaattctgaatttggaaagtttaaaatagacttcttaattcanataagtcagcaaggtaagttacatgattacatatctacaattatggaaaatcaacanatttcaattaattgtttgttncttaaactcaataatttttataataaaaacaaatatttaaaaataaaataacgtgtttactttttattatatatatgattatagttt

SEQ ID NO: 91 - DNA, 801 bp, Brassica napus
  misc_feature (65)..(65): n is a, c, g, or t
  misc_feature (95)..(95): n is a, c, g, or t
  misc_feature (110)..(110): n is a, c, g, or t
  misc_feature (416)..(416): n is a, c, g, or t
  misc_feature (466)..(466): n is a, c, g, or t
  misc_feature (667)..(667): n is a, c, g, or t
  misc_feature (762)..(762): n is a, c, g, or t
  misc_feature (771)..(771): n is a, c, g, or t
aagagtatccaaaaagaaagagagaagaatggatgacgcgcgtctctgtttttagtagcagagangagagagaaatgaagaacaatggtcgctanttttttgacgtcagnggcaacaccggaaatcttagccttttttgacgctgcgttgcttgttaatggccgctgcggtcatcggtgttgtgtgttgccatgactcccgtttaaattttggccgctgccgctgcgtcctgcagctaagaaacgaacacggctattgttattttcgttgttgacatggtcaatgtaagctgcatgtttctcttctgtatttccatacatctttctcgatcaaatgtttgcagccatgggtaagaataatctcccctccttctagagtctgggaatcgaaatttgcgtcawtaaaatttgtaacanagaaaataaagcttttaatgggggtccaaattttctgcagagccaacganaagtaatcaaacaccatatatatctaaactccaaatatcaatcatgatctaagtgttaaacagctcaaaattttgctataattttagacattaatatatatatataaacccaaaaaaaactaacaatttaaaatataattttatattaattataataatatgatttataatatttacataatataaagtgttaatattgtncatttattttaaactgatgtcaaccggttataattatcccacaaacataccaatttctaattgattgtaccagtcgtactaatcggttaataacntttgaaacngcatccgcaaactcgcatttacaccagtta

SEQ ID NO: 92 - DNA, 462 bp, Brassica napus
ggaatttctgggtcgacgattccgtcccaacgtcaccacttccctcccagatctactatcaccctgcaagttcatctacacttaatccgacacagcgccctcgcctatcaaagcamgtctcagatggtcagatctgtggaatgaactcacttagcagaagctcgataactgaagagaggcagggaactcctttaagatgtgattcttctgagagtggaccatctgaaggttggtcactgcaggccttttctgaaatgatgtcatcttctcgcagcaccgagcctttgtcttatgataacgaccactttgggcttgaacgggacatgataggccatcacagcaaccgaatgtccaatcatcagcagcaaagctgtggtgcgtgctctagacccttgtcagagaaatccttgtggagcagccaaaagatgtttatgaccaacgagctctctgtgtctgcaattc

SEQ ID NO: 93 - DNA, 801 bp, Brassica napus
  misc_feature (200)..(200): n is a, c, g, or t
atagatagttcataatcaagagattataatttgtaatatttccatttatttatgacggtgtaatcttttatataaagaacttctatgctttgaataaagataaattttcttatttttataagaaaaatataattttgttaaaaaccgacatacaatgagacttgtgtcgccgtctcatcgtgtttttcttttcccttcangactattttataaatcttgcgttagacgttaacgctccaattgatttgtgcgagaaaattttacataaaccctagaaaactctcttattgttcgcgtttaattcttcaggtacgatttgccatcctctctctctctctcttttcaaaaggtatctgcttttcatcgtctacgatcgagagaaacttcgagactttgcctcytttgttgggattgaaattggttaaaggtttaattgtttttggtgttgattgttttatcggcgcgcagatatgccggtgatgaatccgtcgtcgttgtgtattggtgcacaaccattggtcttcctccctcctcgctttaatcatcgaccagctaatggtatctctctacttttgggatatacacttcttcttgatttgcttcttgccactaatttatgattgctcatgaaaaaactgatgttcttgtagcattagatccttgcttaatcagatttctcaagcttttgattttcgtattctattgaatgtttcaagtgttaataaaagctcttcttctttttgttctgtggtaggacaatttcgtgggcgttactaccctacaagagtttctatgcaattc

SEQ ID NO: 94 - DNA, 401 bp, Brassica napus
atgtaaaagaacgtaaacagattaatagtatataaagtaatttgtatatagaatatttattccactcaaggcgcggttaagtagttattattcagcatgtatatatttgttaactattattaaaatgcaaaaaatatgtatagtagaatacttaatgtttataatcacgagatataattgttttcataaattcatccccamatgatgcgggttatcacctagtgtgatattatacatggccaccaggttgatccgatccaacagagtccatcggtcctcttcaaaaagaacaaagctttattgtacaacagataaaacgtagcatatcgtgctgcttagacttatcttctccatatggttgcagagctctcggatacagtcgttgttttctagcaggctga

SEQ ID NO: 95 - DNA, 151 bp, Brassica napus
acgaccgaggaaagcacctgcggaatagagaccaaggcccaacagcaggaaggaatcgatactctatagatccacmactagcaacctagaatttgaagcagagatggagcggagaaccgcaccacacaaataagccaccaccaaaatacct

SEQ ID NO: 96 - DNA, 801 bp, Brassica napus
  misc_feature (168)..(168): n is a, c, g, or t
  misc_feature (263)..(263): n is a, c, g, or t
  misc_feature (421)..(421): n is a, c, g, or t
  misc_feature (493)..(493): n is a, c, g, or t
  misc_feature (559)..(559): n is a, c, g, or t
  misc_feature (722)..(722): n is a, c, g, or t
  misc_feature (753)..(753): n is a, c, g, or t
  misc_feature (772)..(772): n is a, c, g, or t
tactagcacttgtttgcaagatcggtggactcacactttgatgatggagtttctgtgtgttgtatagagtcaatgacctacatgagtaaccctgtttgtagtccttattatcacgtaatggaaggttccccttctggtgatcaaggtcgatgttattgtgctaacaangaaggcgagaatacttggattttaaaataaatttgaatagttaaacaattttgtatttatctttgaagtttacatgtgtttataaagaaatctangccaacataagccaaagccctcatcatattttcactatgaaagcaatacccttttgtttaatcctactctaacttgttttactacttaaggatgtaaactgagtaattatagtattgtgccaacccttttgttagacsgacttctttgtccttctccncttgcacaagtcaaacaaaagcccctaggcccatcctcatggccttagctcgtgatctttttatcggcccangtgtaaaaagaaatagatctttaacttggatgatagactcatttttgcctgtgaaaagcccatttngaccatctttctttaaaggtggttctaggttctctttgacttgtccatgatgttcatcgcttccaattagtcaaaaatgtccttacatagtcatttccagctccgagtcatctttctcattcttattctcatttcacgaccataacgcatagtcgacctcatntcaggttgatcgaagatcgaatcgtccattnccagctagtccatgttcangtgtcgcatttcccgcctactcatggttg

SEQ ID NO: 97 - DNA, 401 bp, Brassica napus
ttggtgattgaataataagaaaagaacttcttattgatattgtgattctatagataacactcccatcatccagcaggacgcaactcagcagttcaatcctgaaggaactcccacaccacccccaactggcagtgttaccaacggcatcaaccatcaatctgaatggtatgttatcacaaatacgtgataatttgcaaaaakttctctgttttgatttaacatacaggtcagtaggatgccgtggcacagcaagctttttaacgcttcaagcaactcaatcaggtctagaccaaccagtaggcgcaaatcaattccttaagtgcatatcaccaaagactccacgccagccctaatcaccaaagactccacgccagccctaggtggacgtacaaactcaatag

SEQ ID NO: 98 - DNA, 801 bp, Brassica napus
  misc_feature (271)..(271): n is a, c, g, or t
  misc_feature (587)..(686): n is a, c, g, or t
tgagatttgggccatgactcgaagataaagctttatgacgatcatcacactacaagaagagatctggaaacttctccaaaggccagcatcgatcgacaccgccaacccaacatcgatcgaccccgcccacctgataccgatcgacatccacctaatgatatcgatcgacacccatcgttggacgacctgccaaggtcacagttgggctgaaagtagttgaggagagaatgcacacgtctacgacctcacaccttgctgtccccgaacatcngagaccacctatatgcacagaagaagctgctgggtttcacaaaagagtcaagaggatacatgaccatgtgaagtttgtggtcccatgcattgtatttgaagttgaatctcctattccaacaaatagaagygtgcatctaggttcttacattgggaaatttgatgatcatatgtatgcactagtttttgagagagggttgagacatataagtgacgtcgacacagccccaacagaaacaacatcgatcgacactaccacttcatcgtcgatcgacattggacgtgtatcagatcagaaggagtttgaagtgtgtcgnnnnnnnnnnnnnnnnnnnnnnnnnnnnnnnnnnnnnnnnnnnnnnnnnnnnnnnnnnnnnnnnnnnnnnnnnnnnnnnnnnnnnnnnnnnnnnnnnnnncggcgaagagtagtaactgttagcaccatcagagatttaagatttgtgcacccgggaaaagccatattcaattagtcttctttatccggagatgctaggtctgctggtaaaaaaa

SEQ ID NO: 99 - DNA, 801 bp, Brassica napus
  misc_feature (117)..(117): n is a, c, g, or t
  misc_feature (152)..(152): n is a, c, g, or t
  misc_feature (198)..(198): n is a, c, g, or t
  misc_feature (427)..(427): n is a, c, g, or t
  misc_feature (459)..(459): n is a, c, g, or t
  misc_feature (464)..(464): n is a, c, g, or t
  misc_feature (773)..(773): n is a, c, g, or t
  misc_feature (784)..(784): n is a, c, g, or t
tttaatacgaaaaagaaaattcagtttttaacaaataacgaccataaaaatactaaaataaaaaacaagaaacattatttaacatttcactttttgtctatactttattaaatttgnaacatgttctcatacatagaggaaaaaacaaattncaaatacatagttaattttaacgtgcaaacatgtcattattttaantatttcactctgcacagggcgcggattattattatgaatgagataagtatgtttgatacgatcattcatatttatgcaattagtatatttttggtatacggtttatattatatgcattctttgtttgggatatgaatattaaataactagccagaaaacattatcataatgtcatgactgcctggttttaattaacatgatamacatatgggatgtgtaagaccaatcnaattaacgatgtgtgtagttggtttttaagantggtntggtccaatggttttaatcttttattgaattagaaatctaatttgattggattttaataataaagtaaagactatctgattagtaattaaaaattaataattttaatacgattaaaattagtttaattatttataattcagttaaaatacataaaagatttgtattagttatatttatattttatattatatataaattttaaatgtaaaattaaattagattaaaattgtttcctcaattgatttcaagtattttttatgtttacacagtcttatcaactatcaaagctcgtttcgttgtaagatgantttggcaaagnaaggtgtcgttagttac

SEQ ID NO: 100 - DNA, 801 bp, Brassica napus
  misc_feature (434)..(434): n is a, c, g, or t
  misc_feature (460)..(460): n is a, c, g, or t
  misc_feature (537)..(537): n is a, c, g, or t
  misc_feature (609)..(609): n is a, c, g, or t
aattaatttgtatagttacatttttttagttgtattacaaatctcataacgtaaaatcattaatgaatctttagttaaattattagactagactcgctagatagatttccacaaaccctattacattttctttataataacagtgaaaattacatgaaaatgtgaaaggctactgcacattttcttatgtggtataaaaatattaaattataaatttggtatatatgccgaaactatttatgttggttcatatacggttacatataaatactttttatcggtatattccactaaacactaaaatattgaagatattaaatatttaagatatcattgtccgtttagaatttcaaagttaagcgtgttcgacctggaatatcggaagaatagatgacttatcrgaaagtgattcgcgatatcgtgcaagtgaatcnaaaacacggagaaaagtcacgtggtnaacgggtggatagtttggtaggcggtcgggccgttacatctaccacgtcctgtaacacaggtgcagcctctgtgaanaaaaatgctggttccatacggacaggtgcagccagtggtatggacgggcagggccgggtctgaatagaagtncatcgagcatgtgtttggagcctgacgaatatatagatattttggggccaattatttttcatacagaacatgcagctctattggcttggggtccaacgaaaatatagatggacctctgttcgcttctccgcaatcgcatcttatattattatcactattttttagaaacaagggtcaaaaatatttttttag

SEQ ID NO: 101 - DNA, 801 bp, Brassica napus
  misc_feature (229)..(229): n is a, c, g, or t
  misc_feature (270)..(270): n is a, c, g, or t
  misc_feature (492)..(492): n is a, c, g, or t
  misc_feature (570)..(570): n is a, c, g, or t
  misc_feature (768)..(768): n is a, c, g, or t
  misc_feature (782)..(782): n is a, c, g, or t
cttgactatttttatgtgaatttaagaaaaaaaataaaagtaaaaaattattattttttattgttttcagttattgtctaatgagtgataactcctaacttcttaagaagtcttaaataagaataattatgaaagctagttattttttttgtcaaccggatgtttattaaacaaggtctataatataaaacaggtccaagaagatgggcagtaaaactattacaaaaangtccaactgaaaggcaaataaaacataaatgaaaggcctancatataaagcccaatatacaaagcatcttgaggccttaagcccacgagagaaagatctgttggggaagagggtcacacgacgccatatacgatcacccaacgatcaatgtacacgcgtcaagacgcggttycaacattcttcctccggagccagcgaagaggcgtgatggaactccgacgtcgaccaagcctattagatcgttgaacgaaaacatcaatcgnctgtaatcgatcagaaatccaattttcttgcatgcgcaaaactccatctttgatgatttatataagcttgaaaatggngacaaccctaaccgaggggaggaaagagacattgaaccttcagatcaagaggtacggtgctatagaagccaccacttcccgtaaacctaaagccggcgaagatggtgataagggatccaccgcttccagaggcagaaacccgaccattgggagactgagtccaaagagatccgacaaacaaaactcgacgctctctcnctgaaagatagganagagataagagagagcaga

SEQ ID NO: 102 - DNA, 801 bp, Brassica napus
  misc_feature (279)..(279): n is a, c, g, or t
  misc_feature (528)..(528): n is a, c, g, or t
  misc_feature (670)..(670): n is a, c, g, or t
agatctcttgtccgaagcagagcattttttcgctgaaatatgctctaagaagttttttcgccctgatgttccaacgtatcgaacgatgatggatgcatatgtgaagaagggtagagtcagcgatgctgtcaaaactgtgaaccaaactttggatgcctctctaacctatattgctaagaaggtcttagtaatgtaacttccgtttatgtgcatcactatgcaattcagattcttagttgcataccaactgttgtttatccacaaatctggtggaacttnattagtagtgcttaatcttgattgtttatcttttaagtctagttaacaagatcgttaatactcctttcttaaagctagcaataaaacaaaaacaataatctgacgcacatatttgaacttaycaaactatgaagcgggcttccagacttttaattggggctatcaatctgagactccgtttggtcataatctgcccaccattaattgggcgtataatggctcttgagggagagtatagtttatattatnagcagtcacaatgaaccttctgcatattgagtcaagctataatgtggtttcatgtgttcataacgcagaaggagctcgaaatgggtctatccgaaagcaactgttgtacctaacttccatctcccagtgcgcagctttgggnttaatgtagaatattttgttttcaacgacgcgcgtgtttggttctactatatgaaacggcgcacatgtttgattatgttgatagaaacggcatggctttgccgtcttcgaacggtcacggcatggccatgt

SEQ ID NO: 103 - DNA, 801 bp, Brassica napus
  misc_feature (76)..(175): n is a, c, g, or t
  misc_feature (476)..(476): n is a, c, g, or t
  misc_feature (478)..(478): n is a, c, g, or t
  misc_feature (486)..(486): n is a, c, g, or t
  misc_feature (526)..(526): n is a, c, g, or t
  misc_feature (631)..(631): n is a, c, g, or t
  misc_feature (636)..(636): n is a, c, g, or t
tctctggtaaaatcacatatatactataaataaatagtaatctctccgcttcataatatatgatgtgttagaagannnnnnnnnnnnnnnnnnnnnnnnnnnnnnnnnnnnnnnnnnnnnnnnnnnnnnnnnnnnnnnnnnnnnnnnnnnnnnnnnnnnnnnnnnnnnnnnnnnnatctattcttccctccttagtcatgaaaataaactttagaaatgttagtttatagtatataaataaacttttgttatcgtatattaagattgttagtgactatagtaaatgttattctgtaaagatttagtgtttattagaagaaatgagacccacctgtgtttttagagcctggtgcgtatgtatcataaaatattgttggcacgaaacaactctaaaactgtgrtggtttaaactaataaactagagatggttattaatcattactctatgcatctttcgatgtatattaagatggttnangtccaaanaaagaggattctacgtaaaacgttgagtgttgcgtaaagnatgtaacctacaatacagcattaaaatatgcattcactagtgttggggtgtaataatatgattaacacgtattataaggaaaaagaaattaaaaatcttgccccnagatntaggttattcgataacaaaaagagtatgcgttaactctgaacattggtgtatcaggaaatccttagacgaaattggtgttagtttaggattttatgtaattttctcaatgcttataaggcctctaagaatgcgagaaggagataatataaatattacattcgtat

SEQ ID NO: 104 - DNA, 496 bp, Brassica napus
  misc_feature (1)..(57): n is a, c, g, or t
  misc_feature (123)..(123): n is a, c, g, or t
  misc_feature (321)..(321): n is a, c, g, or t
  misc_feature (441)..(441): n is a, c, g, or t
nnnnnnnnnnnnnnnnnnnnnnnnnnnnnnnnnnnnnnnnnnnnnnnnnnnnnnnnncttgtcatgttatgatcaagcatctggtcaagagaagcgaccatatgaatgtacttctttcttggnaaacactttaagaaacttttaacaagctttggctcttctatcatctgtcccaaagaagccgatttggaggagatttcggatagcttcccggaaaaggtatcgattgtatcttcatatttcatcttgaktctattgaattctgtctttagggtttgaagcgtagcctattttaccctctcagctcctacatgtcttgtntttatagcatcccatatcgcttttgttgtgtctaagtcgccaacttgcataatcaaaccctccggtatagactggaacaaaagcacagtggccatactgtttttcttctcgtctttggtnccagggtctattgcttcccaaacttcgctaaccttgagtgcaatcttcattctca

SEQ ID NO: 105 - DNA, 401 bp, Brassica napus
ctttaagtagttgtactatgacttcttaatagtagataaaaataggaccctaaactaatagattagatatattgttatttataataatgataaaaaagataaaacattattcgaaatttagagatttaaatgaatcatggaaaatgcaagacctatttggaccaggatcgatttgagatgaaagctaaggatatagctagrcaattcaattgttgaatgttaccttttttgttcaaaagttgactgttgaacaatctattgattattcaagccaagattaatacaaaacaaatcatctttggcatcaacagcttctaggattttagatgcttacatattttgtgcaaggaccgccagtgtttttgataacagtgttgaaacacaagtggtcatcaaaaacg

SEQ ID NO: 106 - DNA, 801 bp, Brassica napus
  misc_feature (165)..(166): n is a, c, g, or t
  misc_feature (456)..(456): n is a, c, g, or t
  misc_feature (476)..(476): n is a, c, g, or t
  misc_feature (555)..(555): n is a, c, g, or t
  misc_feature (576)..(576): n is a, c, g, or t
  misc_feature (623)..(623): n is a, c, g, or t
ctttaaagaattcaatttaaggaatatctgaagaagaaaatcaaaatgactatggatactagaaagaattagagaagcaaagtgagaaaattcaaaattgtaacgctttatggtctgaaaatataaaatttgacgctgaaatgatcaaagttgactcaaaaggtnnataaaagtcttgaaaattatgataataaattttgagaatagttatgattgatgtgaaataatgtctacaaataaaagagaatatgatgttttcggtgaatgaatgtcatatttatatattttaccttgatgaggctgaactgaattcgagtcatgaaattattattctcattggatttggagtttcggtaaaccagtacaaaatatccaaatgtttttcatctatcacttgtgcwaatctcttgacaagccattatttatcttcaaactattttaaatccgtacaactancaaattcgatgctagaaagnttggaaaaaactctcataccttatcttttgttatatttaattaatccaatgcttttatgtatcacatgcagaagataancaatatctggtttaatcaatntcccatgagcagaagttttaaaaaagtagtttagcaatcgcggtgangagatatataattacaattaacttttgtctttgacaaaaaaatactacgagtttcgtcccaattattacaaaacaaaagttttaaaaagcattaaaatatatacatattaaaaatcattcttctgaaaataatgcttgcatccaaagtgaaaatgcgacacttaatctgaatttttga

SEQ ID NO: 107 - DNA, 151 bp, Brassica napus
gtcttcaggacttcaaaatcactccccagtacccaatgctcatctcttttgccaagaaatgaagagaaactgcctktgttttgtttgtcttttaagatgatgacagtgagacttggtgtgtataaccgacggtttaatgtttcggttcgat

SEQ ID NO: 108 - DNA, 401 bp, Brassica napus
gaggaattatatacgcgaaagcaataagcaaccagacagacaccttaccaccacagggtgtatttattcatttaatctatttttttagttaaaccttgcaaggtttaacgaaacttctggtgtctatctggcttgaccggcagggggccaagcggttatttccatgctttgcctaagagattgcttcatgtgcagctaatyttcgttcaaccatagtcagatgactacaagcacaagcacagtgcggaagagtgtgacgccgctgtccctgcaaaagaattgcaatcaaactataattatgttaagatagtattggttatagaggaaattaaataaaaagtaccaaaaagggtatgagacaagtccttggagatcggtttcagcatgaaaaaacatgggta

SEQ ID NO: 109 - DNA, 801 bp, Brassica napus
  misc_feature (396)..(396): n is a, c, g, or t
ttctttccctctagtacttgtctcctgaacctaatcgtatgtatctttgaccaggtgaaaggtgttaagagtggtatggtttagtaaggtctactaaaccaaaccgagactcgggttgttaaggttgttgagataagtacaatgtattagaagataaagatgcacggtagatgtagataaagtagaatctccttgtaaagatacgaaggtcgagtatatgtatccaacgtgatcaatgagatccacacacagtttactaaatacagtttctctctgagtttacatggtatcaaagcgggcccaacatttccatattcatctcctcaggaaacatcttgatcatgatcagaagaaaagcttcggggaggatttgttataccattgcatcaagcaatnagccwttgagaagtgtgctaccgttgtccaacgaccctctgtttcctcggagatcagtaaaggaaatgcttttgcagtcttaaaatgttaatggcaatcaaagttgcctcctcatgaaaatattatacgaggcctaagtaggtccatatctttcagttaacaagtttgaagttcacccttttgcatatggagtctgaatgatcaacaccaaaatttcatgtggtttcagatttatagcgtaatccttgataaacaatatcaacaagaatcatttttaagcaagttttcaaaactctgcttcctgctttctgatctaatcagtgctaagatcatcacttgttaagtagttcaacatcaagcttttctgaaaatgagaaacatctcacatgttctgcctgctttcag

SEQ ID NO: 110 - DNA, 801 bp, Brassica napus
  misc_feature (269)..(269): n is a, c, g, or t
  misc_feature (308)..(308): n is a, c, g, or t
  misc_feature (427)..(427): n is a, c, g, or t
  misc_feature (538)..(538): n is a, c, g, or t
  misc_feature (595)..(595): n is a, c, g, or t
  misc_feature (643)..(643): n is a, c, g, or t
  misc_feature (752)..(752): n is a, c, g, or t
  misc_feature (765)..(765): n is a, c, g, or t
tgtatcgatcgacggcactggatgtgcatcgatcgattgcgtcttcttcgtatcgacctctaatggtcagctcggatgaaatctattttaagctcctaaatgctccatagtcatcactttactccaaaatactcctgaacctgaaaacatacctaatatgatagaatatataatatatagatagtaaaacacttatataccatggatgaaaatgggtcaaatccatggtatatcaagcatcccaaatacttcgtcaaatccaacctcantggtattggggaatacactcagtgctgctttgtatgtcntgtatttcaatgtaatacatctaagaattttcttcactagtttctttccttgtacttccttccaggaataagagcctattctgacaaggaacwaagtttagagtgtgggaaccgaaatncgcactgtcaatttccgataaaaataggaaagctaagtaatcctaactttcccagaggtcccggatatctgctaaaccacacgccaagcgatcaaacaatgagaacaaacnaaataaaaaatagtagaaaacgaaaagagagcagagaagatcttattccgaattgantgaacgagcattacaacagataaagcctcggcggttagagatgtcggngagttcctagttctaaccttgtgagacttgattaacctagttgagtcgcagctcgaaaacagaaaacggaaatatgcctaagtttccctaagtgctatgctttgttctnaataaaaaatgcntcccttcagcatctgcaacctcgacatccttatata

SEQ ID NO: 111 - DNA, 401 bp, Brassica napus
tttattgatgaaattcccaagaatcattaagcttttgttaatgtacttcccttccgtcaagcgtactccaccagcaccagttttggcaattctttcagatccagccaaatcaaccagattctagaatccattaaaagaaggcacataagagaataaacagctttctacacccgtagagaaaatgatcactcaccaagactragacacggataggatccatagaattgtttcctttccccctgctctcaatcaccttatcccaccagagatattgtatcagaacaaatacttcaaaaaaaaaaacagttgaaggtttcattcataggtttcgaaaaccccaccattctgaagatggtgtgggacgtgctactgtgaacgttcatgtttgtctcaccaaagtg

SEQ ID NO: 112 - DNA, 401 bp, Brassica napus
ggctcccaaccactcacccgagaccagcaaacatcaatcaagaaaaatctctacccaaatatcacggtggattctcttatcgattcaacatcccacacgtggaattccaaggttattcggtcattggtggaaccagaggacgcaaagatcatagaaagcatacctggcatcgtctggttgatcaagatgcatgacattttrccattaatggaaaatatacgataaaatcgggttatcaagtggaatgggtatacccagatagggagaaatcgttgccggtatttggacctacaataaaccttttaaaagcatactcttggaaaatacgttgtccaccaaaaataaaacattttttatggcagttagtgtcgggctgtatatcagtaaagaaaaatttacgg

SEQ ID NO: 113 - DNA, 401 bp, Brassica napus
gactattttaagagcttctaaaggatgtcacatgggcagaaatattctcaccaatcattttgccatgtcgttacgggctgggtttcaaactaatttaaataattccagcccaaccttgccccattccgatccaacctagttaataaagttacattttatttcttcatagacctccacatcaccaagaaaaagggagacacrtgtcattaaaaaatattcaccaaaactttattgtgtttgggtttttgctttacacttacgcatgggcttcagacccatcgtaaaattaagtttccttgccttctcgcctaaggacaggattatcgggggttttagtgaggttttagtgggttttttaagagaggagggacctacaggaaggaaaaaccggtggcagaaag

SEQ ID NO: 114 - DNA, 801 bp, Brassica napus
  misc_feature (419)..(419): n is a, c, g, or t
  misc_feature (756)..(756): n is a, c, g, or t
  misc_feature (800)..(800): n is a, c, g, or t
gtatgatcaagggtcgactaaataaaaatgttggcttgaagagcttcagctgggatccggttaacgttcggaatgatcctataggatcggagtttgttctgtttccaattgagttgttgattgttttacgaagctgacgagctcgagtaaaacatgatgtgtgcgttatgaccttcgaatcttcgtcgcaatcaattaatatcagtttctcttgagttccataacttcaacttcaatgtttttattctctgcttcttattctttcatttaaataatcgagacacgttacttaaccaaaagtatggctcgttatactgcactactgacaaattgctaagagtaaagcacacaaaggtttcttaggaagattattattagactctcatgagaattaggtctgsgcattcgggtttctgccnagtccgggtctttcgtgtcctaaacatttgaacctgactaggtatttaaaaattttggttcgggttcggatcattcttgtgggtccgaatcggttctaattcatatacccgtaaaaccctaattttcgggtaattttgagttccgttcggtttgggtatttaggacccgaagtaaagtatccgaactggatttgaaaacccgaaaataccttaaaaccaacaaaaaaaatccggaaaatacccaattttttttaccattaatctaacacaaagatctaaaaataccaaattttttattcaaatacacgaattatatttctgaaaattttaaattttnacctgaaacctgaaactatacacgaaaacctgaacccaaaactna

SEQ ID NO: 115 - DNA, 801 bp, Brassica napus
  misc_feature (1)..(76): n is a, c, g, or t
  misc_feature (428)..(428): n is a, c, g, or t
  misc_feature (498)..(498): n is a, c, g, or t
  misc_feature (627)..(726): n is a, c, g, or t
nnnnnnnnnnnnnnnnnnnnnnnnnnnnnnnnnnnnnnnnnnnnnnnnnnnnnnnnnnnnnnnnnnnnnnnnnnnngcagaaaaaaagaaaccgtttctaaatacacctctctctctctctctccggatttgcttacttgaagtttttgaatcgcgtctcgttgaagttatggatgattttgcagtcccccttgaaaagcaattttgaccaaatatagtataatatataattcctattttacaatattctaatatacaccgttatttttttttcagtaaattgatgaagaaggattatccatattgcatttcaagatttttagatatccttaagactcataaaaatctaacataaattacatctattcccagagaatacgttttttcgaaatcaattcctsgtctctgaactaatcgggttttatatngtgttacctcattcttttcactaggggcattgctggacagagttcttgtttcatcttaatatttgctaangttattgtagttgtgaattttgcgttttgagttgtttttcaagttttttttattgttatgggattagagttgtgatgatgatctgtgtatgctttgttctccacttatgaaggactaaactgtgttagnnnnnnnnnnnnnnnnnnnnnnnnnnnnnnnnnnnnnnnnnnnnnnnnnnnnnnnnnnnnnnnnnnnnnnnnnnnnnnnnnnnnnnnnnnnnnnnnnnnnaaaagtttcttcattttttcttttcttgatgatttctgggaagaggaagaggtagttgaacttgttgggcttgat

SEQ ID NO: 116 - DNA, 801 bp, Brassica napus
  misc_feature (3)..(3): n is a, c, g, or t
  misc_feature (95)..(95): n is a, c, g, or t
  misc_feature (137)..(137): n is a, c, g, or t
  misc_feature (215)..(215): n is a, c, g, or t
  misc_feature (282)..(282): n is a, c, g, or t
tgnatatgttgatgtggtcgtgttcaagtttcgaagtttcgaactcattatctagattgttgtttctggacatatttttttttgtaaccgattgntgtgttgataatgagtaatcaatctacctacattacattttnaaaggatgataacatgatcattgatcactaacatacgtgtgtagtttgatgattggttatgtcatgttacattgagtntttacttgttacaaatgttctcgaatggtgtacaaaaacgagcttcgactcatcaatatgaaaactntatccaaggattatgttcatgaaataacagatccgaactaactctaatcgtgatcaatgtattaaaatcggataatgcttacccacctccattcatcattcccaatcccaacaccaagwtcttactttcagtgtgattcttagccgagcaggctctcggctaataaaatgcacaaatcactaataaaatctgtaaactaataaaattccaaaattgaaaaaaaatttaacctatccaaaattgcattatttataatacaacactaaatttaaaagttattaattgtattgaagatttatcattttaatcaaagttattaatctacaacactcaaatatttttttaaatacacataaacgtaaaattcaattaaaagtatttaatgttttagaaacttttcttgtaaacaacacattttgttttctattgtgatcgcaatactaagtgaaaattgtaggtgccacattttaaaaagaaaccttgtttttggccgaggaataaacatcataagtattaaaa

SEQ ID NO: 117 - DNA, 801 bp, Brassica napus
  misc_feature (267)..(267): n is a, c, g, or t
  misc_feature (350)..(350): n is a, c, g, or t
  misc_feature (362)..(362): n is a, c, g, or t
  misc_feature (478)..(478): n is a, c, g, or t
  misc_feature (596)..(596): n is a, c, g, or t
  misc_feature (655)..(655): n is a, c, g, or t
  misc_feature (730)..(730): n is a, c, g, or t
ttccatgtttggctcataagccacctatgtgtgtttagtggttttccattttgtattttcaacaggtagaacaaacttaaccaagtataatctattctactttagttttacttttacaacaagtccatttactcattcagtcagtgacggtcctaaaaaaatttgggctggacgcaaattataaattgtgtgacctataaatttataataaaacaaaaatatgctaattatatcccacaaaaggttcgaacctctccatactttttnaaaaaatatcacgattaaccaacaacgctactaaaggtttggtgcaaaacacggccaaaatattacatactgtaaaccgggcnggaagcacatgnttctgccgcttttgcccatggccgatattgcattcagtwgttgaataataaatttaaaatccaagtgtattcttaacgttggtagtataatgctttatcttttctctctttaaatnttattgaaaatgagttattttaaaagtacttctaagtgtcttacaaaattgtttaggtttttctggagcaaggtgacgagtatggtggcttccatatgtgaacacaatattcttttgnattttgttctctttttgatgttatcacttcttggtaatagattaaccggcttcatctcntttctgttttgctatgccatcatttcttttctggactgtttgtatatagtcccaaccgatccctgcacaacgaanatcatgaattttcttttctgaaaatcaacttgttggatctgtaaaatgatgataagaatagacaaaggaaa

SEQ ID NO: 118 - DNA, 801 bp, Brassica napus
  misc_feature (1)..(63): n is a, c, g, or t
  misc_feature (143)..(143): n is a, c, g, or t
  misc_feature (318)..(318): n is a, c, g, or t
  misc_feature (419)..(419): n is a, c, g, or t
  misc_feature (465)..(465): n is a, c, g, or t
  misc_feature (480)..(480): n is a, c, g, or t
  misc_feature (694)..(793): n is a, c, g, or t
nnnnnnnnnnnnnnnnnnnnnnnnnnnnnnnnnnnnnnnnnnnnnnnnnnnnnnnnnnnnnnncaagtttctagtttcttgtttaattctgaaaagggataaagatttcttgtcgactgagaaagaagagtcgaagacaacgntagagttctgtttctttttttttcttaatgtttttactttgtatttcattatagtttaaagtaaaatgttaattttattaactgtattttaaagaaaatgacaaaactggattattattattatttatactaaaggaacaatgattttggttttagttctaagatgataagagtntagttgttttgttactttttaccaaatttccttttataatacattgaacaacagtttgccatttccttactattttactttcscttttacggaaaggtcgngtcaacataaacatccaagaaattgataggtaatggatgccttttntaatgaactggaccnctccttgaggcatttgtctacttttgacaaaatattcacatggttttgtttatggttttaagagcatgattaaccctagaattccattagagtctcttaatgattttttaagtattaaatgttagttaagaaccttagttaagagacatctagtttttgttgctccaatgctattctttttaattaagggttcttaaaacacaactagattttnnnnnnnnnnnnnnnnnnnnnnnnnnnnnnnnnnnnnnnnnnnnnnnnnnnnnnnnnnnnnnnnnnnnnnnnnnnnnnnnnnnnnnnnnnnnnnnnnnnnaagtgggg

SEQ ID NO: 119 - DNA, 401 bp, Brassica napus
atttgacactctaactaaaacaactaagtttttttgtcatttgttggattaataatcaaaatagaaatgagagttacaccaagccggcaaaggtacacaacatttacagagccataagctaacatttatatatgatttaaaagcgaaaagattacactttgtttctttgaaatatttcaacgatcttgttttggtttttckggtttatgatttggcaatgaaactagagtatactaaggctgaaaagattgtgtatgatactttagcttttaatatttcaagatcttgttttcgtttttcgagtttatgaatttcatcccaattaaattttggatttttgggttttttgaatttcggcctcatgaaaatactataaaatttttattcaaatttagttcggg

SEQ ID NO: 120 - DNA, 401 bp, Brassica napus
tccatggtatattttgatttaggattgatttatcttagaatatagaatttggtatggtcgatttttgcagatataagatatttatagtaaagatcagtcgcaaaccggatatgtttttattattggtggaaccacaattaatagagttcccaaaaataaactccagttgcaacttcttcaaatcatacggaaacaatagcrtttcattaaacatgtatagaatgtatatggctttggtctatgggtcatcacatataagaagcaagcaaaatagttacaaaaaagagccaacaaaattgtttgaagataattggcttgtgacgttcaactcaaagaaagttatgttaagaatgatagaacaaagcatattcctaaatatgagatatcaagaaaaataagaa

SEQ ID NO: 121 - DNA, 401 bp, Brassica napus
tcttgagaagtgcgtgtatgcgcttggtatgctaaaccctccacagattcaggaacacctaacatttcttgcttcgaattcaaatcgcaccctgtaacagaatcctagtggagatacaagacatcagtcatatacgttactaatctaccaatggaaggattcagtcaaatgactaacctgcgcaagtggcggcccggttgrttcgacacagatatctactttcccactcccttgactagtaacagagaacacagtagtcgaacacgaaccattatcaacaagaagaagtgaataatcttcttccgcattgttgctttcacgaaaatcctgctctttctcatcgagatactgcaatgtaggagaggcaacaagcggagtttccaatatcgaatcgctatcta

SEQ ID NO: 122 - DNA, 401 bp, Brassica napus
tttcggaagacatctcttcgtaaaggtgaattcaaagctatgattagtctcagtggtcaacaatcaaagttttatacaagtaaacatttgtttcaatatacccaacctttacaccattttctttgtaccaaaactatcaataatgatcgggaaaaatacacttaccaggaaggaggtcaagatcttaaattatttgttaayggagcattagtataaatgataaatataaaaagagaacataatgtagaaagtcgatgctagagcatgattatcggttcaggtgggtttttagtagtaattagaaattaaaaaaaaaaaaaacgggaaaataacttaagcgacgtattctaattaaggcacaagaaccctctcttgtaagacacgcgtcacgtgggaggaga

SEQ ID NO: 123 - DNA, 496 bp, Brassica napus
  misc_feature (70)..(70): n is a, c, g, or t
  misc_feature (284)..(284): n is a, c, g, or t
  misc_feature (289)..(289): n is a, c, g, or t
  misc_feature (362)..(362): n is a, c, g, or t
  misc_feature (480)..(480): n is a, c, g, or t
  misc_feature (495)..(495): n is a, c, g, or t
atgatcgaccgcttattttgtgcataacttagagagagtttttttaatgaaattatttgatgatatttcncaatgggggtacacacatatttataagcaaggataaggcgctgacataagcgcttacctcagcgattacatcatcgcttacatcacgcttacataagcttatagcgattacatcatcgcttacatcattattcattttttagacacacttattttatatgatattttacataattaaacaycgataatggtgtgcttaatgatccatctcgaantcgangatgtgcttgtcgcaactaccgtagtgatcttctggacatatgtagtcttcctctggatattcattttgggtntttttttttgacttcaatgttgaacatttttctgatttcatcaatattcattgagtcactgggagctgcgagtcatggaagtattctggtgggcattcttgggacagagattcgtgcnttactatcttctgana

SEQ ID NO: 124 - DNA, 401 bp, Brassica napus
tgtccgtgtaataaaaaacgggttttaagaacaataaacggccaagcccatttaagacctctttttttgaaaatacaagaattattagtttgatgttctaggttaaacaaatataatcatctcaaatcgtcagccctagaaactgacaagacccttttgctccactgtctcttcagaaacggagagacggaggtggaatcyagcgaatccgagtccaggtttcagttaaggatttgagattaggttatgattactgcaccaagcttattctgttaaaattttaagctttgtggatttgagcttatttctctctctagaaataggtgattactgatctggcagaggtgtcttccaaaactagggcagacaacgaggtatcatcagaaccactgtctccgatt

SEQ ID NO: 125 - DNA, 801 bp, Brassica napus
  misc_feature (119)..(218): n is a, c, g, or t
  misc_feature (357)..(357): n is a, c, g, or t
  misc_feature (533)..(533): n is a, c, g, or t
  misc_feature (727)..(727): n is a, c, g, or t
  misc_feature (768)..(768): n is a, c, g, or t
ggaaaaagcctctgtaactcctcgagaacatcgcctgagagcgttttacatttttttccttttggtattttagtcaaaagaaaattaaccaaatcttttaaatattttttaaaatcctnnnnnnnnnnnnnnnnnnnnnnnnnnnnnnnnnnnnnnnnnnnnnnnnnnnnnnnnnnnnnnnnnnnnnnnnnnnnnnnnnnnnnnnnnnnnnnnnnnnntattgaaaacgtgttttaacagatatggcaatgtttctcattttaatttccagagtttcttgctcctcgttctctctcttatttctctctgtatcgagctttgcttcaggtttgggtgaaggagaaggttgtagagagngatgaccagagttgatccaggaatgtaagagacactgagctcawaggccagaaacggagtcttctgatgtgtccaagatcaccgtgcctgttgaacctcctaaagctatctgcaagacacaacagagaaagagttggagtttagacggtctagaatggttggaagtagttcaacanaagcctgctaatgattctattaccttgcgtggcatcattcctagaagctccatcatcaaaggcaagtgctcctgttagacgcaacaagtgaagtgaattagctcacaagcaacagcctatagctacaataatgtttcatgacagaatcaagaaaccaaaccacagttacctcatctctatcatagttgtctccnctatggggatcgaacagtacatctccagtggcaagttcaanacatatacacgtaaacgaccagaatcagccgat

SEQ ID NO: 126 - DNA, 801 bp, Brassica napus
  misc_feature (122)..(122): n is a, c, g, or t
  misc_feature (242)..(242): n is a, c, g, or t
  misc_feature (276)..(276): n is a, c, g, or t
  misc_feature (325)..(325): n is a, c, g, or t
  misc_feature (331)..(331): n is a, c, g, or t
  misc_feature (373)..(373): n is a, c, g, or t
  misc_feature (576)..(576): n is a, c, g, or t
  misc_feature (640)..(640): n is a, c, g, or t
  misc_feature (650)..(650): n is a, c, g, or t
  misc_feature (665)..(665): n is a, c, g, or t
tcaaaattaatatgacctagttgtgaatgttatcttcttgactcattctcagttgatgcttggagacatgtggttggctttataaccatatgaactttatacaatctgtttcgtgatcttcnagctttgacgagcaattttctgtactgatcttgcatcattaattcttcccctctcatcctgatgtgacaccctgcttttgtagcttaccccaagcttataatattactctttaggttagnaatgaaatacacgtcagtcatctttctcgagtcnctgttcatgtcggtgaagtatattgtgccttttcttttaatgtctctangagaancgtcaccaaaccgtactttccctatgatggtactatcaatcngtgagaagtaccttcgatctcctgtcawatgattactagctccattgtcgagataccatatgttctcccctctagtatttgtctcatatttctcaaggagaacattcttttcgttcaaaatacttcttcatacatcataagttcatcagcttcttgcatctcagtgtttcggtctcttgagcctcctgtaacttaagcttganctccggacattgagccacgaagtgtccaattttatcacactgatagcaagttattctcattgcntttcgtccancattaaaacgtcttngacctcttcctctgtaatagtttgatcgaccgcctctgcctcgacctctgtatgtatctccattgtaatctaggtttgcttgttcttgataagatcagtttggttgatcttgagaagaacgattttggttgacttg

SEQ ID NO: 127 - DNA, 801 bp, Brassica napus
  misc_feature (36)..(36): n is a, c, g, or t
  misc_feature (54)..(54): n is a, c, g, or t
  misc_feature (156)..(156): n is a, c, g, or t
  misc_feature (207)..(207): n is a, c, g, or t
  misc_feature (409)..(409): n is a, c, g, or t
  misc_feature (445)..(445): n is a, c, g, or t
  misc_feature (487)..(487): n is a, c, g, or t
  misc_feature (501)..(501): n is a, c, g, or t
atcgttatttcctttttttcattatgacgtattatnatatccttttccttattnggtttgtccaatcgaagggatatataaacagagctttgtttcttgtttgaagatacgtttgatttaatagaaagagctttgctttataccttgtttagattngattaaattcatcaaaacagaagttggtctcaagaagctatcgaaagaaanttttgatcgatccaagaacacgtctcgaagaaccctaaattcttatatcgagcgttcacccattcgtacgctgcgccattatgagatgcttactcttatccatgccggtcagtctagtacgtctcgttttcatcaatttctctgttccagagtacctgcattggcaggttttaaatctcagatttgtgcataawgacacccnagtaagaaacacaaagattgtttgtgcgttatgttnatctacagtaacacttccattggttttgagcaaggccaagtnatacttatcagttntctcttcagaactggaaaaatctttgtcgctactattagacaccagaatgggaccgatacgtaagttagatgactcagagaaaaccacttagacgacaagttgcatataagaaagccgaataataagaatgcattttcaagggatgtactaaaaatgaatggaggtcaattttgggagttgaatgtctttctaaagcaaaacaagacttataatattctacagctttgcataccatttcagatatagaacagccaaattcagtcaggtcgtacaaagcgatcaaaccaatagaattcaaa

SEQ ID NO: 128 - DNA, 801 bp, Brassica napus
  misc_feature (198)..(198): n is a, c, g, or t
  misc_feature (217)..(217): n is a, c, g, or t
  misc_feature (254)..(254): n is a, c, g, or t
  misc_feature (274)..(274): n is a, c, g, or t
  misc_feature (443)..(443): n is a, c, g, or t
  misc_feature (521)..(521): n is a, c, g, or t
  misc_feature (544)..(544): n is a, c, g, or t
  misc_feature (603)..(702): n is a, c, g, or t
attcgtccaagacttcaggcaagatatttaaattagtctcacacctttagttgcttcagttttcctgtccatgatttcttgtccatgattttctgtccatgatcaatcaggttcttcatgtttttagtcttgctctttattctcttcacgtcaacagaaaccagctacttaggcagttaatcaatgtattgaacatgnagagatcatttcgaatccntacagcttccatctttttccacagagagatgacgacntcgtacttcttcagtttganaatggcgttcaacagtttattgagatcgatgattgaagggaaggggcgagatttggccatgtcgttgaacaaatcgatagcgtcatctagtttgatatcacgacgacggtttctgctcagtctctcwcggagatcaatcacgctggagaaagctcgtacccagcaaccnagagaagggagagcgcttttgcgtttactattttcgaaaagattccgatgaagcaatgtcttcgccgtcatcgcaatngatctctgcatcgttttgcgatngtctctctgattccgaatcctaaaacgagacatgtttatggagagagagagagagagannnnnnnnnnnnnnnnnnnnnnnnnnnnnnnnnnnnnnnnnnnnnnnnnnnnnnnnnnnnnnnnnnnnnnnnnnnnnnnnnnnnnnnnnnnnnnnnnnnnattctcaggggtaaactctttgccgcttggaataattaaactgttccttgcgttgcaagtaatcatgttatgaaagttaattcacgcaaatccaaagtc

SEQ ID NO: 129 - DNA, 801 bp, Brassica napus
  misc_feature (98)..(98): n is a, c, g, or t
  misc_feature (594)..(594): n is a, c, g, or t
  misc_feature (660)..(660): n is a, c, g, or t
tgtgcaggatagaacgttatatggggagttggaatactttcatttgtttgaagctgccaatgaaggaggatggttgggacactactgtttatagatgntctgctttctttctacaacggaatacccctgcgttactgccttgacaatgagtctgacctcaagacctatcccgacattagccaagctgcgtctgataccagcagacgtatctttgtttcggtaaagggatgtctatcgttaattattatcttatatataatactattggtaattctatttggctatgaatgttttcgttgctttatcaaccacaaaacgaacctgaattctgcaaatgaataaatatcttatataagtatttgaaatcctacacgattttaagcatgtcaatttttaagccwggggtgtatcgcgagacggaatgagggtgatgcgcctgttctcaaacgagaaggagtatgtgttagccaagaagaaggtgacacgcatccattgggacaacgtcgcaacagatcacatcactgatagttctgtccaacagagaatgggactttgcaacgacgtgatgtacgaatatctgtctgtttattcagncacaccagtttgtaaggtgttgggtgtggttcggcaaataaggcaagcttggccacagcttcttcngagataacattggtgcagctaccgaaatcgatcacgaaacgacaaacctttccccggatggtgcaagaggagcgcgattcgtcaatcacctgaggagtcagcatatttcgacgaataaccaatagttgtccaatatctcca

SEQ ID NO: 130 - DNA, 801 bp, Brassica napus
  misc_feature (90)..(90): n is a, c, g, or t
  misc_feature (94)..(94): n is a, c, g, or t
  misc_feature (124)..(124): n is a, c, g, or t
  misc_feature (464)..(464): n is a, c, g, or t
  misc_feature (643)..(643): n is a, c, g, or t
atcgaaccatcgacgaaaccgagcttcttccttgctttaagcgccatacgcaagttagtagcccattcattgtagttaggtcctttgagnaatngctgggaaatcaccgagcctggattgtcantagaagataagtcatacggagatatcctccttcgttggacttcaacacgagattgtgaagaagcagatttcgtagccgaagcgttagtcaaatcgtcaccatcattactacccatattggcaaacttagagaagaacaaaagaggatgaaaaaccccaagaacaaagaaatttttttgtgtttaatgctctgataccatgtcaagaaaccagagaaagcatagaagagtttcttgtattcatctaggtcaacgaccataagtatatatacatgctasgttacctaataccgtaagatatgtacatcgagataaaaggaatattaacataatagattacanccaaatatatggcaagatatgcatgtatatcctcaatattgccgctcttccagctgaagtatagctgcattgacctcatcaatagtcgtgtaacgggtcatattggtctcaaattggcaaatagatcctgcgttgagacagaagttgacacattaatttgttacagatatgcggaaccnaagtgaaaactgaataaacaaatgttttaagaactaacctgcaagtcaaattcaatatccagaggaagatgacccttgctcagtatgtatctctggaaatgtatcaaaaaattgatcaatccttttctttgaagaaccttatatgatgttgaagttaa

SEQ ID NO: 131 - DNA, 801 bp, Brassica napus
  misc_feature (36)..(36): n is a, c, g, or t
  misc_feature (94)..(94): n is a, c, g, or t
  misc_feature (154)..(154): n is a, c, g, or t
  misc_feature (158)..(158): n is a, c, g, or t
  misc_feature (264)..(264): n is a, c, g, or t
  misc_feature (280)..(280): n is a, c, g, or t
  misc_feature (367)..(367): n is a, c, g, or t
  misc_feature (381)..(381): n is a, c, g, or t
  misc_feature (509)..(509): n is a, c, g, or t
  misc_feature (610)..(610): n is a, c, g, or t
  misc_feature (703)..(703): n is a, c, g, or t
  misc_feature (791)..(801): n is a, c, g, or t
actcaagaagtatcttctcagcgcaggttttcatanctctcttgctgatacgtctctattcattctccgccatgaaggacagtatgtctacttnctggtttatgtggacgatattctcgttactggtactgatagcactctggttcaacgaggnatcnaacgtctggctgcaaagatctctatcaaggatatgggtcatctcagttattttctcggaatcgaggtgatacgaacgaaacaaggactccatctaatgcagcgganatatgttacagacttnctgcagaagacaaacatgcttcatgcaaaaccggttgctacgcctctcccttcctcaccaaagctaactctgcactctggtcctctnttgtatgatccttntgactatcgacgtgtagtasgcagtctacaataccttgccttaactcgtcctgatgtttcatatgatgttaaccgactctcgcagtttatgcacaagccatcggtggaccattggaatgcagtcaagngtatgctatgctaccttgccggaactctaagccatgggatcttccttcgcaaacaatcatctcctcagctccatgcattatctgacgccgacttggccggngacacagatgattatgggggtgattggttgggctgtaactgtagtaaatttactttagaatttagtctgtaggatttttgatttacctttaanggatgtagctttaaaatttcctacacctaaaaagatggggctttagaaaataagatatttacaaccattttttgtttgtttttgttgnnnnnnnnnnn

SEQ ID NO: 132 - DNA, 496 bp, Brassica napus
  misc_feature (214)..(214): n is a, c, g, or t
  misc_feature (356)..(356): n is a, c, g, or t
  misc_feature (459)..(496): n is a, c, g, or t
caagttgatatggatcttgttatttcatccataaagggtcaattgataactattattggactaccaaagcaagtgtatccttctcatgcctcgctaacaaactactaaagctcaaggacatagtctttcctctcattaagcaaaggctggaaaatggcctctcagctaggttctggttcaataattggacatcttttgggaccttagcatcttnccttgactcctctactactaggctagggattcttctyattgagttgcttctatttgtaggaatggaacttggctaatcccaccttcaagaacagacaactagcttcaaattcaggctttttgaccactatcaactttttttnaccactatcaacttcttgcaaaactaggggtgggcgttcggttcttcggttcagttcgggtcggttctttcggttctcggttctcggttctttcggttcctgnnnnnnnnnnnnnnnnnnnnnnnnnnnnnnnnnnnnnn

SEQ ID NO: 133 - DNA, 801 bp, Brassica napus
  misc_feature (43)..(43): n is a, c, g, or t
  misc_feature (214)..(214): n is a, c, g, or t
  misc_feature (556)..(556): n is a, c, g, or t
  misc_feature (719)..(719): n is a, c, g, or t
acttccgtgtggcaataagcgctcggaaaaagtttgcttttancaacggatctataccaaaacctgcacgactcacccgaccttgaagattggatagctaacaatcacctactggtgaattggatcaaactaacaatcgaaccaaaacttcgatcgaatatctctcacaaagaaatcactcgagacctctgggaccacatcaaaaagcgatttnctcttaaaagtggagctcgttaccaacaactacgagcttccctggcaacttgtcgacatgtgggatctacggtcgaagactactttggacgcttgacaagaatctgggattctatggctaaatgtatgtcaaccaagacatgtgactgcggaaagtgtgaatgcaacttggtcagcactcatgaaayagagcgcgagatcattcgtgctcatgatttcctatatggtgttcaatttcaattaatttagaggacacttccaaaattctgagcttccccggagtttggctgtgatccctacatctggaaaccaaagcatacttagtctcaacaatctaacacanaatgaaaaatgtattaaagtaaatgcactttgtaagaaacaggggactgttatatatttaagtgaatgggtgcaatattatatatgaaccattgcaattgtttatatgaacaattgcaactatataatgaaaccttgcaaccattaatgattgcaacatttgntaattaaccatattgataattgcaacccttggtgattaaccattgcaacttttggtttaaccattgcaactattggttgcaa

SEQ ID NO: 134 - DNA, 801 bp, Brassica napus
  misc_feature (30)..(30): n is a, c, g, or t
  misc_feature (101)..(101): n is a, c, g, or t
  misc_feature (426)..(426): n is a, c, g, or t
  misc_feature (651)..(651): n is a, c, g, or t
tgaatttgttcaccagaaatatattaaacnagattactgaaccaggtttaaccaggtcaaaccatattgaaccgtgacccaaaaattatccggttcagctnccggtccggttttaaaaacactgtccaaaactgattaataacgagtttcagattgttattaataacgatatctaatgtttgccagcagaggacttctgtatatcacggtgatctttatttatttttaagaatattttcatgcgactgcttacttagttatataaaatatcgaagtcgaagaccatataagattttttttttggccaacaataactaatctgctacgaaatactcaccgattcggaatgatcatataagatcaaacttcaaagtatggtgatatgttaatgtctgcactawatctatccgcttattttattaacgntttaacctaaaatatttaaaaactataaagtcttgcatccgtaattacccagctaaattcatgaaattgaatttgattaaagtctttaattatttgaatagtcttaaaagatggtacatagctgatgtaaaaaagcgcgttcttgaagagaacaggaagtcgtacaagcttttagtcaaaaaaaaaaagtcgtacaagcttaatacttcaatgtttttttattcncgagacggttgattatgtctgcttaaaactatatatatactcactgctggtcaagacaagaacaacaacgaaacaatgacaaagattcttctaagcttgctccatatacttttatgtgtgtctttacatggtgtggcagaggctagtttc

SEQ ID NO: 135 - DNA, 801 bp, Brassica napus
  misc_feature (5)..(5): n is a, c, g, or t
  misc_feature (96)..(195): n is a, c, g, or t
  misc_feature (262)..(262): n is a, c, g, or t
  misc_feature (295)..(295): n is a, c, g, or t
  misc_feature (328)..(328): n is a, c, g, or t
  misc_feature (414)..(414): n is a, c, g, or t
  misc_feature (417)..(417): n is a, c, g, or t
gactngtaaaagcctgcccggagaatgtttttgacattgaagacatgggcaatggtaaaagtaaaatccttcctttaaacaataggagaggatgcnnnnnnnnnnnnnnnnnnnnnnnnnnnnnnnnnnnnnnnnnnnnnnnnnnnnnnnnnnnnnnnnnnnnnnnnnnnnnnnnnnnnnnnnnnnnnnnnnnnngaatgtctgtaacaagcttgggtttattgatggaacggtgattcaaccggcgtctacttaccgtgantatggtgcttggtctcgttgcaatgatatggtngcaatatggctgatgaactctgtatccaagaanattggtcagagcttgttattcatcaataccgctgaaggtatatcgaagaatctcttggctcgtttcaaaccgratgatgcaccganggnttttgatattaaacaaaagctgagtaagactgaacaaggttcaatggatgtatcaacatattatactgaacttgtgactttgtgggaagagcaccgacccgcgaacgagtcggtcgctacctagcgaccgaccaaacctttcgttcggtcgatacgtagcgaccgatccagcgcggaccaggtcgctacgtagcgaccgaactatctcggacatcgatcaacgggtacgacccaaatctgtgcattctcgtttattcatcaatgctatctcccatgtaccgcatccatatcatttctcagatcattccgatcaaagttaccgttgaaactttacgataaaaaccgcgagaacttgtttttgtcgaaaagaaaatcgtaacaaac

SEQ ID NO: 136 - DNA, 401 bp, Brassica napus
ttactattttggtttattgatactttgattcaaaattttagtagttcggtttaatttttttttaattagaattgaaataattagggttttgtgcctttagttaacaatctatcgacagcccctctggaaggaaaaaagcaaccaaagaagtgtttgatataacttatttttattcgtactttttgttttttaacttgaacwatatggacgatatgattttaagtcttcccatggattgatggaggagattctctcaagggttccggtgaaatctattggagcagtacgatcaacttgtagaaactggaacgctttatctaaagatcaaagttttgtcaataagcatattgacaaagcagcagcatcatcaagagaaacggaggttcatgtgatcacggtga

SEQ ID NO: 137 - DNA, 401 bp, Brassica napus
tttggtggttgtttggaattgaatcgtgtgtaataaatggttaggttagtgttagattatggttggtgttagtaataaatagaagtgatgaatgagttagataaaggtctagtatatttgttgggttatgaattcactcgatggttgttagatatatgtctagtcctaagtatatttattatcatatattcaacgttcacmatctctactcggttaaacacaaaagtcttcctcttgttcttctcttccatcaaaacaccttcgttcatcttcttcttctctttttctcatatttcacacactagaatatggattataatccataaacgagtggggaaaattttgttgctctttttcaaagtcaacaacaaagtgtcttcggttcatcacaagttcctttt

SEQ ID NO: 138 - DNA, 801 bp, Brassica napus
  misc_feature (16)..(16): n is a, c, g, or t
  misc_feature (525)..(525): n is a, c, g, or t
  misc_feature (563)..(563): n is a, c, g, or t
  misc_feature (595)..(595): n is a, c, g, or t
  misc_feature (768)..(768): n is a, c, g, or t
  misc_feature (785)..(785): n is a, c, g, or t
aaagtttcaccgccanacgaatgagtttgaatggccaggagccccgatacgggatggcccctagtaccagccagattcgaccaatcacgagccagaggtggtgccggttaagcggggacagggtcgtcccaggaaggataagccggcgcccggcatagagtgggtccctgagccacctgtataggagccacccaagaagaaaagggggcgtccgcgcaaggccgctgcccccaaggaagacgcttcaaaaaagagtttggaatcgtgtgggagtgatgtcacggtcccaaagtcttgctcagtgggtgaatacttggaggggttcctgaatacgactaaggggtgcgcacccaagctcgtataagtgtggtgccaattgtttaaggcagggatccgcaagracattcggggggagccggagagcgccaaggatcccctggagttcttgctgatgaaaaggatagtcgggcaaacaataaccgcaggggagtggatcgtggggttgggcgaagaggatcgaagatncgcacttcgtcagacagaggagaacccagagccgaganatgatgacctaggacctacacctcgcgatgcngggatggttggtttaggaccggaggccgaccgtgtatttccacatccttgtggctagttgaggctttatgatcacttcgtaggagtaggacgtgagcttttctattggatttattctaactattgagtggttgctttggtgttgtttctccatttctaaaggcattttgtgtntgtacatatgccttgancttttcaaattattgt

SEQ ID NO: 139 - DNA, 401 bp, Brassica napus
aaaccggagttccaaacatagacaacagaagctcggctccagcgtaaaatccaaactacagaggccatgggagatcttcttacagaggcagaggaggctacacctccagaggaagaggctttattcaacatcagtcacaaccaacatcctctggagagcgtcttgtttgccaaatctgtggtcgcactggttatacagctmtgaagtgctacaacagattcaacaacaactaccaaagtaatgaagcttatacggttgttcgtgttgctgatgaacacggaagagaatggtaccctgattctggttcctcagttcatgtcacctcgtcgactcagaatctacaaacctcccacccctacgaagctcatgatgctgtcatggtgggagatggagctttcctt

SEQ ID NO: 140 - DNA, 401 bp, Brassica napus
acgaacttatcatacaagatgattcggaaatagtatcacactcacgagggtcatggaaatcaaaaatataatggtcgagatccgagaactacatataattaacgtggatgagttgctcaaaagcatatgtacagcttgcaacgaacaaaataaaagatggagatgtaacattttatagagataaaataaaaggctgaatcmgtttttcagaaattggaagggcttaaaagaaagtacagacagatcgagactggtttctttatgtgcggcagatccaaacactgtggtcgccattaaacaatctttgtaataatcgcaagttcacaacatttacacataaatttccacattatcaaagaattaattagatgttgagaaaagaaaatcaaagtactaattaa

SEQ ID NO: 141 - DNA, 151 bp, Brassica napus
  misc_feature (98)..(98): n is a, c, g, or t
tacctcaaacttgaagaatccatcaagaacatcaagaaggagtggtttgctacctccgtttctgttgagctcatakccactgttgctactaaagtcgngtaactcagacttccatgaatcttttgccttttgcataggtttccagaatgtt

SEQ ID NO: 142 - DNA, 496 bp, Brassica napus
  misc_feature (160)..(160): n is a, c, g, or t
  misc_feature (240)..(240): n is a, c, g, or t
cacattaatggagtcatgccggaagccttgatttcactccacagccaaatacttcctcttctccaacatgaaatcatgtttcttgatgaactagaatgcaatatcgacatctactggagggtgtgtttgcatatgttgatcctgttcgtacagtgttcantggcagaacaacaatttctttgtggcgatgttgttggacggctcatgttggatcgtggggttttgatagcttttctttcnacgaaaaaggsaaaacaaaatatttgtggcgaccatgggtttatgaattcttcatggttcttcttcaaacattctcagttgagtggcagttcatacttttctattggagagttggagacgttgctcaagagttggattgttatagtaatggtgcttgcgaatctaacaacgtgttgtgcattctggtttcgaatattgtaccaaaacctgtttggaagtgcatgtctttgagtacagctggcaagaaggtcgtgat

SEQ ID NO: 143 - DNA, 801 bp, Brassica napus
  misc_feature (24)..(24): n is a, c, g, or t
  misc_feature (262)..(262): n is a, c, g, or t
  misc_feature (347)..(347): n is a, c, g, or t
  misc_feature (356)..(356): n is a, c, g, or t
  misc_feature (518)..(518): n is a, c, g, or t
  misc_feature (778)..(778): n is a, c, g, or t
  misc_feature (790)..(790): n is a, c, g, or t
tctgtgagctcttcattgtcaacnacccagacataggtgtcctcaattgttgatagagagggtagttgcagataagtcaaatatataaggagttcctcagccgcctctgatcgagcaccagggaatatccaaccagctctgttgcaagcgtcagagactgttgctgtgtttgggatttgaagttcccttggggccaagatccccaaacctgtgaaagagcggtcctagcggtgtccaacaatcatgccagaagcttatgacnctgccatttcccagatttccatgttgaggaggaagcgttgttttcatcaacagcccatagattttcacccttcagtctgtattcncgagtccantctgcccaaagtgaatcagtattcaaaaatagtttccataaaagsttcaggcagagagttctgtgacatatcctcttgcacaaatttaggccctgtgcaagctaattccttacgtttggaagaagcaagaaagtggttcagcccaggattgaaatgcctaantaataaaaatttgagaagagagacttcactatgacatatcctcttgtgtaaacaggggggattgcaagagcagatttgaagcgagaaagatttgttgctaggaatagccaagaatctgcttcagaaaacaatagattgaacaaaatcattttgaatctgagatcaaatgaaatttaaagaaaaaacataagtcacattagactcaactgaagctctctaggcaggtatatatagtcatgaaatatattactttttgtctnttaatatatagncttcgaaagtg

SEQ ID NO: 144 - DNA, 801 bp, Brassica napus
  misc_feature (549)..(549): n is a, c, g, or t
taaacacaacaaagatcacaaaaatatgctgaaaaacagaatataattaaatcacatcgtaaactggtagcaaatataaatatgcaatttcaaaaccatttgctataaattagaaatgtaaataaagcttaaataaacataacaatatcagataaagcattttctaattagagtactaaaatccatttaatcaaattactttcacagggagataattagataagaagataacaaacttgtgaccaaaactagacgcgagacaagatttcttagaatctactgtcaataccattcaatagcgatcctacagctgcaaatacaaatcgtctaattaactagaacaaaacaaaagaaggtttgaatcgagcattaatgacttaccatccttcaatcaaaccagsgttactactctgcttctgatgttcctgaggctgtgggtattgcggtgcatacggaggtggatagccttgctgaggatatccctgcggtggtggataacattgttgaggatagggttgttgttgtgccggaggattttctggaggcgtnggagaagcgtccttagggttagggtgtccatctgacggattacctgttcaaccataatatgaaataaactaatcagaagaaaaaacgattagaagttaggatggaacatttaaattgaccccctccccccccccccccaaaagagttattatatgatatatagatgtcatgacacctaattatcaaaaaaattaatttatataagcctaaaaatgtttatgatctatgacaacaatacttatatctgtcttg

SEQ ID NO: 145 - DNA, 801 bp, Brassica napus
  misc_feature (10)..(10): n is a, c, g, or t
  misc_feature (133)..(133): n is a, c, g, or t
  misc_feature (324)..(324): n is a, c, g, or t
  misc_feature (489)..(489): n is a, c, g, or t
  misc_feature (724)..(724): n is a, c, g, or t
ttaaattaanaattaacctttcttttatggaaaaactgtcctggtcgaacttgggagactttttgagttcgcctagaatgggtgagaggtaaagaacatgattggtttgtaacgaatgaaaataattgatttngaaagaaaaaaacatagttatatatgatctttgggaattttaaatgttagactgtggcctaccaatatgtagtattaaagtttaattggttaaagatgctttaggtacattatgcatcctctgtataaaatgtttatcagttgcacctaagccggacgtatgtggattttcgttcacattaacaagtaaantgaataagccattacttgtatcgaccgtgttaagctgtaaatcgataacaaactaaaacgttttttttattatgaargtcatgcaagtgagatacatttcttcactactagttacttattttaagagaccagtttcaaacattccaccaagcttttccattagtnatatatattgtccaaaaacactaacaatcacccaccaaaataattttatatttccatctaaatctacctttactatatacattcatggacgaattagtttggagttaaaatcctaatcgtaccaccacattttcccaagcataaataaacaacgaacgaagttgatgctactttgtggtaaaccagtggtaagagttgatttgaattaaagcgaaaatccatcgattctgtattnaagttttggtaaaacgaaattactgtcaatcagacgaagatgggattatactttagacctcgttaaaaatctgtacc

SEQ ID NO: 146 - DNA, 723 bp, Brassica napus
  misc_feature (308)..(308): n is a, c, g, or t
  misc_feature (333)..(333): n is a, c, g, or t
  misc_feature (335)..(335): n is a, c, g, or t
  misc_feature (351)..(351): n is a, c, g, or t
  misc_feature (354)..(354): n is a, c, g, or t
  misc_feature (430)..(430): n is a, c, g, or t
tttttttttttttttttttttttttttttgaaaattaattattcgtgaccattttattttgaaacaaaagaacgacagagacataacgagattacatttattacaagcgaaaatactactagtctactactacaaaacatctataacaacaatataacatgggaataacaaaatggtagtaaaaagaataataagccgagccaccaagtaaaccaagcttctstcgcttacacaagaatctcaacacgccatctgaacatttcctccctcgtcacaggtaggttcaacgtcacaagcccaacctccgngtcgtagttgaactcagtctcggtncnatcaacagcgcatctnagnggacgctgagaagagtaagccccaaaacgaccacaacctctaacacctagagatatcagagctgttggagaacggntttcgctgaccactgaagaagaagagagctcaggtttctcgtctgtcacggtattgatctccatggactggatagctccacttgagttgaacatgtccaggagtccaataggtgcgaatgagatgcttgcagtgatttcctttagaggagagatgtggaagagttcatattcaagaaccttgagagtgagtgggattgatgcaccctttggtagtctaaccagctcccctgatttgtaagcgtagactattgaatctccactccagtcttcaccagccacttcagagatgaga

SEQ ID NO: 147 - DNA, 801 bp, Brassica napus
  misc_feature (373)..(373): n is a, c, g, or t
  misc_feature (497)..(497): n is a, c, g, or t
  misc_feature (560)..(560): n is a, c, g, or t
  misc_feature (605)..(605): n is a, c, g, or t
  misc_feature (640)..(640): n is a, c, g, or t
  misc_feature (679)..(679): n is a, c, g, or t
  misc_feature (755)..(755): n is a, c, g, or t
gctttttgtgaaatgaatggttggctggtttttgcaagtcatgcttctgaagataaccttgctttcattaggtagccgcgaatcacccctcttggacattgtggcatatgcaggctatgctttcactggtctcttcttggcaagatcatttggggatattcttactatgttttgattccgtggacttgcttatgcaccggagttctcttggtgaagacaatgaagcgagttctctttgcagaagctaggagttatgactcaagcagaaaatcattacctcttgattttttagcattagcacagtttcctcttttgatctggcttggtaacattagtgtcgattggctcttttgagattcattagttgtgaatnaaaagaacacttatgatgttatgagatstacgatactcctgatgaagtagtacacctctctcttttcataacttctttttaatgtcaattttttttgcatagactacatttccaacatgatttnaaaccaaacaaggacatgaactttggtcatatagtattattatctatactccaagccctcctnttgcattgcattggtgcattgtgatactccttggcagatggttcnttttaaacctgaatgaaagacatggaaccctttcntttaaagatagtattcttatacaaagaaaaagaagaagnaggtcgtcgtgttgaacctaattaggatctaatatgcttcccatctttgtagcgttgttgataagttacatcaaancaaatattgaccgacctcaaaaactagttttaaatcattttcactt

SEQ ID NO: 148 - DNA, 656 bp, Brassica napus
  misc_feature (83)..(83): n is a, c, g, or t
  misc_feature (86)..(86): n is a, c, g, or t
  misc_feature (100)..(100): n is a, c, g, or t
  misc_feature (189)..(189): n is a, c, g, or t
  misc_feature (216)..(217): n is a, c, g, or t
  misc_feature (251)..(251): n is a, c, g, or t
  misc_feature (256)..(256): n is a, c, g, or t
  misc_feature (338)..(338): n is a, c, g, or t
  misc_feature (347)..(347): n is a, c, g, or t
  misc_feature (353)..(353): n is a, c, g, or t
  misc_feature (407)..(407): n is a, c, g, or t
  misc_feature (409)..(409): n is a, c, g, or t
  misc_feature (413)..(413): n is a, c, g, or t
  misc_feature (432)..(432): n is a, c, g, or t
  misc_feature (434)..(434): n is a, c, g, or t
  misc_feature (467)..(467): n is a, c, g, or t
  misc_feature (476)..(476): n is a, c, g, or t
  misc_feature (500)..(500): n is a, c, g, or t
  misc_feature (528)..(528): n is a, c, g, or t
  misc_feature (548)..(548): n is a, c, g, or t
  misc_feature (556)..(556): n is a, c, g, or t
  misc_feature (606)..(606): n is a, c, g, or t
  misc_feature (626)..(626): n is a, c, g, or t
  misc_feature (635)..(635): n is a, c, g, or t
  misc_feature (641)..(641): n is a, c, g, or t
  misc_feature (653)..(653): n is a, c, g, or t
cgctgtaacttctcaagagtttctcgctaacatcaccgttgctttctcctttagccactctcctaagcttcaagagagactcngcnagagaaccctccantgcatttcctccaagtttcaaactttgctcggttttaacctcgttgttcttcgctktatcacctttcctctgaatcaacccccaaagantccatcctttcccccatttctttccanncttcttcaaaccaaaaccatcctgcttcacctcnccacnaccagcaacacaaactacgcctttggaagctaactctaagctctccggtttgtagtttttgatggaataccaattcgaatcnctcagttcnctctcngtaacaagcaacttagctccatgaaacaaaccaacaccttcaggtgacaacttngntttnacatccaccaatccatgcntngatgaccgatcaaagcttcttctccgccgtgantccaagtantaatccctcgtctgagctgtcccncctggcttcttctccggcgaggctttancatcttcggtcacggatganaaaggtancagctttggatacgtcttcccgatcaagcatccgtcccatgacgctctangctcctcgaaagagactcgncacaacctnggatcnacatcacatgancga

SEQ ID NO: 149 - DNA, 801 bp, Brassica napus
  misc_feature (285)..(285): n is a, c, g, or t
  misc_feature (429)..(429): n is a, c, g, or t
  misc_feature (549)..(549): n is a, c, g, or t
  misc_feature (595)..(595): n is a, c, g, or t
  misc_feature (661)..(661): n is a, c, g, or t
  misc_feature (666)..(666): n is a, c, g, or t
  misc_feature (721)..(721): n is a, c, g, or t
  misc_feature (764)..(764): n is a, c, g, or t
atatttaattattatatatatggagtaaaagtataagagtctttttcctcttaatgaagtagatatttttgaaaatatttatttagtgatgataaacatgaataatgatacgagcaaagtgttaaacatgaaaattccccttaaatattctctttgttttacaaagtattattattattttgacatatttttttgttacacaaagaatatcattttagaatttaagtgtgatttatatttattttaaacttaatctttatttctaaatgcattgattttataaantattttacttatctcaaatatgatttgttagataaatatgattaataaaaatataatttttttgtttgaataacctgaaggtttcctcgtggaatgactccgattaatccctaagmagagaagtaacccaaaaataaactattncttcgtgtatttaaatagaccgcaaggacccatatctatataggtgtctaggataatgtaacttaatttcacacataagatatatcgaatttgaaatgtgttggcattctaattcatttntcctcgtcactcgaccacacaaaaacataaatattcaaatcatatntttaaccggtgtgagaattaaaattgagaaattgccacaaataccacattcatagtaccacttttnatgtntacactaatcacttttatcctcaattttaataaagggtaaaagacatttataccnctatggttaactaatctaaacttagggtttagagttgagaganggtaggttttttggcatctgaaatttaggattctaat

SEQ ID NO: 150 - DNA, 121 bp, Brassica napus
  misc_feature (87)..(87): n is a, c, g, or t
  misc_feature (97)..(97): n is a, c, g, or t
aatacgtctacaatttcattagtctcaagaaaaacaatataaaaacaaaataaatagccarattacatcccaaattcatcaagtagncttgagtggngccccaatccaattatccagaagc

SEQ ID NO: 151 - DNA, 801 bp, Brassica napus
  misc_feature (26)..(26): n is a, c, g, or t
  misc_feature (64)..(64): n is a, c, g, or t
  misc_feature (197)..(197): n is a, c, g, or t
  misc_feature (283)..(283): n is a, c, g, or t
  misc_feature (463)..(463): n is a, c, g, or t
  misc_feature (487)..(487): n is a, c, g, or t
  misc_feature (602)..(603): n is a, c, g, or t
  misc_feature (632)..(632): n is a, c, g, or t
tgtgttttgcttgtgcaaatgtgcanctttgagtctgtgtgatggacctttagggtttgataangggaagggaaagatggtagatgcaggggtgttgcaggacagccaaggagcaagggcttatgaaggttcttcccaacttcatggcaggtttgcgcatgggggaaaactgaccatcgcagaatgtacggccatgnataatttgtgaaatttcatgcatcttcagtcaataaattcccgtaactgtcattacaacttactgtactgggacatcagttggccntcttctactcggcttcatgagtataagtatgagtttgttgagatctcgtcagaatacgctgaagagttgccaataacgattgcgtttttgcgtgaagtcaaaggctttgcaagtgtcwttcatgactggtggtggtggtagatcaaacacgtttcagtatgagttgcttagattctctcncagcatcccttcaactaaattganagggaaagaaaggaactgtgttcctgttggttcttatgagcttgatacagctgcgttaccacaaatgatagaagatggtgaagaggaagactggtgatatttgggcaatgtacannaactggaggaatgaaatcagggtagggancttgaagaagtgtgcttacgaggttgttgatgttggagtgggtggacgggtttgtatattgtgcaaagtctctagcttttaatgttttagattcagacattaacttgcatcggatctgtcttttgactctagttttagtcaatctggtgaaatgttcttttacctcttc

SEQ ID NO: 152 - DNA, 688 bp, Brassica napus
  misc_feature (29)..(29): n is a, c, g, or t
  misc_feature (89)..(89): n is a, c, g, or t
  misc_feature (209)..(209): n is a, c, g, or t
  misc_feature (221)..(221): n is a, c, g, or t
  misc_feature (265)..(265): n is a, c, g, or t
  misc_feature (269)..(269): n is a, c, g, or t
  misc_feature (404)..(404): n is a, c, g, or t
  misc_feature (656)..(656): n is a, c, g, or t
  misc_feature (659)..(659): n is a, c, g, or t
gaccgacggcgttcttcaagagcttaggnggacaggtggacatcgtcaaagacgggaagccttacgtgatgttcggagacgggaagctntgcgcttgcaagcccatcagcgaggaggatttagcttcgttcatagcggactgtgtcttggaagaggataagatcaataaggttttgcctatcggtggaccggggaaggccttgacgccnttggagcaaggngagattctgtttaggatacttgggagagagcctaagtttctganagtncctattgagattatggactttgtgattggggtkcttgatggtgtggcgaaggtgtttcctagtgttgcggaggctgctgagtttgggaagattgggaggtattatgctgcggagagtatgttgattcttgatccngagactggggagtatagtgaggagaagactccgagctatgggaaggatactcttgaggacttctttgagaaagtggttagagaagggatggctggtcaagagcttggtgaacagttcttctagtggggagaagtttttatgctaatgagtttgagctgtgttgagtgttgttagctgttgagattataaaaactgtgaatttgagagatttgttgatccaaaaaaaacagttataaaacacatatttcacangtncaaaaaaaaaaaaaaaaaaaaaaaaaaaa

SEQ ID NO: 153 - DNA, 706 bp, Brassica napus
  misc_feature (247)..(248): n is a, c, g, or t
  misc_feature (334)..(334): n is a, c, g, or t
  misc_feature (350)..(350): n is a, c, g, or t
  misc_feature (354)..(354): n is a, c, g, or t
  misc_feature (373)..(373): n is a, c, g, or t
  misc_feature (433)..(433): n is a, c, g, or t
  misc_feature (435)..(435): n is a, c, g, or t
  misc_feature (455)..(455): n is a, c, g, or t
  misc_feature (572)..(572): n is a, c, g, or t
  misc_feature (581)..(581): n is a, c, g, or t
  misc_feature (639)..(639): n is a, c, g, or t
gaaacaatatgttcatctacatttacacttccatttgttttgagatagtaatctcttcaaaactggaaaagcattgtcgctactgttagacaccagaatgggaccgatatataagttagatgactcaaagaaacaacacttagacgacaagttgcacaacaaagacctataataagaatgcattttcgaggggtgttctaaaaatgtgaaccaagaagcgtgatctgatataagtagacataaattnnacctcaagcgtcgaccgagatgaggaggaggttgatgaagaaagcttatcggcaccagatatagcgctgattatgatgatgctganggcaaagcgtaaaacncttntggaggatccctttgatangcaaagtccatatacagaatctctaacttggagtgaagcgattgagcatctctcaactcnanatctcgaattagagacatanccaagtgccagtgattccatcaccactgaaacagatgtgttcccargacaaaacccaagcataacatcatagtggaaatgcaaaacccacagtaatagttacaagagagaaacagcntttttgcancccccggatggtgcatagccacggctcaacatttctttgataagctcggccgataagnttatatcaccatctctaagacatagcgtgccatcattcagcataagcccatctcctttcatctttgt

SEQ ID NO: 154 - DNA, 801 bp, Brassica napus
  misc_feature (117)..(117): n is a, c, g, or t
  misc_feature (124)..(124): n is a, c, g, or t
  misc_feature (300)..(300): n is a, c, g, or t
  misc_feature (461)..(461): n is a, c, g, or t
  misc_feature (598)..(598): n is a, c, g, or t
  misc_feature (761)..(801): n is a, c, g, or t
tagacgtaataaatgtagatctgttgaggttctttttatatatattttccgtatttggtcggtctttgagatgagtttgtttaagaaaaacgtaaaatgaagttgcttggggtctangtgattncctgattggcacgaagagcgacgcatccccgaagcgcggcactctccacgtgctcttgtgatccactaaacaagcccatactaatataaagtcatcttaaaaccgacgctgcataatctttaggttcatgcacattcttgaatagatttcgaggaacatactgtagttaatatttnagcctggaccagaaataatatactcggattgcatctcaataaagagtattaaaaaacaaaaacaaaaacaaaatcattctgagactttgaaacgaaaaagyaattagtttattgagcgcggggaagagtatatacattattaaacatacatctctcacttncttttctatacggcgagttcatcttcaagataactgtattcaaacgtgaactcgtttttgatcctttgaaccctacacagagttttcataaagaaaaaagattaggatcatcacctcgaacgacaaagagaacaagnagacgagaaatcgatagatcataccatcctccttcttggctctcatctttgggggtttggaaatcaaagtaaacataggctccttgttcatactcatcagttgcaatctttggctccttgtgtctctgaaaccatgtgttgaactttctgtggtatctccacnnnnnnnnnnnnnnnnnnnnnnnnnnnnnnnnnnnnnnnnn

SEQ ID NO: 155 - DNA, 496 bp, Brassica napus
  misc_feature (383)..(383): n is a, c, g, or t
  misc_feature (439)..(439): n is a, c, g, or t
  misc_feature (455)..(455): n is a, c, g, or t
  misc_feature (463)..(463): n is a, c, g, or t
  misc_feature (466)..(466): n is a, c, g, or t
cttgttctcgctgagactgtctttcttttctaggaagaagacgctaataccgcggagccgccacctcctcttccttgccgatacaggtctctgcggagcctgtttaaaacttgtcctctactcggctgtttcctgaaagttgagcaaaatcgcagccactgctgctacggccattttcagttggcacgagaatttgcccaacgagctgtggcttttcattacttcgacggattccttgatggagaacatcraaagagggtttgtatcttggctctgctgaacagtgtccgaggcttacaaacaggtgttccaaatctggatcacgttgctggattattcaccacacttccttggcagctaaagatcataccagaaaatgcagnaaattggctatttttcaagacacccccactacgctacacatcgatgagctacacancgacgaactgtggcantaagccgncgnccatctggtggaaaaaaaatccattcctaa

SEQ ID NO: 156 - DNA, 801 bp, Brassica napus
  misc_feature (5)..(5): n is a, c, g, or t
  misc_feature (181)..(181): n is a, c, g, or t
  misc_feature (215)..(215): n is a, c, g, or t
  misc_feature (263)..(263): n is a, c, g, or t
  misc_feature (279)..(279): n is a, c, g, or t
  misc_feature (331)..(331): n is a, c, g, or t
  misc_feature (423)..(423): n is a, c, g, or t
  misc_feature (446)..(446): n is a, c, g, or t
  misc_feature (462)..(462): n is a, c, g, or t
ttctntgcaatatgggaagttgtatctctctctcgctatcatgtgatcagtgtacgaatcaagtctttcagtggttatgcatcagaaggggttatattcacaatctcgaggagaatctcaaggctttggagacaaccatggaggagcttcaggcaaatcgggatgatttgtcaaaaagggnggagagagaggagggtaaaggactaaaaaggctntcccaaatccaggtatggcttacgagagtcgacacaatcaaaacacangtgaatgctatatttngtgcaatacctgttggaagtcaaaggttgtctctctgtgggttttgctctangaatttaaaatctagatatcgttacgggaaaagggtttttctgatgttgaaggaggttgagaatctaaaytctggtggagactttgaagtcnttgccgagcaagctcaagcatcngaggtagaggagcggnctatccaaccgggaattgttggtcgggacacgatgctcaaaaaggcatgggtgtagaagaatttagcttaggttacttaggtttcaagttagccttagaacagtaaatacataatcaatttaacgagttcccggccctcggcacggtacgtctcgtgggagaacttctgctcccaaacttgactagatcaaaagagtcaccagccacaccaaataagtgtgctagttagtttacaatgaaccaaatactccaagctagagaatacaacaagcccttagataatagacttaagcctaagctagttatcttgtatgttgtcttctttctcttgctaatctc

SEQ ID NO: 157 - DNA, 24 bp, Artificial sequence
  primer
acgtcggtactcttttctgttgtc

SEQ ID NO: 158 - DNA, 25 bp, Artificial sequence
  primer
cccttactctaggatgggtgataca

SEQ ID NO: 159 - DNA, 18 bp, Artificial sequence
  probe
aactcaggaattaatgat

SEQ ID NO: 160 - DNA, 17 bp, Artificial sequence
  probe
actcaggaatgaatgat

SEQ ID NO: 161 - DNA, 20 bp, Artificial sequence
  primer
ttcggggattagagctttcc

SEQ ID NO: 162 - DNA, 22 bp, Artificial sequence
  primer
tcatcagtaccgtttgatttcg

SEQ ID NO: 163 - DNA, 17 bp, Artificial sequence
  probe
tcgatctctcactacgg

SEQ ID NO: 164 - DNA, 18 bp, Artificial sequence
  probe
tctctcactagggactac

SEQ ID NO: 165 - DNA, 32 bp, Artificial sequence
  primer
tagctattcataattaatcaaaaaggtggtcc

SEQ ID NO: 166 - DNA, 29 bp, Artificial sequence
  primer
gcagtatcatatgttccactctagagatg

SEQ ID NO: 167 - DNA, 22 bp, Artificial sequence
  probe
attttacaccttagtgctgtga

SEQ ID NO: 168 - DNA, 23 bp, Artificial sequence
  probe
aattttacaccttagtgctatga

SEQ ID NO: 169 - DNA, 25 bp, Artificial sequence
  primer
ccgcttagctctcttcggttatttt

SEQ ID NO: 170 - DNA, 25 bp, Artificial sequence
  primer
aacagcacatgacgagatgacatat

SEQ ID NO: 171 - DNA, 18 bp, Artificial sequence
  probe
ctgaatgtggtctatcac

SEQ ID NO: 172 - DNA, 18 bp, Artificial sequence
  probe
ctgaatgtggtttatcac

SEQ ID NO: 173 - DNA, 24 bp, Artificial sequence
  primer
aacaagccctctcatgtacaatgt

SEQ ID NO: 174 - DNA, 22 bp, Artificial sequence
  primer
accaccgctatgcatcaaatct

SEQ ID NO: 175 - DNA, 20 bp, Artificial sequence
  probe
actagttgattatgaagaaa

SEQ ID NO: 176 - DNA, 19 bp, Artificial sequence
  probe
ctagttgattgtgaagaaa

SEQ ID NO: 177 - DNA, 25 bp, Artificial sequence
  primer
ccgtacgatgaatcagacgaaagta

SEQ ID NO: 178 - DNA, 35 bp, Artificial sequence
  primer
gaaacgaataaattatagaacgaagctactaatgg

SEQ ID NO: 179 - DNA, 18 bp, Artificial sequence
  probe
aacagagagattaattgg

SEQ ID NO: 180 - DNA, 17 bp, Artificial sequence
  probe
acagagagatgaattgg

SEQ ID NO: 181 - DNA, 25 bp, Artificial sequence
  primer
tgatgcttcccttcaaagaaagaca

SEQ ID NO: 182 - DNA, 35 bp, Artificial sequence
  primer
acatgttaccaatcaaagcctatattacatttaca

SEQ ID NO: 183 - DNA, 15 bp, Artificial sequence
  probe
tttttgtgcaacttc

SEQ ID NO: 184 - DNA, 19 bp, Artificial sequence
  probe
cttgtttttgtacaacttc

SEQ ID NO: 185 - DNA, 21 bp, Artificial sequence
  primer
cccatcaaatgaaaaggagga

SEQ ID NO: 186 - DNA, 20 bp, Artificial sequence
  primer
ctatggcgatgttgctcaaa

SEQ ID NO: 187 - DNA, 15 bp, Artificial sequence
  probe
atggttccataactc

SEQ ID NO: 188 - DNA, 15 bp, Artificial sequence
  probe
catggttccgtaact

SEQ ID NO: 189 - DNA, 25 bp, Artificial sequence
  primer
cctctttgagctaacactagtcaca

SEQ ID NO: 190 - DNA, 24 bp, Artificial sequence
  primer
atccaagggacaaaatgctaccaa

SEQ ID NO: 191 - DNA, 15 bp, Artificial sequence
  probe
acccatggtggttct

SEQ ID NO: 192 - DNA, 18 bp, Artificial sequence
  probe
caaacccatgttggttct

SEQ ID NO: 193 - DNA, 20 bp, Artificial sequence
  primer
ttgcaaaactccaggtcaga

SEQ ID NO: 194 - DNA, 21 bp, Artificial sequence
  primer
aaagcttgtgtcgaagcaaat

SEQ ID NO: 195 - DNA, 17 bp, Artificial sequence
  probe
acgtacataacacgctt

SEQ ID NO: 196 - DNA, 15 bp, Artificial sequence
  probe
aacgtacacaacacg

SEQ ID NO: 197 - DNA, 22 bp, Artificial sequence
  primer
cacaataaaaccagagcttcca

SEQ ID NO: 198 - DNA, 20 bp, Artificial sequence
  primer
gcaacgaaccaaaaatcaca

SEQ ID NO: 199 - DNA, 19 bp, Artificial sequence
  probe
cttttccaaatgattacac

SEQ ID NO: 200 - DNA, 17 bp, Artificial sequence
  probe
cttttccagatgattac

SEQ ID NO: 201 - DNA, 25 bp, Artificial sequence
  primer
cacctgaccgaaagaaacactagtt

SEQ ID NO: 202 - DNA, 36 bp, Artificial sequence
  primer
tctttctgtaagaattattcttcatttagctatgct

SEQ ID NO: 203 - DNA, 23 bp, Artificial sequence
  probe
aagataaaattactgttattagc

SEQ ID NO: 204 - DNA, 23 bp, Artificial sequence
  probe
aagataaaattactgatattagc

SEQ ID NO: 205 - DNA, 22 bp, Artificial sequence
  primer
tcttttgttgaatggggatttt

SEQ ID NO: 206 - DNA, 26 bp, Artificial sequence
  primer
cgtcaaaagaaaatagaaaaagacag

SEQ ID NO: 207 - DNA, 16 bp, Artificial sequence
  probe
tccaacttccaaatta

SEQ ID NO: 208 - DNA, 17 bp, Artificial sequence
  probe
tccaacttccaaagtat

SEQ ID NO: 209 - DNA, 21 bp, Artificial sequence
  primer
aacgacatagacgatcgttgg

SEQ ID NO: 210 - DNA, 24 bp, Artificial sequence
  primer
tctccatcacttcgttagtattcg

SEQ ID NO: 211 - DNA, 17 bp, Artificial sequence
  probe
cacaagaatccacaact

SEQ ID NO: 212 - DNA, 17 bp, Artificial sequence
  probe
acacaagagtccacaac

SEQ ID NO: 213 - DNA, 27 bp, Artificial sequence
  primer
gagagaaagagtgggaaagaaaagagt

SEQ ID NO: 214 - DNA, 25 bp, Artificial sequence
  primer
gctctctgaagatgggaagaaatga

SEQ ID NO: 215 - DNA, 15 bp, Artificial sequence
  probe
ctccacgccttagct

SEQ ID NO: 216 - DNA, 16 bp, Artificial sequence
  probe
tctccacgctttagct

SEQ ID NO: 217 - DNA, 20 bp, Artificial sequence
  primer
acaatctggccacacagacg

SEQ ID NO: 218 - DNA, 30 bp, Artificial sequence
  primer
gttattcataaagccaaggttttcacttct

SEQ ID NO: 219 - DNA, 22 bp, Artificial sequence
  probe
agagaagaatcaactagaagta

SEQ ID NO: 220 - DNA, 20 bp, Artificial sequence
  probe
agaagaatcaacgagaagta

SEQ ID NO: 221 - DNA, 47 bp, Artificial sequence
  primer
gaaggtgaccaagttcatgctcaacaactagcaaatcaaaagtgacc

SEQ ID NO: 222 - DNA, 50 bp, Artificial sequence
  primer
gaaggtcggagtcaacggattgatcaacaactagcaaatcaaaagtgaca

SEQ ID NO: 223 - DNA, 29 bp, Artificial sequence
  primer
ggtggaataaagtgttctttgacgaactt

SEQ ID NO: 224 - DNA, 47 bp, Artificial sequence
  primer
gaaggtgaccaagttcatgctaatgtaaaggagaagaagaagagcac

SEQ ID NO: 225 - DNA, 47 bp, Artificial sequence
  primer
gaaggtcggagtcaacggattaatgtaaaggagaagaagaagagcag

SEQ ID NO: 226 - DNA, 24 bp, Artificial sequence
  primer
tcccaaccaattggtcgccagtaa

SEQ ID NO: 227 - DNA, 46 bp, Artificial sequence
  primer
gaaggtgaccaagttcatgctaacagatcattctaactcattgccg

SEQ ID NO: 228 - DNA, 48 bp, Artificial sequence
  primer
gaaggtcggagtcaacggattgtaacagatcattctaactcattgcca

SEQ ID NO: 229 - DNA, 25 bp, Artificial sequence
  primer
gaggtaatctacaccgccccttata

SEQ ID NO: 230 - DNA, 52 bp, Artificial sequence
  primer
gaaggtgaccaagttcatgctgtcgtgaaaaaataattttctatatttccaa

SEQ ID NO: 231 - DNA, 54 bp, Artificial sequence
  primer
gaaggtcggagtcaacggattctgtcgtgaaaaaataattttctatatttccat

SEQ ID NO: 232 - DNA, 30 bp, Artificial sequence
  primer
gtaccattttattgtaatgaactatctttt

SEQ ID NO: 233 - DNA, 47 bp, Artificial sequence
  primer
gaaggtgaccaagttcatgctgttgagctgatcttacaggtccatta

SEQ ID NO: 234 - DNA, 44 bp, Artificial sequence
  primer
gaaggtcggagtcaacggattgagctgatcttacaggtccattg

SEQ ID NO: 235 - DNA, 25 bp, Artificial sequence
  primer
tcagctccggtgaagaaaacagaga

SEQ ID NO: 236 - DNA, 53 bp, Artificial sequence
  primer
gaaggtgaccaagttcatgctttaaagtttacttttatacatcacgagattaa

SEQ ID NO: 237 - DNA, 44 bp, Artificial sequence; identical to SEQ ID NO: 234
  primer

SEQ ID NO: 238 - DNA, 30 bp, Artificial sequence
  primer
ctcaactagtttcttttaatttctgttgaa

SEQ ID NO: 239 - DNA, 51 bp, Artificial sequence
  primer
gaaggtgaccaagttcatgctgagataattcaaggtgattaagtgatattg

SEQ ID NO: 240 - DNA, 53 bp, Artificial sequence
  primer
gaaggtcggagtcaacggattatgagataattcaaggtgattaagtgatatta

SEQ ID NO: 241 - DNA, 29 bp, Artificial sequence
  primer
cagcccatttccaaaagtttttgggtttt

SEQ ID NO: 242 - DNA, 48 bp, Artificial sequence
  primer
gaaggtgaccaagttcatgctgaatcgatcagaatctaaacggttatg

SEQ ID NO: 243 - DNA, 49 bp, Artificial sequence
  primer
gaaggtcggagtcaacggattcgaatcgatcagaatctaaacggttatt

SEQ ID NO: 244 - DNA, 30 bp, Artificial sequence
  primer
gagatctgatcaaaattgactttgcactta

SEQ ID NO: 245 - DNA, 51 bp, Artificial sequence
  primer
gaaggtgaccaagttcatgctccaatatagaaaaaaacaaaacactcttcg

SEQ ID NO: 246 - DNA, 54 bp, Artificial sequence
  primer
gaaggtcggagtcaacggattaaaccaatatagaaaaaaacaaaacactcttca

SEQ ID NO: 247 - DNA, 29 bp, Artificial sequence
  primer
gttggaagctttaacggttatggaatgta

SEQ ID NO: 248 - DNA, 18 bp, Artificial sequence
  primer
caacgcgttgcccgaaaa

SEQ ID NO: 249 - DNA, 28 bp, Artificial sequence
  primer
ttgaagtactaaagtggatagcggaaaa

SEQ ID NO: 250 - DNA, 18 bp, Artificial sequence
  probe
tttaaagaaggaaaattc

SEQ ID NO: 251 - DNA, 21 bp, Artificial sequence
  probe
tgatttaaagaaagaaaattc

SEQ ID NO: 252 - DNA, 52 bp, Artificial sequence
  primer
gaaggtgaccaagttcatgcttttattttcttctggatacagataagaataa

SEQ ID NO: 253 - DNA, 51 bp, Artificial sequence
  primer
gaaggtcggagtcaacggattttattttcttctggatacagataagaatac

SEQ ID NO: 254 - DNA, 29 bp, Artificial sequence
  primer
ctcagacttcattgcaaagctgaatagaa

SEQ ID NO: 255 - DNA, 51 bp, Artificial sequence
  primer
gaaggtgaccaagttcatgctacaagtcatgtatttgtaacgacttgaaaa

SEQ ID NO: 256 - DNA, 50 bp, Artificial sequence
  primer
gaaggtcggagtcaacggattcaagtcatgtatttgtaacgacttgaaag

SEQ ID NO: 257 - DNA, 25 bp, Artificial sequence
  primer
ggagtccggactgaaatgcagatta

SEQ ID NO: 258 - DNA, 45 bp, Artificial sequence
  primer
gaaggtgaccaagttcatgctctgaagagctgatgtcttttggtg

SEQ ID NO: 259 - DNA, 45 bp, Artificial sequence
  primer
gaaggtcggagtcaacggattctgaagagctgatgtcttttggtt

SEQ ID NO: 260 - DNA, 30 bp, Artificial sequence
  primer
caatgtttctgaacagaaacttctcagttt

SEQ ID NO: 261 - DNA, 49 bp, Artificial sequence
  primer
gaaggtgaccaagttcatgctcaatagccttttaagagttttctaacca

SEQ ID NO: 262 - DNA, 49 bp, Artificial sequence
  primer
gaaggtcggagtcaacggattcaatagccttttaagagttttctaacct

SEQ ID NO: 263 - DNA, 29 bp, Artificial sequence
  primer
ccttttgtgttattaaaagcgggagtgtt

SEQ ID NO: 264 - DNA, 50 bp, Artificial sequence
  primer
gaaggtgaccaagttcatgctcctcaacagcctgaaaaatataacataat

SEQ ID NO: 265 - DNA, 50 bp, Artificial sequence
  primer
gaaggtcggagtcaacggattcctcaacagcctgaaaaatataacataac

SEQ ID NO: 266 - DNA, 29 bp, Artificial sequence
  primer
gtcccggatatataactgctgtatacata

SEQ ID NO: 267 - DNA, 45 bp, Artificial sequence
  primer
gaaggtgaccaagttcatgctcattgttgcgtatgacaagctcgt

SEQ ID NO: 268 - DNA, 41 bp, Artificial sequence
  primer
gaaggtcggagtcaacggattgttgcgtatgacaagctcgc

SEQ ID NO: 269 - DNA, 25 bp, Artificial sequence
  primer
ggtatcgttcgtgagagattggcta

SEQ ID NO: 270 - DNA, 54 bp, Artificial sequence
  primer
gaaggtgaccaagttcatgctcaataagacaaaaattcaaaacaagaaaaaatg

SEQ ID NO: 271 - DNA, 54 bp, Artificial sequence
  primer
gaaggtcggagtcaacggattcaataagacaaaaattcaaaacaagaaaaaata

SEQ ID NO: 272 - DNA, 30 bp, Artificial sequence
  primer
ggctttgtaaatttccgttttcaaacgttt

SEQ ID NO: 273 - DNA, 47 bp, Artificial sequence
  primer
gaaggtgaccaagttcatgctgattacacgcacaaattcgagaaatg

SEQ ID NO: 274 - DNA, 43 bp, Artificial sequence
  primer
gaaggtcggagtcaacggattacacgcacaaattcgagaaata

SEQ ID NO: 275 - DNA, 29 bp, Artificial sequence
  primer
atctcgctgatccagtttgttcttgattt

SEQ ID NO: 276 - DNA, 49 bp, Artificial sequence
  primer
gaaggtgaccaagttcatgcttggttcattttatttaatggacctttgc

SEQ ID NO: 277 - DNA, 51 bp, Artificial sequence
  primer
gaaggtcggagtcaacggattcttggttcattttatttaatggacctttga

SEQ ID NO: 278 - DNA, 30 bp, Artificial sequence
  primer
gaaccactgtgttaacaaaacaacaacgtt

SEQ ID NO: 279 - DNA, 47 bp, Artificial sequence
  primer
gaaggtgaccaagttcatgctcccattatcattgtgcaatttccgag

SEQ ID NO: 280 - DNA, 47 bp, Artificial sequence
  primer
gaaggtcggagtcaacggattcccattatcattgtgcaatttccgac

SEQ ID NO: 281 - DNA, 30 bp, Artificial sequence
  primer
cctttcttgcttctccagatacaatttgtt

SEQ ID NO: 282 - DNA, 44 bp, Artificial sequence
  primer
gaaggtgaccaagttcatgctgtttgatcctcagttcgctcgtc

SEQ ID NO: 283 - DNA, 44 bp, Artificial sequence
  primer
gaaggtcggagtcaacggattgtttgatcctcagttcgctcgtg

SEQ ID NO: 284 - DNA, 25 bp, Artificial sequence
  primer
tccccttccgatcctcatcatctta

SEQ ID NO: 285 - DNA, 21 bp, Artificial sequence
  primer
ttcttccatcgtctctcctga

SEQ ID NO: 286 - DNA, 22 bp, Artificial sequence
  primer
tgcaattcagtgtttcgatttt

SEQ ID NO: 287 - DNA, 15 bp, Artificial sequence
  probe
ctcccacctatcaaa

SEQ ID NO: 288 - DNA, 15 bp, Artificial sequence
  probe
ctcccagctatcaaa

SEQ ID NO: 289 - DNA, 27 bp, Artificial sequence
  primer
acttaaagacctctccttactctccaa

SEQ ID NO: 290 - DNA, 29 bp, Artificial sequence
  primer
gctggtaattgaaaaggattgatctttga

SEQ ID NO: 291 - DNA, 17 bp, Artificial sequence
  probe
caagccaaagtcttaac

SEQ ID NO: 292 - DNA, 17 bp, Artificial sequence
  probe
caagccaaagacttaac

SEQ ID NO: 293 - DNA, 18 bp, Artificial sequence
  primer
ctcgtctccgttggtggt

SEQ ID NO: 294 - DNA, 20 bp, Artificial sequence
  primer
ggcaaccctttcaaaacaga

SEQ ID NO: 295 - DNA, 15 bp, Artificial sequence
  probe
acaggtctcctccac

SEQ ID NO: 296 - DNA, 13 bp, Artificial sequence
  probe
acaggtcgcctcc

SEQ ID NO: 297 - DNA, 22 bp, Artificial sequence
  primer
ggaaagttgaatttgattcgcc

SEQ ID NO: 298 - DNA, 23 bp, Artificial sequence
  primer
cattcctcaacaacaacccctaa

SEQ ID NO: 299 - DNA, 17 bp, Artificial sequence
  probe
cttgatcatcacaaaac

SEQ ID NO: 300 - DNA, 17 bp, Artificial sequence
  probe
tcacgaaactcgactgg

SEQ ID NO: 301 - DNA, 27 bp, Artificial sequence
  primer
tcctgtacacacaaattcaagacatca

SEQ ID NO: 302 - DNA, 33 bp, Artificial sequence
  primer
gggtctttgaagtttaatacttgtttagttctc

SEQ ID NO: 303 - DNA, 15 bp, Artificial sequence
  probe
caaagagcaacaacg

SEQ ID NO: 304 - DNA, 17 bp, Artificial sequence
  probe
cacaaagagaaacaacg

SEQ ID NO: 305 - DNA, 23 bp, Artificial sequence
  primer
tgcgcttgtttctaagactccaa

SEQ ID NO: 306 - DNA, 22 bp, Artificial sequence
  primer
gggtcttcctaggagtgcacta

SEQ ID NO: 307 - DNA, 16 bp, Artificial sequence
  probe
cctgaaaccgcattgc

SEQ ID NO: 308 - DNA, 16 bp, Artificial sequence
  probe
cctgaaaccacattgc

SEQ ID NO: 309 - DNA, 25 bp, Artificial sequence
  primer
caatctcaaactgccactcttggta

SEQ ID NO: 310 - DNA, 21 bp, Artificial sequence
  primer
tcctgtcatgtgagctttgca

SEQ ID NO: 311 - DNA, 17 bp, Artificial sequence
  probe
ccatcacgttactaccg

SEQ ID NO: 312 - DNA, 16 bp, Artificial sequence
  probe
catcacgtgactaccg

SEQ ID NO: 313 - DNA, 25 bp, Artificial sequence
  primer
ttctggccattcacagttaatacgt

SEQ ID NO: 314 - DNA, 33 bp, Artificial sequence
  primer
aattaaagcaccaactatcttacaatgttgaac

SEQ ID NO: 315 - DNA, 20 bp, Artificial sequence
  probe
caacgaattgaaccgagtga

SEQ ID NO: 316 - DNA, 20 bp, Artificial sequence
  probe
caacgaattgaacggagtga

SEQ ID NO: 317 - DNA, 24 bp, Artificial sequence
  primer
cctatctggaagtttgagcttgct

SEQ ID NO: 318 - DNA, 25 bp, Artificial sequence
  primer
ctcaacaagatgtcaccgtcataga

SEQ ID NO: 319 - DNA, 19 bp, Artificial sequence
  primer
aagttgagctaagaatata

SEQ ID NO: 320 - DNA, 19 bp, Artificial sequence
  primer
aagttgagctaacaatata

SEQ ID NO: 321 - DNA, 38 bp, Artificial sequence
  primer
cagtttttcagtttaagaaatatataaaccgcttagat

SEQ ID NO: 322 - DNA, 25 bp, Artificial sequence
  primer
gatagttcatggtagacctcagcat

SEQ ID NO: 323 - DNA, 20 bp, Artificial sequence
  probe
cgaaaagtaaactaaaccga

SEQ ID NO: 324 - DNA, 20 bp, Artificial sequence
  probe
cgaaaagtaaactgaaccga

SEQ ID NO: 325 - DNA, 19 bp, Artificial sequence
  primer
ccactgcaccccgtaatct

SEQ ID NO: 326 - DNA, 19 bp, Artificial sequence
  primer
gggaccagagacgtctgag

SEQ ID NO: 327 - DNA, 17 bp, Artificial sequence
  probe
aacatctgcgtcgctag

SEQ ID NO: 328 - DNA, 20 bp, Artificial sequence
  probe
ttgaacatctgcatcgctag

SEQ ID NO: 329 - DNA, 24 bp, Artificial sequence
  primer
cggctccaagttgcttttagtttg

SEQ ID NO: 330 - DNA, 30 bp, Artificial sequence
  primer
gctatacttacgtaaaaaaaagccttgaga

SEQ ID NO: 331 - DNA, 19 bp, Artificial sequence
  probe
ttatcaaacagagtaaatg

SEQ ID NO: 332 - DNA, 17 bp, Artificial sequence
  probe
atcaaacggagtaaatg

SEQ ID NO: 333 - DNA, 28 bp, Artificial sequence
  primer
agatcttgttgacttctcggtttaactc

SEQ ID NO: 334 - DNA, 22 bp, Artificial sequence
  primer
agggtcttggcatgttcctttt

SEQ ID NO: 335 - DNA, 15 bp, Artificial sequence
  probe
tcggtgacactttta

SEQ ID NO: 336 - DNA, 18 bp, Artificial sequence
  probe
atttcggtgaaactttta

SEQ ID NO: 337 - DNA, 33 bp, Artificial sequence
  primer
acctttttatatagagtagtcgagatggtttga

SEQ ID NO: 338 - DNA, 30 bp, Artificial sequence
  primer
gttgactctgtgaagttagatggatctaaa

SEQ ID NO: 339 - DNA, 18 bp, Artificial sequence
  probe
tttgcttatgttattctc

SEQ ID NO: 340 - DNA, 17 bp, Artificial sequence
  probe
ttgcttatgctattctc

SEQ ID NO: 341 - DNA, 34 bp, Artificial sequence
  primer
aaatgttatattttcgtttaattgtctgctggtt

SEQ ID NO: 342 - DNA, 22 bp, Artificial sequence
  primer
aaaacgtgggctttttcacagg

SEQ ID NO: 343 - DNA, 15 bp, Artificial sequence
  probe
acttgcgacggtcaa

SEQ ID NO: 344 - DNA, 17 bp, Artificial sequence
  probe
tgacttgcgatggtcaa

SEQ ID NO: 345 - DNA, 26 bp, Artificial sequence
  primer
aaccaacacaactattacccaaacct

SEQ ID NO: 346 - DNA, 25 bp, Artificial sequence
  primer
ccgcgttttagaacatggagtagaa

SEQ ID NO: 347 - DNA, 19 bp, Artificial sequence
  probe
caatgagagtctccacttt

SEQ ID NO: 348 - DNA, 19 bp, Artificial sequence
  probe
caatgagagtgtccacttt

SEQ ID NO: 349 - DNA, 25 bp, Artificial sequence
  primer
caatgttaaattctggtggccaaca

SEQ ID NO: 350 - DNA, 25 bp, Artificial sequence
  primer
gtagcacttgaggaataaccctgat

SEQ ID NO: 351 - DNA, 15 bp, Artificial sequence
  probe
actgcaggttcaccg

SEQ ID NO: 352 - DNA, 16 bp, Artificial sequence
  probe
aactgcagattcaccg

SEQ ID NO: 353 - DNA, 26 bp, Artificial sequence
  primer
aactggatgatcgtttaccactgaaa

SEQ ID NO: 354 - DNA, 25 bp, Artificial sequence
  primer
tcgattgttcatagctgccttttga

SEQ ID NO: 355 - DNA, 22 bp, Artificial sequence
  probe
cctaatttaggatatgtcccac

SEQ ID NO: 356 - DNA, 23 bp, Artificial sequence
  probe
ccctaatttaggatatatcccac

SEQ ID NO: 357 - DNA, 20 bp, Artificial sequence
  primer
tatcttcaccgacggctttc

SEQ ID NO: 358 - DNA, 20 bp, Artificial sequence
  primer
gaagtgccgactcaccaagt

SEQ ID NO: 359 - DNA, 15 bp, Artificial sequence
  probe
ctcttttgtttctcc

SEQ ID NO: 360 - DNA, 15 bp, Artificial sequence
  probe
actctttcgtttctc

SEQ ID NO: 361 - DNA, 19 bp, Artificial sequence
  primer
cgatgcaccatcatgtgag

SEQ ID NO: 362 - DNA, 25 bp, Artificial sequence
  primer
cctctaatttcactgacactcttga

SEQ ID NO: 363 - DNA, 18 bp, Artificial sequence
  probe
cagttctcctttcctatt

SEQ ID NO: 364 - DNA, 15 bp, Artificial sequence
  probe
cagttctcgtttcct

SEQ ID NO: 365 - DNA, 26 bp, Artificial sequence
  primer
tggtagagctgaaagatgatgttctc

SEQ ID NO: 366 - DNA, 24 bp, Artificial sequence
  primer
agccaaccgcttattaccactatg

SEQ ID NO: 367 - DNA, 18 bp, Artificial sequence
  probe
ttcggtatgacaagataa

SEQ ID NO: 368 - DNA, 19 bp, Artificial sequence
  probe
cttcggtatgacgagataa

SEQ ID NO: 369 - DNA, 23 bp, Artificial sequence
  primer
tggtctctgcatcttcgaatctg

SEQ ID NO: 370 - DNA, 24 bp, Artificial sequence
  primer
cgatataccaaggttgctgatgct

SEQ ID NO: 371 - DNA, 14 bp, Artificial sequence
  probe
ccagaagcatttgc

SEQ ID NO: 372 - DNA, 16 bp, Artificial sequence
  probe
aaccagaagaatttgc

SEQ ID NO: 373 - DNA, 30 bp, Artificial sequence
  primer
gaacctaaaccaatggatagaaacttgact

SEQ ID NO: 374 - DNA, 38 bp, Artificial sequence
  primer
tcgaactaaaactagatgattatgattaaagcagtaaa

SEQ ID NO: 375 - DNA, 18 bp, Artificial sequence
  probe
cttagggtgtaggttaat

SEQ ID NO: 376 - DNA, 19 bp, Artificial sequence
  probe
ccttagggtgtaagttaat

SEQ ID NO: 377 - DNA, 30 bp, Artificial sequence
  primer
gtagacttttccaagctaatcttcagacaa

SEQ ID NO: 378 - DNA, 28 bp, Artificial sequence
  primer
ggtgtttattgaaggcactagaagatca

SEQ ID NO: 379 - DNA, 19 bp, Artificial sequence
  probe
caaatactttcagtatccc

SEQ ID NO: 380 - DNA, 19 bp, Artificial sequence
  probe
caaatactttcaatatccc

SEQ ID NO: 381 - DNA, 25 bp, Artificial sequence
  primer
ggccttgggattaagaatctttcga

SEQ ID NO: 382 - DNA, 23 bp, Artificial sequence
  primer
cgagcctgcctgaaagaaaagta

SEQ ID NO: 383 - DNA, 17 bp, Artificial sequence
  probe
cagatcaacctaaggca

SEQ ID NO: 384 - DNA, 18 bp, Artificial sequence
  probe
ccagatcaacttaaggca

SEQ ID NO: 385 - DNA, 25 bp, Artificial sequence
  primer
gcagctctttgtttcaaacccatta

SEQ ID NO: 386 - DNA, 21 bp, Artificial sequence
  primer
gtaccgatgaaacgcgagaag

SEQ ID NO: 387 - DNA, 18 bp, Artificial sequence
  probe
cacatcaattcagttttt

SEQ ID NO: 388 - DNA, 18 bp, Artificial sequence
  probe
cacatcaattgagttttt

SEQ ID NO: 389 - DNA, 20 bp, Artificial sequence
  primer
gtggcacaagatgcgatgag

SEQ ID NO: 390 - DNA, 30 bp, Artificial sequence
  primer
aagtttcattagttttgatgggtagtgcta

SEQ ID NO: 391 - DNA, 15 bp, Artificial sequence
  probe
aagatccgcatggct

SEQ ID NO: 392 - DNA, 18 bp, Artificial sequence
  probe
aagaagatcagcatggct

SEQ ID NO: 393 - DNA, 20 bp, Artificial sequence
  primer
catctggatcaccggttggt

SEQ ID NO: 394 - DNA, 21 bp, Artificial sequence
  primer
ccgtcactgtctcaggaggaa

SEQ ID NO: 395 - DNA, 15 bp, Artificial sequence
  probe
aacgcccgccagaga

SEQ ID NO: 396 - DNA, 16 bp, Artificial sequence
  probe
caacgcccgctagaga

SEQ ID NO: 397 - DNA, 27 bp, Artificial sequence
  primer
gataactatattcatcgactcccaaac

SEQ ID NO: 398 - DNA, 19 bp, Artificial sequence
  primer
ggaccatctgcgtggtaga

SEQ ID NO: 399 - DNA, 19 bp, Artificial sequence
  probe
acataagttaccaccagtt

SEQ ID NO: 400 - DNA, 19 bp, Artificial sequence
  probe
acaaaagttaccaccagtt

SEQ ID NO: 401 - DNA, 36 bp, Artificial sequence
  primer
cttatacacttaagtctttgaatttcaaactatgca

SEQ ID NO: 402 - DNA, 28 bp, Artificial sequence
  primer
ccacaacaaacagctctacttacaatac

SEQ ID NO: 403 - DNA, 16 bp, Artificial sequence
  probe
cttcgcatcctaatcg

SEQ ID NO: 404 - DNA, 16 bp, Artificial sequence
  probe
cttcgcatcttaatcg

SEQ ID NO: 405 - DNA, 28 bp, Artificial sequence
  primer
cgcttgagagcttttaaagagagatagt

SEQ ID NO: 406 - DNA, 24 bp, Artificial sequence
  primer
gcccatttaagcaccataccaatc

SEQ ID NO: 407 - DNA, 19 bp, Artificial sequence
  probe
actgcatgcaattatatat

SEQ ID NO: 408 - DNA, 18 bp, Artificial sequence
  probe
ctgcatgcaatgatatat

SEQ ID NO: 409 - DNA, 22 bp, Artificial sequence
  primer
aaactgtgagtccctggagaga

SEQ ID NO: 410 - DNA, 28 bp, Artificial sequence
  primer
gtatggcttcttgattaagtttgaagca

SEQ ID NO: 411 - DNA, 18 bp, Artificial sequence
  probe
cacaacctgaactctact

SEQ ID NO: 412 - DNA, 18 bp, Artificial sequence
  probe
cacaacctgaaatctact

SEQ ID NO: 413 - DNA, 22 bp, Artificial sequence
  primer
cagattggtaatggttccctgt

SEQ ID NO: 414 - DNA, 20 bp, Artificial sequence
  primer
catggattttcctgccctaa

SEQ ID NO: 415 - DNA, 16 bp, Artificial sequence
  probe
ttgcatatcatcccca

SEQ ID NO: 416 - DNA, 15 bp, Artificial sequence
  probe
ttgcatatcatcgcc

SEQ ID NO: 417 - DNA, 25 bp, Artificial sequence
  primer
ccatgcaacgtaggaaacaagtatc

SEQ ID NO: 418 - DNA, 25 bp, Artificial sequence
  primer
cgaggtcgaattgttttggtatgtg

SEQ ID NO: 419 - DNA, 18 bp, Artificial sequence
  probe
aacttctctatattttcc

SEQ ID NO: 420 - DNA, 20 bp, Artificial sequence
  probe
tgaacttctctatcttttcc

SEQ ID NO: 421 - DNA, 21 bp, Artificial sequence
  primer
aagagaagcgtctcctcgttc

SEQ ID NO: 422 - DNA, 20 bp, Artificial sequence
  primer
tcgacgtctatccccaagat

SEQ ID NO: 423 - DNA, 14 bp, Artificial sequence
  probe
acgcaaccaccgat

SEQ ID NO: 424 - DNA, 14 bp, Artificial sequence
  probe
acgcaacgaccgat

SEQ ID NO: 425 - DNA, 37 bp, Artificial sequence
  primer
gaaaagataattaaataaaacgaaccaacaaacaaca

SEQ ID NO: 426 - DNA, 31 bp, Artificial sequence
  primer
ccaaacatttattactaggattttcctccct

SEQ ID NO: 427 - DNA, 16 bp, Artificial sequence
  probe
aatagccacgaatgaa

SEQ ID NO: 428 - DNA, 19 bp, Artificial sequence
  probe
agaaatagccacaaatgaa

SEQ ID NO: 429 - DNA, 23 bp, Artificial sequence
  primer
cggagaccttcagtgtgttagac

SEQ ID NO: 430 - DNA, 24 bp, Artificial sequence
  primer
gttcccaatgtaagcacaaaggtt

SEQ ID NO: 431 - DNA, 17 bp, Artificial sequence
  probe
acgtgataaccaactac

SEQ ID NO: 432 - DNA, 17 bp, Artificial sequence
  probe
acgtgataacaaactac

SEQ ID NO: 433 - DNA, 22 bp, Artificial sequence
  primer
tcaacaactggttcatctggaa

SEQ ID NO: 434 - DNA, 21 bp, Artificial sequence
  primer
ccagtgaagatggatgcaaag

SEQ ID NO: 435 - DNA, 16 bp, Artificial sequence
  probe
ctaccacagacttatc

SEQ ID NO: 436 - DNA, 17 bp, Artificial sequence
  probe
tctaccacagacttgtc

SEQ ID NO: 437 - DNA, 28 bp, Artificial sequence
  primer
cttactgatcatgttagttggcagtttt

SEQ ID NO: 438 - DNA, 32 bp, Artificial sequence
  primer
gagccattgtttgtaagagaaattgaatatga

SEQ ID NO: 439 - DNA, 19 bp, Artificial sequence
  probe
ttgagtatgcaggtatgtc

SEQ ID NO: 440 - DNA, 19 bp, Artificial sequence
  probe
ttgagtatgcagatatgtc

SEQ ID NO: 441 - DNA, 24 bp, Artificial sequence
  primer
cgtctctgcttacctcactatgaa

SEQ ID NO: 442 - DNA, 23 bp, Artificial sequence
  primer
gcagtagacaacagcttttggaa

SEQ ID NO: 443 - DNA, 17 bp, Artificial sequence
  probe
acataaacatggtctgc

SEQ ID NO: 444 - DNA, 17 bp, Artificial sequence
  probe
acataatcatggtctgc

SEQ ID NO: 445 - DNA, 29 bp, Artificial sequence
  primer
tgatttgcctagaccaatttttagaacac

SEQ ID NO: 446 - DNA, 27 bp, Artificial sequence
  primer
ggttaaaacatgaaccgttaagctgaa

SEQ ID NO: 447 - DNA, 20 bp, Artificial sequence
  probe
tttgtctttggttgtagttg

SEQ ID NO: 448 - DNA, 22 bp, Artificial sequence
  probe
tgtttgtctttggttatagttg

SEQ ID NO: 449 - DNA, 21 bp, Artificial sequence
  primer
tccttctcctccgagaaagtt

SEQ ID NO: 450 - DNA, 21 bp, Artificial sequence
  primer
cctccgtatccgtagacatca

SEQ ID NO: 451 - DNA, 19 bp, Artificial sequence
  probe
acgttaaatcgtttagttg

SEQ ID NO: 452 - DNA, 18 bp, Artificial sequence
  probe
caacgttaagtcgtttag

SEQ ID NO: 453 - DNA, 40 bp, Artificial sequence
  primer
cactaatttatatagaaaatatgtaaaactttttccatca

SEQ ID NO: 454 - DNA, 37 bp, Artificial sequence
  primer
gatgggtgccataataatctatttatactttttttgt

SEQ ID NO: 455 - DNA, 19 bp, Artificial sequence
  probe
tttctaacatcgtggaaat

SEQ ID NO: 456 - DNA, 22 bp, Artificial sequence
  probe
ccatttctaacatagtggaaat

SEQ ID NO: 457 - DNA, 31 bp, Artificial sequence
  primer
tgtgaaaatataagtttcacatcgagatcga

SEQ ID NO: 458 - DNA, 37 bp, Artificial sequence
  primer
tcatgttaagtttggatttatcatgagttttcaaatt

SEQ ID NO: 459 - DNA, 17 bp, Artificial sequence
  probe
tcaatccacgtattacc

SEQ ID NO: 460 - DNA, 18 bp, Artificial sequence
  probe
atcaatccacatattacc

SEQ ID NO: 461 - DNA, 23 bp, Artificial sequence
  primer
aaacgccaaaactggtcatcttg

SEQ ID NO: 462 - DNA, 25 bp, Artificial sequence
  primer
accgtaaccagctctctctgtaata

SEQ ID NO: 463 - DNA, 18 bp, Artificial sequence
  probe
acgtgtcgtaattcatgt

SEQ ID NO: 464 - DNA, 18 bp, Artificial sequence
  probe
acgtgtcgtagttcatgt

SEQ ID NO: 465 - DNA, 35 bp, Artificial sequence
  primer
ccgccaagttttaaacaaaatcaataaatcatatt

SEQ ID NO: 466 - DNA, 32 bp, Artificial sequence
  primer
tgtgcagttaatagttgtatagtgtatctttg

SEQ ID NO: 467 - DNA, 19 bp, Artificial sequence
  probe
tgaagtttcaaccaccatt

SEQ ID NO: 468 - DNA, 19 bp, Artificial sequence
  probe
tgaagtttcaagcaccatt

SEQ ID NO: 469 - DNA, 37 bp, Artificial sequence
  primer
agccaattttaagtaaatcattgaatattgttagtgt

SEQ ID NO: 470 - DNA, 26 bp, Artificial sequence
  primer
cggagggatttcgaaatagtatgtgt

SEQ ID NO: 471 - DNA, 18 bp, Artificial sequence
  probe
cctctctgagttaattga

SEQ ID NO: 472 - DNA, 18 bp, Artificial sequence
  probe
cctctctgagtaaattga

SEQ ID NO: 473 - DNA, 34 bp, Artificial sequence
  primer
gtagggtatcattttatttttctatcgactgagt

SEQ ID NO: 474 - DNA, 20 bp, Artificial sequence
  primer
cgcgtgcttagtggttacca

SEQ ID NO: 475 - DNA, 17 bp, Artificial sequence
  probe
agtgcttgtgtctcatg

SEQ ID NO: 476 - DNA, 18 bp, Artificial sequence
  probe
cagtgcttgtgtgtcatg

SEQ ID NO: 477 - DNA, 39 bp, Artificial sequence
  primer
gcatgaatagtagtagctttctttttttaaatgtgtata

SEQ ID NO: 478 - DNA, 40 bp, Artificial sequence
  primer
aaattaacaacagtgttacctaattattataaagaattga

SEQ ID NO: 479 - DNA, 18 bp, Artificial sequence
  probe
ttgagaagtctcgaaaat

SEQ ID NO: 480 - DNA, 18 bp, Artificial sequence
  probe
ttgagaagtctggaaaat

SEQ ID NO: 481 - DNA, 25 bp, Artificial sequence
  primer
cgccaactacacaagagcataattt

SEQ ID NO: 482 - DNA, 25 bp, Artificial sequence
  primer
gaagctgtggaagttacaatgcaaa

SEQ ID NO: 483 - DNA, 17 bp, Artificial sequence
  probe
cctcaagtcttaaactt

SEQ ID NO: 484 - DNA, 16 bp, Artificial sequence
  probe
ctcaagtctgaaactt

SEQ ID NO: 485 - DNA, 26 bp, Artificial sequence
  primer
tccacaatctctccttccaaattcac

SEQ ID NO: 486 - DNA, 21 bp, Artificial sequence
  primer
actcgggtctgtacgttgaga

SEQ ID NO: 487 - DNA, 14 bp, Artificial sequence
  probe
cggagacaaggaag

SEQ ID NO: 488 - DNA, 16 bp, Artificial sequence
  probe
accggagacgaggaag

SEQ ID NO: 489 - DNA, 29 bp, Artificial sequence
  primer
tcacctctcatgttgctataaggttatct

SEQ ID NO: 490 - DNA, 29 bp, Artificial sequence
  primer
ctgaagcaatcacaaattgaactaaagga

SEQ ID NO: 491 - DNA, 16 bp, Artificial sequence
  probe
aacttctcacattgcc

SEQ ID NO: 492 - DNA, 16 bp, Artificial sequence
  probe
aacttctcgcattgcc

SEQ ID NO: 493 - DNA, 34 bp, Artificial sequence
  primer
ttttctcacaaagatcatgtactcattacttctt

SEQ ID NO: 494 - DNA, 23 bp, Artificial sequence
  primer
aagcttgcaagccaaaagagatg

SEQ ID NO: 495 - DNA, 14 bp, Artificial sequence
  probe
cgcaacacaagatt

SEQ ID NO: 496 - DNA, 16 bp, Artificial sequence
  probe
accgcaacataagatt

SEQ ID NO: 497 - DNA, 25 bp, Artificial sequence
  primer
ctccttctagagtctgggaatcgaa

SEQ ID NO: 498 - DNA, 25 bp, Artificial sequence
  primer
gcagaaaatttggacccccattaaa

SEQ ID NO: 499 - DNA, 16 bp, Artificial sequence
  probe
tttgcgtcattaaaat

SEQ ID NO: 500 - DNA, 16 bp, Artificial sequence
  probe
tttgcgtcaataaaat

SEQ ID NO: 501 - DNA, 27 bp, Artificial sequence
  primer
aagttcatctacacttaatccgacaca

SEQ ID NO: 502 - DNA, 25 bp, Artificial sequence
  primer
gagttcattccacagatctgaccat

SEQ ID NO: 503 - DNA, 17 bp, Artificial sequence
  probe
cctatcaaagcacgtct

SEQ ID NO: 504 - DNA, 16 bp, Artificial sequence
  probe
ctatcaaagcaagtct

SEQ ID NO: 505 - DNA, 24 bp, Artificial sequence
  primer
cgatcgagagaaacttcgagactt

SEQ ID NO: 506 - DNA, 32 bp, Artificial sequence
  primer
ccgataaaacaatcaacaccaaaaacaattaa

SEQ ID NO: 507 - DNA, 16 bp, Artificial sequence
  probe
cccaacaaaagaggca

SEQ ID NO: 508 - DNA, 16 bp, Artificial sequence
  probe
cccaacaaaggaggca

SEQ ID NO: 509 - DNA, 45 bp, Artificial sequence
  primer
agtagaatacttaatgtttataatcacgagatataattgttttca

SEQ ID NO: 510 - DNA, 25 bp, Artificial sequence
  primer
cctggtggccatgtataatatcaca

SEQ ID NO: 511 - DNA, 15 bp, Artificial sequence
  probe
atccccacatgatgc

SEQ ID NO: 512 - DNA, 16 bp, Artificial sequence
  probe
catccccaaatgatgc

SEQ ID NO: 513 - DNA, 20 bp, Artificial sequence
  primer
tagagaccaaggcccaacag

SEQ ID NO: 514 - DNA, 20 bp, Artificial sequence
  primer
ttatttgtgtggtgcggttc

SEQ ID NO: 515 - DNA, 16 bp, Artificial sequence
  probe
tccacaactagcaacc

SEQ ID NO: 516 - DNA, 14 bp, Artificial sequence
  probe
ccaccactagcaac

SEQ ID NO: 517 - DNA, 29 bp, Artificial sequence
  primer
ctgagtaattatagtattgtgccaaccct

SEQ ID NO: 518 - DNA, 23 bp, Artificial sequence
  primer
gggcttttgtttgacttgtgcaa

SEQ ID NO: 519 - DNA, 18 bp, Artificial sequence
  probe
caaagaagtccgtctaac

SEQ ID NO: 520 - DNA, 18 bp, Artificial sequence
  probe
caaagaagtcggtctaac

SEQ ID NO: 521 - DNA, 27 bp, Artificial sequence
  primer
gcatcaaccatcaatctgaatggtatg

SEQ ID NO: 522 - DNA, 25 bp, Artificial sequence
  primer
ggcatcctactgacctgtatgttaa

SEQ ID NO: 523 - DNA, 18 bp, Artificial sequence
  probe
atttgcaaaaatttctct

SEQ ID NO: 524 - DNA, 19 bp, Artificial sequence
  probe
aatttgcaaaaagttctct

SEQ ID NO: 525 - DNA, 26 bp, Artificial sequence
  primer
gtcccatgcattgtatttgaagttga

SEQ ID NO: 526 - DNA, 31 bp, Artificial sequence
  primer
tgcatacatatgatcatcaaatttcccaatg

SEQ ID NO: 527 - DNA, 17 bp, Artificial sequence
  probe
ctagatgcacacttcta

SEQ ID NO: 528 - DNA, 17 bp, Artificial sequence
  probe
ctagatgcacgcttcta

SEQ ID NO: 529 - DNA, 26 bp, Artificial sequence
  primer
atcataatgtcatgactgcctggttt

SEQ ID NO: 530 - DNA, 27 bp, Artificial sequence
  primer
tcttaaaaaccaactacacacatcgtt

SEQ ID NO: 531 - DNA, 18 bp, Artificial sequence
  probe
tcccatatgtgtatcatg

SEQ ID NO: 532 - DNA, 20 bp, Artificial sequence
  probe
catcccatatgtttatcatg

SEQ ID NO: 533 - DNA, 23 bp, Artificial sequence
  primer
gttcgacctggaatatcggaaga

SEQ ID NO: 534 - DNA, 22 bp, Artificial sequence
  primer
cacttgcacgatatcgcgaatc

SEQ ID NO: 535 - DNA, 20 bp, Artificial sequence
  probe
tagatgacttatcggaaagt

SEQ ID NO: 536 - DNA, 21 bp, Artificial sequence
  probe
atagatgacttatcagaaagt

SEQ ID NO: 537 - DNA, 23 bp, Artificial sequence
  primer
gatcaatgtacacgcgtcaagac

SEQ ID NO: 538 - DNA, 21 bp, Artificial sequence
  primer
ggagttccatcacgcctcttc

SEQ ID NO: 539 - DNA, 17 bp, Artificial sequence
  probe
aagaatgttgaaaccgc

SEQ ID NO: 540 - DNA, 17 bp, Artificial sequence
  probe
aagaatgttggaaccgc

SEQ ID NO: 541 - DNA, 32 bp, Artificial sequence
  primer
caataaaacaaaaacaataatctgacgcacat

SEQ ID NO: 542 - DNA, 25 bp, Artificial sequence
  primer
gagtctcagattgatagccccaatt

SEQ ID NO: 543 - DNA, 20 bp, Artificial sequence
  probe
cttcatagtttgataagttc

SEQ ID NO: 544 - DNA, 19 bp, Artificial sequence
  probe
ttcatagtttggtaagttc

SEQ ID NO: 545 - DNA, 25 bp, Artificial sequence
  primer
agcctggtgcgtatgtatcataaaa

SEQ ID NO: 546 - DNA, 34 bp, Artificial sequence
  primer
atcgaaagatgcatagagtaatgattaataacca

SEQ ID NO: 547 - DNA, 19 bp, Artificial sequence
  probe
ctaaaactgtggtggttta

SEQ ID NO: 548 - DNA, 21 bp, Artificial sequence
  probe
ctctaaaactgtgatggttta

SEQ ID NO: 549 - DNA, 25 bp, Artificial sequence
  primer
cttcccggaaaaggtatcgattgta

SEQ ID NO: 550 - DNA, 25 bp, Artificial sequence
  primer
acgcttcaaaccctaaagacagaat

SEQ ID NO: 551 - DNA, 20 bp, Artificial sequence
  probe
atttcatcttgattctattg

SEQ ID NO: 552 - DNA, 20 bp, Artificial sequence
  probe
atttcatcttgagtctattg

SEQ ID NO: 553 - DNA, 25 bp, Artificial sequence
  primer
ccaggatcgatttgagatgaaagct

SEQ ID NO: 554 - DNA, 29 bp, Artificial sequence
  primer
tcaacagtcaacttttgaacaaaaaaggt

SEQ ID NO: 555 - DNA, 18 bp, Artificial sequence
  probe
atatagctaggcaattca

SEQ ID NO: 556 - DNA, 21 bp, Artificial sequence
  probe
aggatatagctagacaattca

SEQ ID NO: 557 - DNA, 30 bp, Artificial sequence
  primer
cggtaaaccagtacaaaatatccaaatgtt

SEQ ID NO: 558 - DNA, 37 bp, Artificial sequence
  primer
cggatttaaaatagtttgaagataaataatggcttgt

SEQ ID NO: 559 - DNA, 16 bp, Artificial sequence
  probe
acttgtgctaatctct

SEQ ID NO: 560 - DNA, 15 bp, Artificial sequence
  probe
cttgtgcaaatctct

SEQ ID NO: 561 - DNA, 20 bp, Artificial sequence
  primer
cccagtacccaatgctcatc

SEQ ID NO: 562 - DNA, 21 bp, Artificial sequence
  primer
ccgtcggttatacacaccaag

SEQ ID NO: 563 - DNA, 17 bp, Artificial sequence
  probe
aactgcctttgttttgt

SEQ ID NO: 564 - DNA, 15 bp, Artificial sequence
  probe
ctgcctgtgttttgt

SEQ ID NO: 565 - DNA, 25 bp, Artificial sequence
  primer
gctttgcctaagagattgcttcatg

SEQ ID NO: 566 - DNA, 23 bp, Artificial sequence
  primer
tgcttgtgcttgtagtcatctga

SEQ ID NO: 567 - DNA, 16 bp, Artificial sequence
  probe
ttgaacgaaaattagc

SEQ ID NO: 568 - DNA, 16 bp, Artificial sequence
  probe
ttgaacgaagattagc

SEQ ID NO: 569 - DNA, 27 bp, Artificial sequence
  primer
ggatttgttataccattgcatcaagca

SEQ ID NO: 570 - DNA, 20 bp, Artificial sequence
  primer
acagagggtcgttggacaac

SEQ ID NO: 571 - DNA, 16 bp, Artificial sequence
  probe
acacttctcaaaggct

SEQ ID NO: 572 - DNA, 17 bp, Artificial sequence
  probe
cacacttctcaatggct

SEQ ID NO: 573 - DNA, 28 bp, Artificial sequence
  primer
ctagtttctttccttgtacttccttcca

SEQ ID NO: 574 - DNA, 30 bp, Artificial sequence
  primer
gctttcctatttttatcggaaattgacagt

SEQ ID NO: 575 - DNA, 19 bp, Artificial sequence
  probe
tgacaaggaactaagttta

SEQ ID NO: 576 - DNA, 19 bp, Artificial sequence
  probe
tgacaaggaacaaagttta

SEQ ID NO: 577 - DNA, 27 bp, Artificial sequence
  primer
agaataaacagctttctacacccgtag

SEQ ID NO: 578 - DNA, 24 bp, Artificial sequence
  primer
tctggtgggataaggtgattgaga

SEQ ID NO: 579 - DNA, 17 bp, Artificial sequence
  probe
caccaagactgagacac

SEQ ID NO: 580 - DNA, 18 bp, Artificial sequence
  probe
tcaccaagactaagacac

SEQ ID NO: 581 - DNA, 22 bp, Artificial sequence
  primer
ggcatcgtctggttgatcaaga

SEQ ID NO: 582 - DNA, 25 bp, Artificial sequence
  primer
cccattccacttgataacccgattt

SEQ ID NO: 583 - DNA, 19 bp, Artificial sequence
  probe
catgacattttgccattaa

SEQ ID NO: 584 - DNA, 21 bp, Artificial sequence
  probe
tgcatgacattttaccattaa

SEQ ID NO: 585 - DNA, 25 bp, Artificial sequence
  primer
catagacctccacatcaccaagaaa

SEQ ID NO: 586 - DNA, 30 bp, Artificial sequence
  primer
tgtaaagcaaaaacccaaacacaataaagt

SEQ ID NO: 587 - DNA, 17 bp, Artificial sequence
  probe
agggagacacgtgtcat

SEQ ID NO: 588 - DNA, 18 bp, Artificial sequence
  probe
aagggagacacatgtcat

SEQ ID NO: 589 - DNA, 30 bp, Artificial sequence
  primer
agcacacaaaggtttcttaggaagattatt

SEQ ID NO: 590 - DNA, 27 bp, Artificial sequence
  primer
ggttcaaatgtttaggacacgaaagac

SEQ ID NO: 591 - DNA, 16 bp, Artificial sequence
  probe
cccgaatgcccagacc

SEQ ID NO: 592 - DNA, 15 bp, Artificial sequence
  probe
ccgaatgcgcagacc

SEQ ID NO: 593 - DNA, 29 bp, Artificial sequence
  primer
atctattcccagagaatacgttttttcga

SEQ ID NO: 594 - DNA, 25 bp, Artificial sequence
  primer
gcccctagtgaaaagaatgaggtaa

SEQ ID NO: 595 - DNA, 16 bp, Artificial sequence
  probe
tcagagaccaggaatt

SEQ ID NO: 596 - DNA, 16 bp, Artificial sequence
  probe
tcagagacgaggaatt

SEQ ID NO: 597 - DNA, 24 bp, Artificial sequence
  primer
acctccattcatcattcccaatcc

SEQ ID NO: 598 - DNA, 24 bp, Artificial sequence
  primer
gctcggctaagaatcacactgaaa

SEQ ID NO: 599 - DNA, 17 bp, Artificial sequence
  probe
caacaccaagttcttac

SEQ ID NO: 600 - DNA, 17 bp, Artificial sequence
  probe
caacaccaagatcttac

SEQ ID NO: 601 - DNA, 17 bp, Artificial sequence
  primer
ccgcttttgcccatggc

SEQ ID NO: 602 - DNA, 30 bp, Artificial sequence
  primer
actaccaacgttaagaatacacttggattt

SEQ ID NO: 603 - DNA, 19 bp, Artificial sequence
  probe
attgcattcagttgttgaa

SEQ ID NO: 604 - DNA, 19 bp, Artificial sequence
  probe
attgcattcagtagttgaa

SEQ ID NO: 605 - DNA, 26 bp, Artificial sequence
  primer
gaacaacagtttgccatttccttact

SEQ ID NO: 606 - DNA, 28 bp, Artificial sequence
  primer
ggcatccattacctatcaatttcttgga

SEQ ID NO: 607 - DNA, 16 bp, Artificial sequence
  probe
cgtaaaagcgaaagta

SEQ ID NO: 608 - DNA, 17 bp, Artificial sequence
  probe
ccgtaaaagggaaagta

SEQ ID NO: 609 - DNA, 30 bp, Artificial sequence
  primer
agcgaaaagattacactttgtttctttgaa

SEQ ID NO: 610 - DNA, 30 bp, Artificial sequence
  primer
gccttagtatactctagtttcattgccaaa

SEQ ID NO: 611 - DNA, 20 bp, Artificial sequence
  probe
ttttggtttttctggtttat

SEQ ID NO: 612 - DNA, 18 bp, Artificial sequence
  probe
ttggtttttcgggtttat

SEQ ID NO: 613 - DNA, 26 bp, Artificial sequence
  primer
ctccagttgcaacttcttcaaatcat

SEQ ID NO: 614 - DNA, 25 bp, Artificial sequence
  primer
gatgacccatagaccaaagccatat

SEQ ID NO: 615 - DNA, 20 bp, Artificial sequence
  probe
tgtttaatgaaacgctattg

SEQ ID NO: 616 - DNA, 22 bp, Artificial sequence
  probe
catgtttaatgaaatgctattg

SEQ ID NO: 617 - DNA, 23 bp, Artificial sequence
  primer
caaatgactaacctgcgcaagtg

SEQ ID NO: 618 - DNA, 24 bp, Artificial sequence
  primer
agtcaagggagtgggaaagtagat

SEQ ID NO: 619 - DNA, 15 bp, Artificial sequence
  probe
ccggttggttcgaca

SEQ ID NO: 620 - DNA, 16 bp, Artificial sequence
  probe
cccggttgattcgaca

SEQ ID NO: 621 - DNA, 25 bp, Artificial sequence
  primer
accaggaaggaggtcaagatcttaa

SEQ ID NO: 622 - DNA, 31 bp, Artificial sequence
  primer
agcatcgactttctacattatgttctctttt

SEQ ID NO: 623 - DNA, 17 bp, Artificial sequence
  probe
aatgctccattaacaaa

SEQ ID NO: 624 - DNA, 16 bp, Artificial sequence
  probe
atgctccgttaacaaa

SEQ ID NO: 625 - DNA, 33 bp, Artificial sequence
  primer
cgcttacatcattattcattttttagacacact

SEQ ID NO: 626 - DNA, 21 bp, Artificial sequence
  primer
ggtagttgcgacaagcacatc

SEQ ID NO: 627 - DNA, 19 bp, Artificial sequence
  probe
caccattatcgatgtttaa

SEQ ID NO: 628 - DNA, 18 bp, Artificial sequence
  probe
accattatcggtgtttaa

SEQ ID NO: 629 - DNA, 23 bp, Artificial sequence
  primer
tgctccactgtctcttcagaaac

SEQ ID NO: 630 - DNA, 25 bp, Artificial sequence
  primer
aatccttaactgaaacctggactcg

SEQ ID NO: 631 - DNA, 15 bp, Artificial sequence
  probe
attcgctagattcca

SEQ ID NO: 632 - DNA, 15 bp, Artificial sequence
  probe
attcgctggattcca

SEQ ID NO: 633 - DNA, 25 bp, Artificial sequence
  primer
gaccagagttgatccaggaatgtaa

SEQ ID NO: 634 - DNA, 21 bp, Artificial sequence
  primer
gcacggtgatcttggacacat

SEQ ID NO: 635 - DNA, 19 bp, Artificial sequence
  probe
tttctggcctatgagctca

SEQ ID NO: 636 - DNA, 19 bp, Artificial sequence
  probe
tttctggcctttgagctca

SEQ ID NO: 637 - DNA, 25 bp, Artificial sequence
  primer
caaaccgtactttccctatgatggt

SEQ ID NO: 638 - DNA, 24 bp, Artificial sequence
  primer
tggtatctcgacaatggagctagt

SEQ ID NO: 639 - DNA, 18 bp, Artificial sequence
  probe
atctcctgtcatatgatt

SEQ ID NO: 640 - DNA, 17 bp, Artificial sequence
  probe
tctcctgtcaaatgatt

SEQ ID NO: 641 - DNA, 25 bp, Artificial sequence
  primer
gcattggcaggttttaaatctcaga

SEQ ID NO: 642 - DNA, 26 bp, Artificial sequence
  primer
ctcaaaaccaatggaagtgttactgt

SEQ ID NO: 643 - DNA, 18 bp, Artificial sequence
  probe
ttgtgcataatgacaccc

SEQ ID NO: 644 - DNA, 17 bp, Artificial sequence
  probe
tgtgcataaagacaccc

SEQ ID NO: 645 - DNA, 23 bp, Artificial sequence
  primer
tgatatcacgacgacggtttctg

SEQ ID NO: 646 - DNA, 21 bp, Artificial sequence
  primer
gagctttctccagcgtgattg

SEQ ID NO: 647 - DNA, 19 bp, Artificial sequence
  probe
ctcagtctctctcggagat

SEQ ID NO: 648 - DNA, 19 bp, Artificial sequence
  probe
ctcagtctctcacggagat

SEQ ID NO: 649 - DNA, 29 bp, Artificial sequence
  primer
gaaatcctacacgattttaagcatgtcaa

SEQ ID NO: 650 - DNA, 18 bp, Artificial sequence
  primer
gcgcatcaccctcattcc

SEQ ID NO: 651 - DNA, 16 bp, Artificial sequence
  probe
tacaccccaggcttaa

SEQ ID NO: 652 - DNA, 15 bp, Artificial sequence
  probe
acacccctggcttaa

SEQ ID NO: 653 - DNA, 29 bp, Artificial sequence
  primer
gagtttcttgtattcatctaggtcaacga

SEQ ID NO: 654 - DNA, 34 bp, Artificial sequence
  primer
tgaggatatacatgcatatcttgccatatatttg

SEQ ID NO: 655 - DNA, 21 bp, Artificial sequence
  probe
cggtattaggtaacctagcat

SEQ ID NO: 656 - DNA, 21 bp, Artificial sequence
  probe
cggtattaggtaacgtagcat

SEQ ID NO: 657 - DNA, 23 bp, Artificial sequence
  primer
caccaaagctaactctgcactct

SEQ ID NO: 658 - DNA, 21 bp, Artificial sequence
  primer
caggacgagttaaggcaaggt

SEQ ID NO: 659 - DNA, 19 bp, Artificial sequence
  probe
attgtagactgcctactac

SEQ ID NO: 660 - DNA, 19 bp, Artificial sequence
  probe
attgtagactgcgtactac

SEQ ID NO: 661 - DNA, 25 bp, Artificial sequence
  primer
gacatcttttgggaccttagcatct

SEQ ID NO: 662 - DNA, 25 bp, Artificial sequence
  primer
ggattagccaagttccattcctaca

SEQ ID NO: 663 - DNA, 19 bp, Artificial sequence
  probe
aagcaactcaataagaaga

SEQ ID NO: 664 - DNA, 19 bp, Artificial sequence
  probe
aagcaactcaatgagaaga

SEQ ID NO: 665 - DNA, 20 bp, Artificial sequence
  primer
tgcaacttggtcagcactca

SEQ ID NO: 666 - DNA, 27 bp, Artificial sequence
  primer
caccatataggaaatcatgagcacgaa

SEQ ID NO: 667 - DNA, 15 bp, Artificial sequence
  probe
tcgcgctctatttca

SEQ ID NO: 668 - DNA, 15 bp, Artificial sequence
  probe
tcgcgctctgtttca

SEQ ID NO: 669 - DNA, 32 bp, Artificial sequence
  primer
cgattcggaatgatcatataagatcaaacttc

SEQ ID NO: 670 - DNA, 30 bp, Artificial sequence
  primer
gggtaattacggatgcaagactttatagtt

SEQ ID NO: 671 - DNA, 19 bp, Artificial sequence
  probe
atgtctgcactatatctat

SEQ ID NO: 672 - DNA, 18 bp, Artificial sequence
  probe
tgtctgcactaaatctat

SEQ ID NO: 673 - DNA, 25 bp, Artificial sequence
  primer
ccgctgaaggtatatcgaagaatct

SEQ ID NO: 674 - DNA, 26 bp, Artificial sequence
  primer
ccttgttcagtcttactcagcttttg

SEQ ID NO: 675 - DNA, 15 bp, Artificial sequence
  probe
caaaccggatgatgc

SEQ ID NO: 676 - DNA, 17 bp, Artificial sequence
  probe
ttcaaaccgaatgatgc

SEQ ID NO: 677 - DNA, 38 bp, Artificial sequence
  primer
aaagcaaccaaagaagtgtttgatataacttattttta

SEQ ID NO: 678 - DNA, 25 bp, Artificial sequence
  primer
ctccatcaatccatgggaagactta

SEQ ID NO: 679 - DNA, 18 bp, Artificial sequence
  probe
tcgtccatatagttcaag

SEQ ID NO: 680 - DNA, 19 bp, Artificial sequence
  probe
atcgtccatattgttcaag

SEQ ID NO: 681 - DNA, 33 bp, Artificial sequence
  primer
cgatggttgttagatatatgtctagtcctaagt

SEQ ID NO: 682 - DNA, 27 bp, Artificial sequence
  primer
ggaagagaagaacaagaggaagacttt

SEQ ID NO: 683 - DNA, 16 bp, Artificial sequence
  probe
aacgttcaccatctct

SEQ ID NO: 684 - DNA, 16 bp, Artificial sequence
  probe
aacgttcacaatctct

SEQ ID NO: 685 - DNA, 25 bp, Artificial sequence
  primer
cgtataagtgtggtgccaattgttt

SEQ ID NO: 686 - DNA, 18 bp, Artificial sequence
  primer
ggatccttggcgctctcc

SEQ ID NO: 687 - DNA, 13 bp, Artificial sequence
  probe
cgcaaggacattc

SEQ ID NO: 688 - DNA, 14 bp, Artificial sequence
  probe
ccgcaagaacattc

SEQ ID NO: 689 - DNA, 22 bp, Artificial sequence
  primer
gcgtcttgtttgccaaatctgt

SEQ ID NO: 690 - DNA, 28 bp, Artificial sequence
  primer
ctttggtagttgttgttgaatctgttgt

SEQ ID NO: 691 - DNA, 21 bp, Artificial sequence
  probe
ctggttatacagctctgaagt

SEQ ID NO: 692 - DNA, 21 bp, Artificial sequence
  probe
ctggttatacagctatgaagt

SEQ ID NO: 693 - DNA, 31 bp, Artificial sequence
  primer
gcaacgaacaaaataaaagatggagatgtaa

SEQ ID NO: 694 - DNA, 27 bp, Artificial sequence
  primer
tctgtactttcttttaagcccttccaa

SEQ ID NO: 695 - DNA, 18 bp, Artificial sequence
  probe
aaaggctgaatccgtttt

SEQ ID NO: 696 - DNA, 17 bp, Artificial sequence
  probe
aaggctgaatcagtttt

SEQ ID NO: 697 - DNA, 20 bp, Artificial sequence
  primer
tggtttgctacctccgtttc

SEQ ID NO: 698 - DNA, 20 bp, Artificial sequence
  primer
tgcaaaaggcaaaagattca

SEQ ID NO: 699 - DNA, 17 bp, Artificial sequence
  probe
ctcatatccactgttgc

SEQ ID NO: 700 - DNA, 16 bp, Artificial sequence
  probe
ctcatagccactgttg

SEQ ID NO: 701 - DNA, 19 bp, Artificial sequence
  primer
acggctcatgttggatcgt

SEQ ID NO: 702 - DNA, 19 bp, Artificial sequence
  primer
acccatggtcgccacaaat

SEQ ID NO: 703 - DNA, 19 bp, Artificial sequence
  probe
attttgttttccctttttc

SEQ ID NO: 704 - DNA, 18 bp, Artificial sequence
  probe
ttttgttttgcctttttc

SEQ ID NO: 705 - DNA, 25 bp, Artificial sequence
  primer
tctgcccaaagtgaatcagtattca

SEQ ID NO: 706 - DNA, 25 bp, Artificial sequence
  primer
tgcaagaggatatgtcacagaactc

SEQ ID NO: 707 - DNA, 16 bp, Artificial sequence
  probe
ctgcctgaacctttta

SEQ ID NO: 708 - DNA, 16 bp, Artificial sequence
  probe
ctgcctgaagctttta

SEQ ID NO: 709 - DNA, 27 bp, Artificial sequence
  primer
cgagcattaatgacttaccatccttca

SEQ ID NO: 710 - DNA, 22 bp, Artificial sequence
  primer
acagcctcaggaacatcagaag

SEQ ID NO: 711 - DNA, 20 bp, Artificial sequence
  probe
cagagtagtaaccctggttt

SEQ ID NO: 712 - DNA, 20 bp, Artificial sequence
  probe
cagagtagtaacgctggttt

SEQ ID NO: 713 - DNA, 27 bp, Artificial sequence
  primer
gaccgtgttaagctgtaaatcgataac

SEQ ID NO: 714 - DNA, 37 bp, Artificial sequence
  primer
ggtctcttaaaataagtaactagtagtgaagaaatgt

SEQ ID NO: 715 - DNA, 18 bp, Artificial sequence
  probe
acttgcatgaccttcata

SEQ ID NO: 716 - DNA, 19 bp, Artificial sequence
  probe
cacttgcatgactttcata

SEQ ID NO: 717 - DNA, 20 bp, Artificial sequence
  primer
taataagccgagccaccaag

SEQ ID NO: 718 - DNA, 20 bp, Artificial sequence
  primer
gacgagggaggaaatgttca

SEQ ID NO: 719 - DNA, 14 bp, Artificial sequence
  probe
accaagcttctctc

SEQ ID NO: 720 - DNA, 15 bp, Artificial sequence
  probe
ccaagcttctgtcgc

SEQ ID NO: 721 - DNA, 25 bp, Artificial sequence
  primer
tgtcgattggctcttttgagattca

SEQ ID NO: 722 - DNA, 31 bp, Artificial sequence
  primer
agaagttatgaaaagagagaggtgtactact

SEQ ID NO: 723 - DNA, 19 bp, Artificial sequence
  probe
aggagtatcgtacatctca

SEQ ID NO: 724 - DNA, 19 bp, Artificial sequence
  probe
aggagtatcgtagatctca

SEQ ID NO: 725 - DNA, 20 bp, Artificial sequence
  primer
ttgctcggttttaacctcgt

SEQ ID NO: 726 - DNA, 20 bp, Artificial sequence
  primer
aagaaatgggggaaaggatg

SEQ ID NO: 727 - DNA, 16 bp, Artificial sequence
  probe
tcttcgctttatcacc

SEQ ID NO: 728 - DNA, 15 bp, Artificial sequence
  probe
cttcgctgtatcacc

SEQ ID NO: 729 - DNA, 23 bp, Artificial sequence
  primer
gaaggtttcctcgtggaatgact

SEQ ID NO: 730 - DNA, 24 bp, Artificial sequence
  primer
gatatgggtccttgcggtctattt

SEQ ID NO: 731 - DNA, 16 bp, Artificial sequence
  probe
tccctaagcagagaag

SEQ ID NO: 732 - DNA, 21 bp, Artificial sequence
  probe
attaatccctaagaagagaag

SEQ ID NO: 733 - DNA, 32 bp, Artificial sequence
  primer
cgtctacaatttcattagtctcaagaaaaaca

SEQ ID NO: 734 - DNA, 22 bp, Artificial sequence
  primer
gcttctggataattggattggg

SEQ ID NO: 735 - DNA, 19 bp, Artificial sequence
  probe
tgggatgtaatctggctat

SEQ ID NO: 736 - DNA, 21 bp, Artificial sequence
  probe
tttgggatgtaatttggctat

SEQ ID NO: 737 - DNA, 22 bp, Artificial sequence
  primer
gattgcgtttttgcgtgaagtc

SEQ ID NO: 738 - DNA, 25 bp, Artificial sequence
  primer
gcaactcatactgaaacgtgtttga

SEQ ID NO: 739 - DNA, 18 bp, Artificial sequence
  probe
ttgcaagtgtctttcatg

SEQ ID NO: 740 - DNA, 17 bp, Artificial sequence
  probe
tgcaagtgtcattcatg

SEQ ID NO: 741 - DNA, 22 bp, Artificial sequence
  primer
tgggagagagcctaagtttctg

SEQ ID NO: 742 - DNA, 21 bp, Artificial sequence
  primer
cgcaacactaggaaacacctt

SEQ ID NO: 743 - DNA, 14 bp, Artificial sequence
  probe
acaccatcaagaac

SEQ ID NO: 744 - DNA, 14 bp, Artificial sequence
  probe
acaccatcaagcac

SEQ ID NO: 745 - DNA, 21 bp, Artificial sequence
  primer
ttccatcaccactgaaacaga

SEQ ID NO: 746 - DNA, 18 bp, Artificial sequence
  primer
cgtggctatgcaccatcc

SEQ ID NO: 747 - DNA, 15 bp, Artificial sequence
  probe
ttcccaagacaaaac

SEQ ID NO: 748 - DNA, 13 bp, Artificial sequence
  probe
cccaggacaaaac

SEQ ID NO: 749 - DNA, 34 bp, Artificial sequence
  primer
aaacaaaaacaaaatcattctgagactttgaaac

SEQ ID NO: 750 - DNA, 27 bp, Artificial sequence
  primer
tgaagatgaactcgccgtatagaaaag

SEQ ID NO: 751 - DNA, 22 bp, Artificial sequence
  probe
tcaataaactaattactttttc

SEQ ID NO: 752 - DNA, 21 bp, Artificial sequence
  probe
caataaactaattgctttttc

SEQ ID NO: 753 - DNA, 22 bp, Artificial sequence
  primer
cttcgacggattccttgatgga

SEQ ID NO: 754 - DNA, 23 bp, Artificial sequence
  primer
ctgttcagcagagccaagataca

SEQ ID NO: 755 - DNA, 16 bp, Artificial sequence
  probe
ccctctttcgatgttc

SEQ ID NO: 756 - DNA, 18 bp, Artificial sequence
  probe
aaccctcttttgatgttc

SEQ ID NO: 757 - DNA, 26 bp, Artificial sequence
  primer
gtttttctgatgttgaaggaggttga

SEQ ID NO: 758 - DNA, 20 bp, Artificial sequence
  primer
gtgtcccgaccaacaattcc

SEQ ID NO: 759 - DNA, 16 bp, Artificial sequence
  probe
tccaccagaatttaga

SEQ ID NO: 760 - DNA, 17 bp, Artificial sequence
  probe
ctccaccagagtttaga

SEQ ID NO: 761 - DNA, 151 bp, Brassica napus
agtgtcaatatcaaaygagycctgattcaagaagtcgcagagtttctgtgaatayccaacsgagttcttagtttcrtctgtattcttcccatttgcatatcccttgtctagcttgagcttgggaatgtaggtggtggatcttatcggaatc

SEQ ID NO: 762 - DNA, 801 bp, Brassica napus
ctaagcatgatacaagagtctgcctttcggtccttttctttcaagtgggccacttttttttcccgaacgcagtccgaatatgaagcgcatggatacaagttatgacttggaatgaaagacaattcctttagctttgatttggtttgtttcttacgaatattttatattattatttgattgttttttacaattacgaatatccatatttttttattcgaatcgaaatggataatgaatcaaatcaaaawwtttgaatattccgcctagtcctagtttggagcctagtgaaaattaaaatagcttgacattagttctcaacatttacggtaatgattattaaggacaatcgaacttttcaatatagacgattaccaatttaccatatagggatatatagagcmgaagactcaaaacctttagttggacaaatggttaagtcacgagtgcaataacatattttatatacaaatgtcaacaattctgttagtagtcgttcgtgccacataattatatatctttgtgattttctgtttcgattaatctgtctcatagttgcagtcgttagctagtattaagatcaacaaattttcgggtgcatatttttttaagtttcttaattaaggatataaagtacgcgcgctcaactatttgtaaattaaaacatcactgcaagagttcagtcaaacaggggcagacccccactatggtccaagggagtcacttgacacccctaaaatagttaaataaatgaattgcatagaatatccaatggatttttgtagcagaaatagttactttgwa

SEQ ID NO: 763 - DNA, 527 bp, Brassica napus
  misc_feature (80)..(80): n is a, c, g, or t
aaactatggttctgttacacttgtgtgttctttaacttgaagcatacgagtctccaacgagttaggagcaggaaatccanaagtggcaaaactggctgtatatgtcattgtaggcatagcagttgcccaaggtatcgtggtggtaacggttttgttgtcggttcgaaaggtcctaggccgagcttttagcagtgacccgaaaatcatctcttatgctgcatcgatgatacctattgtcgcatgtggaaacttccttgatggtctccaatgcgttctctcaggttcttattgcttgcasactcgaccatatgtttctggaacaagaaaatattggtttaggctcctcctagcttatatatatatatgtccggttaatcctggtttggtatggtttaggggttgctagaggatgtggatggcagaaaattggagcgtgtgtaaatcttggttcatattatctcgttggagttccgttagggctattacttggtttccatttccacatcggtggtcgggtaataatcttt

SEQ ID NO: 764 - DNA, 801 bp, Brassica napus
  misc_feature (58)..(58): n is a, c, g, or t
  misc_feature (111)..(111): n is a, c, g, or t
  misc_feature (278)..(278): n is a, c, g, or t
  misc_feature (569)..(569): n is a, c, g, or t
  misc_feature (647)..(647): n is a, c, g, or t
  misc_feature (783)..(783): n is a, c, g, or t
aaattcatattatttactttgttatttatttttatttttctacaatttttatgtattntggaacaagtataattttaataaaatatgacgatataagtttgataatacganaagtttgtcaaccataataaaattattgttattcagatactccggtaattttattttttgactgaaaattccagtaaggttccaatcccagattagataattttatttgcattaatctgtatatcaaacattacttttgctaatctataccttgtataatatgtcanaattgcttttatcttttcaatatctatagattaaaatttataatcttttatagtctattcaacttgcgcagcatcatctcgtaggtgttaaaccctctgggttttctgaactttgttaaaccstctttatacgatagactagtagtgcgcaccaaaatcttgaacattattttataaaatcaaaaacaaaataaccaccaccttatctcggtcttgtatctgcagatgacccggtttaagtgcagaggattagctttcggcctgagctgggccaacatcatgggagattcnttctctttattctatgccttcaacttatgggttaaggtcctttcaggagaaaaaatctatgccccggaaacttctatnatagacagaaggtttcagaatccaaatccaacggtgaaagacccggaatcaataaaacaggttgacccggttggagatctatggatcactccaagcaacaagaaaatggtgagttactgtttcaacctcaccgtcnccgaccagatgtcaccgc

SEQ ID NO: 765 - DNA, 801 bp, Brassica napus
  misc_feature (283)..(283): n is a, c, g, or t
  misc_feature (301)..(301): n is a, c, g, or t
  misc_feature (544)..(544): n is a, c, g, or t
  misc_feature (643)..(643): n is a, c, g, or t
  misc_feature (725)..(725): n is a, c, g, or t
gggtaagctcaagcaactagagactgaggcaaaagctaaaaaggagagggtcaaagagctcgaggattctaaatatggtatccgagcttgcatcaatgtcgtaaggagggctctatcagaccaaggttgcagctgagaattttgacaccgatgtcataaaggatctagcagacactcagagggaaagtaagaagctcgttaaccggcttaaactggcgcaaagagctcataaggaggagttccagaggctgaatgaatcaagatccagaaggtttagaaaaanggcttgtcaagctgcagnggtgaaataccagtcgcattttgatcagatatgtgagctttggccgattctaagatcgtaaaggagaatgccttgttgatgtctcaggcggctagtcagwcaggtttgatcgataagatgacacaaaggggactcgtgggtcatgtggcagatcaggagatatgggtgcagtctctcaagaatttctaagtgaagatcgacgagatagacatcgtccaactagatccataaaaggatctaagngtctcacccgtttctgatgtctccagctgaaatagcctccctttggggccaattcctgagctaaatcctatcgatgattaagaggtcaggaattagacngtcatgtcagaaactgtgaccattccaggatggtcgagttgaggatcctcctgctgaccagaagaagaccgatgcaacaacngctgaggagcctctggatatagatcagtttgactcgaaactcgtctgtaactccgttgtggatgtttcgggcgctg

SEQ ID NO: 766 - DNA, 801 bp, Brassica napus
  misc_feature (54)..(54): n is a, c, g, or t
  misc_feature (199)..(199): n is a, c, g, or t
  misc_feature (568)..(568): n is a, c, g, or t
  misc_feature (801)..(801): n is a, c, g, or t
cacttatgcagtttgcgatctttgtggagacagggcagtctctagactcagacnacactttgcccacaagagctcttacctcttcattgtggcgtaatctcctatcgtagcagaaactatacggtcgtttcttccctgtagcagtgaaggacgagataagaggcctgtgatcagagccttcaaaagggagatagacacngtttcctttcgggaaacagtcagaccaggagatattggctagagcttgatccagtctgcagtgcactcgatgagtatgtctcgttcctctccaggagagaaaatttccacggtgtctcagatcaaagagatcattcgttgcgaggaaagtcctaaagttactgaaggagctttccggtctatctctgcctccagttttctcsgagttgtcagtgatttcgttgaaatctccagtcattaaccaaggatcgcttctcgaaccacctagctgtgtaagttggtcccatacttcttgtctatgggatacttcaagagctccataaacgaaggaactgaagaagtttgaatttttgtaggagatatgggtatntatgtagttaggagtcgccgtcagcacctggacctttacgtcagacttccagagcaggcagagcccccctgagcttggactgttcggtgaaacaaggaagtgaaactcaagaagtaaaggttccaggtctttaaggacaaaggcatctggattctttgtttcctggataaagatgatatctggagagaattttttgttgagagcaatgagcctttggactgttctgggattcn

SEQ ID NO: 767 - DNA, 474 bp, Brassica napus
  misc_feature (363)..(363): n is a, c, g, or t
aaaaaaatggagaataacgactaaaatgtccgtgagtaaacatcaaatcaacatactatttagatgttttaacgtgcggttggatttggccttacctccgcccagatcccccctttttgtaactgtgattgcccatcaacacctttctgacctgacccgacatattaacataactttwatttgggggtaaactaaaattgggttttgatccgtttatttctcagttacagacatgacgaagaacataagaagagagagagagagaggacgtacaacagagaagacgatgacgaagagtcgaagaccagtaacagagagagagagacgatgacgacgaccagtaacagagagagacgacgtagnagagagagagaaagacgacttagaacagacagagagagacgacaaccaagaacaaagagagagatgacaatgaacgacgaaacgtggagagcgagacgaagccagagagag

SEQ ID NO: 768 - DNA, 401 bp, Brassica napus
tggaaaattctataggttttattgtaatcttttgtttgaaaatcatttgtgtgtccataattgctctttgagagaattgttttcttgaatgctttgatggaacactttgccgcatatgaaaagggatgtagagaggatatgtggccggagtaccgtttgcaaaacaaccatggcaaggcacaaacaccatgtaagtacacwtctttgtcaatacctaacgagccttcaaactgatatctcattgaatttcgtattaggcttgcctagaatcagggaagggaaggactcaatctatgtagtcgtacataaaatgacacattttattccttgttaaaacgccaacgaataattgaatcgcacgcgagaacactttctttaaaaagtattttgactctattcca

SEQ ID NO: 769 - DNA, 801 bp, Brassica napus
cctaatttccctaatttttactatgtaatacaccaaactataaaaagttttatcaaacggacaatgttgagatttattattctaaatagatgtttgtctccctacattttcatattttgtaccgaaacatttatttaaaagatatgcaaagtagtgtgtagccaaatgctatcatgtttaaatttgccaagagcatatccacctatacagtgcagataattgtttacttttgttaagctacaaaaagatgttaagctgtaagagtgattcgcatgaaaaatctattacaataaaagagagttacctctctctayatgycaccacgtcatcaggaaatataagacgtttttggacacttggcacttcaccaaaccagcccgcgtctgatttgattttgtatmatccggtttwtctcatgcctctatcctggactgggccattattacaacttttccttgggcctttraaaacactatgacaagctcactagaattttatgtttcttcttcttctttgcggttgcgacagtggacaatttttttttcagaactaaagggacgttccaatctctcccgtaacgtatcaatacttcattaatctgttcttaactctgaggttttgcgtgattagccmactcctcccactggaaagcattcaatcgacatctttaatctaactttaagatgatatygtttatttttcttcktgacctttgtgatttctccatcttcttccactcacttcatctgttattgacatcataattcctcttcaacccycattctctctatagaaagccag

SEQ ID NO: 770 - DNA, 801 bp, Brassica napus
  misc_feature (50)..(50): n is a, c, g, or t
  misc_feature (300)..(300): n is a, c, g, or t
  misc_feature (328)..(328): n is a, c, g, or t
  misc_feature (548)..(548): n is a, c, g, or t
  misc_feature (629)..(629): n is a, c, g, or t
  misc_feature (742)..(742): n is a, c, g, or t
gcatcttggcattactagtttgtatttttattttgcaaagagaaccaaancttagttattacaatatgattatcttgcaacagtatttccaacagcgttattttagagtactaatactcatggctgctttttggagtgtctctctgcaaagttatttagctggaaaatcagtttatgatgaggtcagtatcaaccgcaaaggtgatacataaccagttcttaagcaacagctcgacctgccaaaccaccatctgttattttaaatgtcaaacaaagctcgttagcaagacacaaatatanttaccgggtagaatgattacggcaactntaagcctgcagcaaaccaacacgaagtctcattgttcacattaatgaagaacacgccgccttttctgctgaasttgtacttccatttgtcttcaaagaaattggtatgaagacaataagcaaagatgtgatggagtcgtgctttagaaacaattgtcaaagcccaaaaactaagaacaacaaatgccaaaattgtgaaagaacaacgaactggttttgcnagccaggaaatctgatcatgacagttgtccaacacagctgacgccaaccgcttgcattgtgtgttttgagaaacagccgcntcgtcaaacattgtccatgagaagagacatcaatgtgtatgaatgtggtggagcaatgaaataattaccaagtgataaactcccagtggatatgctgataattattatgaaantcaaattgagaaccagctttctcaaacccatgctctcagtttcttgccaccaaacatta

SEQ ID NO: 771 - DNA, 801 bp, Brassica napus
  misc_feature (241)..(241): n is a, c, g, or t
  misc_feature (245)..(245): n is a, c, g, or t
  misc_feature (495)..(495): n is a, c, g, or t
  misc_feature (570)..(570): n is a, c, g, or t
  misc_feature (765)..(765): n is a, c, g, or t
tagattgttatgttttgatatcatcacaaccaaataacatgccatgtatttccatcatcattatcgttatcattattttgccaacattattatcaatttatcactgttttgttaaataacgtatttccattatacggttcctttgttgttgatattatataatataaaaggtcacatgtattactattatcgaacatgacataatataaggattattagagcggaagctaaataaaatttngctngatattgtaatggtgctgcatcatgttttcttttttggtaaaattttaattgattacaccaaaatgttcgtatgttacaacttacaaggttgggactgaaatggctcgttgcttctctttccaaagaggcatcttagctctcctaaaatcgctatwcttgggcagatgatcatcatgaggatggtttcacttttgatttcctcctgctctgttttatgctttttgcccacttgttttgggttattattgnctattggcatttgtttttgcttgaactacctctagtcgttttgactagaatactttatgatttttaatcaatganaaaaaaaacagttacaaaaggatattaatagcagaaaactggatgaaactaaacaacagagctactcaaccacatcttaactttgaacaaagactagaaggtagacagtagagagggaaaccaacgaaacaagcttagaccaaggaattggtaaggaccgcaagaacaaatgggtcgcagcgagaaagagagagntggatgccctcaaaccatgttgcaacaccttcctac

SEQ ID NO: 772 - DNA, 618 bp, Brassica napus
taagacattgttttataatttattcaaacaattatttccattttaaccaaagttgagcaattattgtggaagtttgaaaaattggtagatttgtcagtaatgtactatctaaacccatcaatagagtgatggttgaagagagtattggtttccacccgcaatgcaaggaaatcaacttatctcatttgagttttgccgatgatattgtggtttttacrgatggttctccaatgtcgcttcagggtactctaaaggtctttgaagacttcactgctatgtctggtttgcagataaacatagcaaagtccacggtcttaactgctggtagaggaaagcatgtactagaggatgcagcagctgatgcgggtctctccgtttctgccctgcctattaggtatcttggactaccgcttaccaccaagataatgtgcagggatgattatgagccgcttattactaagatcaggaacyggttcctctcttggacgagcaaagctctctcatatgcaggtcgattacaacttataaaatcagttattgctagtatcacaaacttttggtgtgctgcgttctgtcttccgcaaaactgtatagcggaaatcgagagtatgtgctctg

SEQ ID NO: 773 - DNA, 790 bp, Brassica napus
ccattaacattaggacattacatcttttcttttttgttgctttttgtccgtacgttatcgtcgtccgtttgaaactttttaatcttatccctaattttttatcatcgtaagcaaatctagttttatgttcgagatatgatggttattgaaatatatatgggttgtgctttcaataatcttgtccatagtttttttgtcaaaaaaacccatccataatcaccagctaccgccacaaaatctttatacgttagcttgttgcagtgaactttaaaaaaaatattgttgttatttcaataaacacggacatgggccattatgcttaatagactttagtctacagctttatctctcaaaacccatagtaaaacacaagtctaatgatacaagctyagagcctaagcatttacaaatagaaatttaaggttaacttttataattgttatcaaacatttcataggcaaaagatagaaaatggacaaattaacaggtagtatacgatttctacattttagcagtattttatattaatcatgctattaatttagctgattaaatcattttatgtagtttatcttctttttatcaacttatagtttatctttgttggcaaataatttgttttctttttaaatcaaaatcgttgattttatccatggtaaactttgagtatctaacgcattataattttttaaggtctgggaaaataaatcgaatccaaaaatccaagccgaacccgatccaataaaaatgaatatcaaatggatcttattttatgatattttggattatg

SEQ ID NO: 774 - DNA, 801 bp, Brassica napus
cttgtctttcttttttgatagagagaatattgctctgctttctkattagaggctttgatwacatactttaggtggtaaagggtctgatccagattttctgaagaggtaacttgtattgattacatactttagatccagggtgcgtttataactgatacctttgcttgtggtggattttcttttgccagcgaagagctgtaagttttgtactttagtcaattttgcagctctacagaaccttctaagaagctacctcactagacaggtgattytaaagattctcttgygtctgctactgttcactcttagatctcagtctttcctgtttctgaagttacctttgccaactctacttattctcgtctttctcgctttctcactttttttgttcttagctttgyagacgggttaggttagtaaaagccagtggtaaaaaatatgactctgtagaaaggagtattatatcagtaacaaggagatgccttttcattctgaggacgacaaragtgaagactacctcttcaagattctgcagctcggaaatcaaattttgctcgcaagatttgctagggattagttataccccagttaaaagtcgacgactagagtggagtttcagacggagatcaaataacagatatgggacacagaggtgctgttggagctcttctggttcacaacatcagcagacagaaaacttttcagagcattggtagatggctttaactagctgcatagtaagaaaactactcgtgggtaacaagtcggatctaaagtacataagcactaaacatcggaagg

SEQ ID NO: 775 - DNA, 21 bp, Artificial sequence
  primer
cctgattcaagaagtcgcaga

SEQ ID NO: 776 - DNA, 21 bp, Artificial sequence
  primer
tcccaagctcaagctagacaa

SEQ ID NO: 777 - DNA, 19 bp, Artificial sequence
  probe
cttagtttcatctgtattc

SEQ ID NO: 778 - DNA, 19 bp, Artificial sequence
  probe
cttagtttcgtctgtattc

SEQ ID NO: 779 - DNA, 31 bp, Artificial sequence
  primer
aggacaatcgaacttttcaatatagacgatt

SEQ ID NO: 780 - DNA, 25 bp, Artificial sequence
  primer
tcgtgacttaaccatttgtccaact

SEQ ID NO: 781 - DNA, 15 bp, Artificial sequence
  probe
tagagccgaagactc

SEQ ID NO: 782 - DNA, 20 bp, Artificial sequence
  probe
atatatagagcagaagactc

SEQ ID NO: 783 - DNA, 25 bp, Artificial sequence
  primer
ccaatgcgttctctcaggttcttat

SEQ ID NO: 784 - DNA, 25 bp, Artificial sequence
  primer
agctaggaggagcctaaaccaatat

SEQ ID NO: 785 - DNA, 17 bp, Artificial sequence
  probe
atggtcgagtctgcaag

SEQ ID NO: 786 - DNA, 17 bp, Artificial sequence
  probe
atggtcgagtgtgcaag

SEQ ID NO: 787 - DNA, 24 bp, Artificial sequence
  primer
accctctgggttttctgaactttg

SEQ ID NO: 788 - DNA, 24 bp, Artificial sequence
  primer
aagattttggtgcgcactactagt

SEQ ID NO: 789 - DNA, 19 bp, Artificial sequence
  probe
tcgtataaagacggtttaa

SEQ ID NO: 790 - DNA, 22 bp, Artificial sequence
  probe
ctatcgtataaagagggtttaa

SEQ ID NO: 791 - DNA, 24 bp, Artificial sequence
  primer
ggagaatgccttgttgatgtctca

SEQ ID NO: 792 - DNA, 25 bp, Artificial sequence
  primer
gtcccctttgtgtcatcttatcgat

SEQ ID NO: 793 - DNA, 17 bp, Artificial sequence
  probe
ctagtcagtcaggtttg

SEQ ID NO: 794 - DNA, 17 bp, Artificial sequence
  probe
ctagtcagacaggtttg

SEQ ID NO: 795 - DNA, 23 bp, Artificial sequence
  primer
aaggagctttccggtctatctct

SEQ ID NO: 796 - DNA, 25 bp, Artificial sequence
  primer
cgatccttggttaatgactggagat

SEQ ID NO: 797 - DNA, 18 bp, Artificial sequence
  probe
cagttttctcggagttgt

SEQ ID NO: 798 - DNA, 19 bp, Artificial sequence
  probe
ccagttttctccgagttgt

SEQ ID NO: 799 - DNA, 22 bp, Artificial sequence
  primer
ttgcccatcaacacctttctga

SEQ ID NO: 800 - DNA, 28 bp, Artificial sequence
  primer
ctgagaaataaacggatcaaaacccaat

SEQ ID NO: 801 - DNA, 24 bp, Artificial sequence
  probe
catattaacataacttttatttgg

SEQ ID NO: 802 - DNA, 24 bp, Artificial sequence
  probe
catattaacataactttaatttgg

SEQ ID NO: 803 - DNA, 20 bp, Artificial sequence
  primer
ccatggcaaggcacaaacac

SEQ ID NO: 804 - DNA, 26 bp, Artificial sequence
  primer
cagtttgaaggctcgttaggtattga

SEQ ID NO: 805 - DNA, 19 bp, Artificial sequence
  probe
atgtaagtacacttctttg

SEQ ID NO: 806 - DNA, 19 bp, Artificial sequence
  probe
atgtaagtacacatctttg

SEQ ID NO: 807 - DNA, 21 bp, Artificial sequence
  primer
acttggcacttcaccaaacca

SEQ ID NO: 808 - DNA, 23 bp, Artificial sequence
  primer
cagtccaggatagaggcatgaga

SEQ ID NO: 809 - DNA, 20 bp, Artificial sequence
  probe
atttgattttgtatcatccg

SEQ ID NO: 810 - DNA, 20 bp, Artificial sequence
  probe
atttgattttgtataatccg

SEQ ID NO: 811 - DNA, 20 bp, Artificial sequence
  primer
gaagaacacgccgccttttc

SEQ ID NO: 812 - DNA, 29 bp, Artificial sequence
  primer
tcacatctttgcttattgtcttcatacca

SEQ ID NO: 813 - DNA, 19 bp, Artificial sequence
  probe
atggaagtacaacttcagc

SEQ ID NO: 814 - DNA, 19 bp, Artificial sequence
  probe
atggaagtacaagttcagc

SEQ ID NO: 815 - DNA, 23 bp, Artificial sequence
  primer
gctcgttgcttctctttccaaag

SEQ ID NO: 816 - DNA, 25 bp, Artificial sequence
  primer
caggaggaaatcaaaagtgaaacca

SEQ ID NO: 817 - DNA, 19 bp, Artificial sequence
  probe
ctaaaatcgctattcttgg

SEQ ID NO: 818 - DNA, 20 bp, Artificial sequence
  probe
cctaaaatcgctatacttgg

SEQ ID NO: 819 - DNA, 28 bp, Artificial sequence
  primer
acttatctcatttgagttttgccgatga

SEQ ID NO: 820 - DNA, 21 bp, Artificial sequence
  primer
gtaccctgaagcgacattgga

SEQ ID NO: 821 - DNA, 18 bp, Artificial sequence
  probe
tggtttttacggatggtt

SEQ ID NO: 822 - DNA, 20 bp, Artificial sequence
  probe
tgtggtttttacagatggtt

SEQ ID NO: 823 - DNA, 29 bp, Artificial sequence
  primer
tctcaaaacccatagtaaaacacaagtct

SEQ ID NO: 824 - DNA, 39 bp, Artificial sequence
  primer
tgcctatgaaatgtttgataacaattataaaagttaacc

SEQ ID NO: 825 - DNA, 16 bp, Artificial sequence
  probe
ttaggctctaagcttg

SEQ ID NO: 826 - DNA, 17 bp, Artificial sequence
  probe
cttaggctctgagcttg

SEQ ID NO: 827 - DNA, 25 bp, Artificial sequence
  primer
tcgtctttctcgctttctcactttt

SEQ ID NO: 828 - DNA, 29 bp, Artificial sequence
  primer
cagagtcatattttttaccactggctttt

SEQ ID NO: 829 - DNA, 14 bp, Artificial sequence
  probe
cccgtctacaaagc

SEQ ID NO: 830 - DNA, 15 bp, Artificial sequence
  probe
acccgtctgcaaagc